European Patent Specification EP 3 218 494 B1, published October 30, 2024. Title: Haploideninduktoren. Applicant: KWS SAAT SE. The sequence listing filed with the application follows.

SEQUENCE LISTING (65 sequences)

SEQ ID NO: 1 - DNA, 47944 bp, Zea mays
  misc_feature (12578)..(12677): n is a, c, g, or t
  misc_feature (22322)..(22421): n is a, c, g, or t
  misc_feature (42238)..(42337): n is a, c, g, or t
atggggagcagtgaggagcatgtttttttagatcccaccagaatatgtgcatccgtgtcacttcttgctcatgatctcattggccgaatgcttaatcgagaggtctcttcaaggcccaatgccaaagaagttctccgtaagttcaagcacccttgtaacttgtgctttatatatatgattctcaatttatcattgacttttcctaatggctttcaacacagggcaccatgggtcttattctacactgattgcccgcagaaagctgaattctctaacatatgggatactaacaaaactgcagctcccatgattcatcgggagatagtcaggtttggttactgtgagtcttcatcttcaaaatcctcaagtgacaactctgaagagcgagatgaatgcggtatagttgatgcactggtgacaacaataacacaggtgaggatctcagagcccaagaggagtcggctgttcagcctacccaacgggttgttgccgccaagcaggaacagtctccgaacatgaagatgatgaatccgtgtgtggctttctaacttgacctacctagctcccatccccatgcatgtataaacgacatttggggaatgggtagaaaagcagagattagggattttcgtttccgtcggtgcagttttggtgttccaatggagttgcgagatgtttatgtgccttagtcttcaatttgggggttgggggaaaagtaattttatgtttttgttttgtgtctgcagattcggaagatggacttggaggcaaggagcctacagcctagcattaaggctggtttgcttgcaaagctgagggagtataaatctgacctcaacaacgtcaagagtgagctcaagaggatatttgcgcccaatgccaggcaggctacccgggaggagctcctagagtttggaatggctgatactctcgctgtgagctaatgctaggacttgactgtgtctacgagactgctcctaacaataaactgaagaaagcaaaagaaatcattcaacgtattcgccgaagagaactctacaaggtagtatgatgctttaattgctcatatacaagtgtcattttgtcatgtcattacacatggttaggatacatacttaagtttctaacgtaggcgtccacacaacggattggtgcacggttctgccgatgtatcccacgcacgtgcatggaaggaggcaggcacccttccccgccgccccggatctcgcgccagcccccgccctaccccgcctgcccttccactcttcccccgccgcccccggtcaacgtcacgaacccgggcctcgtgccgctcgtcgtggccacactgttcgacgagcgagtcatagagctgctgagcgtgctcgctgatgcggcggtggggcgaccaggcaggtggtccatcggcgaagcgccatggtcgtcgtcggggggcacgaaccaggcggtgtacgcgcgccgcgcgcccggctcttcatcgcctccacccgctccagcgtctccaccacttccttcatcgagggccgactgcttggctcgctggccaggcagccgagcattagttgcgccgcttggaacgcctgcttttgttgatcgtttgttttggtctgatttcagtgggtctatccgcagagaggaagaagcagaagctctccgagatccaatccggcgttgaggaagctgaatcgctggtaaatagatgtcgcgacgcgttctgttttggggatccccttggctaacgggacatacgacatttggggaatgggtagaaaagcagagattagggatttttcgtttccgtcggtgcagttttggtgttccaacagagttgcgagatgtttatgtgccttagtcttcaatttgggggttgggggaaaagtaattttatgtttttgttttgtgtctgcagattcagaaaatggacctggaggcaaggagcctacagcctagcattaaggctggtttgcttgcaaagccgagggattataaatctgacctcaacaacgtcaagagtgagctcaagaggatatctgcgcccaatgccaggtaggctacccgggaggagctcgtggagtctagaatggctgatactctcgcagtgagctaatgctaggacttgactgtgtctacgagactgctcctaataataaactgaagaaagcaaaagaaatcattcaacgtattcgccgaagagaactctacaaggtagtatgatgctttaattgctcatatacaagtgtcattttgtcatgtcattacacatggttaggatacatacttaagtttctaacgtaggcatccacacaatggattggtgcacggttctgccgatgtatcccacgcacgcgcatggaaggaggcaggcacccttccctgccgccccggatctcgcgccagccatcgccctaccccgcctgcccttccactcttccccctgaaagtcgcatagagggggggtgaatagggcgaatctgaaatttacaaacttaagcacaactacaagccgggttaacgttagaaatataaacgagtccgagagagagggcgcaaaacaaatcatgagcaaataaagagtgagacacgatgatttgttttaccgaggttcggttcttgcaaacctactccccgttgaggtggtcacaaagaccgggtctctttcaaccctttccctctctcaaacggtcacttagaccgagtgagcttctcttctcaatcaaacggaacacaaagttcccgcaaggaccaccacacaattggtgtctcttgccttggttacaattgagtttgatcacaagaagaatgagaaagaaaagaagcgatccaagcgcaagagctcaaatgaacacaaatgtcgctctctctagtcactatttgatttggagtgattccggacttgggagaggatttgatcttttggagtgtctagaattgaatgctatagctcttgtaatatgttgaaggtgggaaacttggatgccattgaatgtggggtggttggggtatttatagccccaaaacaccaaaaaaggccgttggaaggctgctctcgcatggcgcaccggacagtccggtgcgccagccacgtcagcagaccgttggggttcgaccgttggagctctgacttgtggggcctctgggctgtccggtggtgcaccagacaggtcctgtaggatgtctggtgcgccaactgcacgtgctctgtcctctgcgcgcgcaggcgcgcattaaatgcgttgtagtcaaccgttgcgcgcgaagtagccattgctctgctggcacaccggacagtccggtgaattatagcggagcgccctctgattttcccgaaggtagcgagttcagcttcgagtgccctggtgcaccggacactgtccggtgcgccaaaccagggtgccttccgggatgtcttttgctctctttgtttgaaccctttcttggtctttttattggcttattgtgaacctttgacacctgtaaaacttatagactagagcaaactagttagtccaattatttgtgttggacaattcaaccaccaaaatcaattaggaaataggtgtgagcctaattccctttcaatctccccctttttggtgattgatgccaacacaaaccaaagcaagtatagaagtgcataattgaactagtttgcataatgtaagtgcaaaggttacttagaattgaaccaataaatattttcataagttatgcatggattgtttctttattttcatcattttggaccacgcttgcaccacatgttttgtttttgcaaatccttttgtaaatagtcaaaggtaaatgaataagattttgagaagcattttcaaaatttgaaattttctccccctgtttcaaatgcttttcctttgacttaaacaaaactcccccctcaaaaatcctactcatagtgttcaagagggttttaagatatcaattttgaaaatgctactttctcccccttttgaatataataagatatcaattgaaaaattcatcattttaaaaccttttgaaaatgggtggtggtgcggtccttttgctttgggctaatactttctccccctttggcatgaatcgccaaaaacgaatacttgagtgaaatataagcccctttaactactttctcctgctttggcgaacataatatgagtgaagattataccaaagttggagagttgcttgaagcgatggtgaaggatgagttatggagtggaggttaagcctttgtcttcgccgaagattccaattccctttcaatacacctatgacttggttgaaaatatacttgaaaacacattagtcatagcacatgaaagagatatgatcaaaggtatattaatgagctatgtatgcaagacatcaaaagaaattcctagaatcaagaatatttagctcgtgtctaagtttgttcatctagtggcttggtaaagatatcagctaattgttccttagtgttaatataggcaatctcgatatctccctttttttggtgatcccttaggaaatgataccgaatggctatgtgtttagtgcggctatgctcaacgggattatccgccatgcggattgcactctcattatcacatagaagaggaactttggttaatttttaaccatagtccctaagggtttgcctcatccaaagtaattgtgcgcaacaatggcctgcggcaatatactcggcttcggcggtagaaagagctacggaattttgcttctttgaagcccaagacaccagggaccttcccaagaactggcaagtcctcgatgtactctttctattaattttacaccccgcccaatcggcatccgaataaccaatcaaaatcaaaatgtggatcccgtaggataccaaagcccaaacttaggagtatgaactaaatatctcaagattcgttttacggccgtaaggtgagcttccttagggtcggcttggaatcttgcacacatgcatacggaaaagcataatatccggtcgagatgcacataaatagagtaaagagcctatcatcgaccggtatacctttttgatcgacggatttacctcccgtgtcgaggtcgagatgcccattggttcccatgggtgtcttgatgggtttggcatccttcatcccatacttgtttagaatgtcttgaatgtacttcgtttggctaatgaaggtgccctcttagcgttgcttcacttgaaatcacaagaagtacttcaactcccccatcatagacatctcgaatttctgtgtcatgatcctactaaattcctcacatgtagattcattagtagacccaaatataatatcatcaacataaatttggcatacaaacaaatcattgtcaagagttttagtaaataaagtaggatcggcctttccgactttgaaaccattagtgataaggaaatctctaaggcattcataccatgctcttggggcttgcttgagcccataaagcgccttagagagtttatatacgtgattagggtactcactatcttcaaagccgggaggttgctcaacatagacctcttccttgattggtccgttgaggaaggcacttttcacgtccatttgataaagcttgaagccatggtaagtagcataggcaagtaatatgcgaattgactcaagcctagctacgggtgcataggtttcaccaaaatccaaaccttcgacttgtgaataacccttggccacaagtcgggctttgttccttgtcaccacaccatgctcatcttgtttgttgcggaagacccacttggttcctacaacattttggttaggacgtggaactaaatgtcatacctcattcctagtgaagttgttgagctcctcttgcatcgccaccacccaatccgaatcttgaagtgcttcctctaacctatgtggctcaatagaggaaacaaaagagtaatgttcacaaaaatgagcaacccgagatctagtagttacccccttatgaatgtcgccgaggatggtgtcgacggggtggtctcgttggattgcttggtggactcttgggtgtggcgggcgttgctcgtcctccttgtcttgatcatttgcatctcccccttgatctatgccgtcatctagaggtggctcatttgattgatcttcttcttcatcaacttgagcttcatcctcattttgagtcggtggagatgcttgcatggaggaggacggttgatcttgtgtatttggaggctcttcggattccttaggacacacatccccaatggacatgttccttagcgcgatgcatggagcctcttcatcacctatctcatcaagatcaacttgctctacttgagagccgttagtttcatcaaacacaacgtcacatgaggcttcaactagtccagtggacttgttaaagaccctatatgcccttgtgtttgagtcataaccaagtaaaaagccttctacagtcttaggagcaaatttagattttctacctcttttaacaagaataaagcatttgctaccaaaaactctaaaatatgaaatattgggctttttaccggtgaggagttcgtatgatgtcttcttgaggattcggtgtagatataaccggttgatggcgtagcaagcggtgttgactgcctcggcccaaaaccgatccgaagttttgtactcatcaagcatggttcttgccatgtccaatagagttcgattcttcctctccactacaccattttgttgtggcgtgtagggtgaagagaactcatgcttgatgccctcctcctcaagaaagccttcgatttgagagttcttgaactccgtcccgttgtcgcttctaattttcttgatccttaagccgaactcattttgagcccgtcttaagaatccctttaaggtctcttgggtttgagatttttcctgtaaaaagaatacccaagtgaagcgagaataatcatccacaataactagacagtacttactcccgccgatgcttatgtaagcgatcgggccgaatagatccatgtgtaggagctccagtggcctgtcggtcgtcattatgttcttatgcggatgatgagagccaacttgcttccctgcttggcatgcgctacaaatcctgtctttctcaaaataaacatttgtcaatcctaaaatgtgttctccctttagaagcttgtgaagattcttcatcccaacatgtgcaagtcggcgatgccagagccaacccatgttagtcttagcaattaagcaagtgtcgagttcagctctatcgaaatctaccaagtatagctgaccctctaacactcccttaaatgctattgaatcatcacttcttctaaagacagtgacaccaacatcagtaaaaagacagttgtagcccatttgacacaattgggatacagaaagcaaattgtaatctaaagaatctacaagaaaaacattggaaatagaatggtcaggagatatagcaattttacccaatcctttgaccaaaccttgatttccatccccaaatgtgatcgctctttggggatcttggtttttctcatatgaggagaacatctttttctccccagtcatgtggtttgtgcacccgctgtcgagtatccagcttgagcccccggatgcataaacctacaaaataattttagttcttgattttaggtacccaaatggttttgggtcctttggcattagacacaagaactttgggtacccaaacacaagtcttggagcccttgtgcttgcccccaacatatttggcaactaccttgccggatttgttagtcaacacataagatgcatcaaaagttttgaatgaaatgtcatgatcatttgatgcactaggagttttctttctaggcaacttggcacgggttggttgcctagagctagatgtctcacccttatacataaaagcataattaggaccagagtgagacttcctagaatgaattctcctaattttgttctcgggataaccggcagggtataaaatgtaaccctcgttatcctgaggcatgggagccttgcccttaacaaagttggacaatcttttaggaggggcactaattttgacattgtttcccctttggaagccaatgccatctttaatgcccgggcgtctcccattataaagcatgccacgagcaaatttaaatttctcattttctaagttgtgctcggcaattttagcatctagttttgctatatgatcattttgttgtttaattaaggtcatatgatcatgaatagcattaacatcaacatctctacatctagtacaaatagatacatgctcaacagtagatgtagagggtttgcaagaattaagttcaacaatcttagcatgaagaatatcatttttatccctaagatcggaaattgtagttttgcaaacatcaaaatctttagccttagcaattaaattttcatttttctgttctaaggctagcaagagaaatgtttaattcttcaatcctagcaagcaaatcatcattattatctttaggattgggaattgaaacattacaaacatgtgaatcaaccttagcatttaaactagtattttcatgtctaaggttgtcaatcatctcatggcaagtgcttagctcactagatagtttttgacatttttctacttctagggcgtaagcatttttaaccttaacatgtttcttgttttccttaataagacaatcctcttgggaatccaaaaggtcatctttttcatgaatagcactaattaattcatttaatttttccttttgttccatgttaagattagcaaaaagggtacgcaagttatcctcctcatcactagcattttcatcactagaggtttcatatttagtggaggatcttgattttaccttcttccttttgccgtcctttgccatgaggcacttgtggccgacgttggggaagaggagtcccttggtgacggcgatgttggcggcgtcctcgtcgtcggaggagtcgcttgagctttcgtcggaatcccactcccgacaaacatgggcatcgccgcccttcttcttgtagtacttcttcttctcctttcttctccccttcttgtcgtcgccacggtcactgtcactagatatgggacatttagcaataaaatgaccgggcttaccacatttgtagcaaaccttcttggagcgggacttgtagtctttccccctcctttgtttgaggatttggcggaagctcttgatgacgagcgccatttcctcattgtcgagcttggaggcgtctattggttgtcgacttggtgtagcctcctccttcttttcttccgttgccttgaatgcgacgggttgagcttcggatgtggtgggttcgtcaagctcattgatctttctcgagccttcgatcatgcactcaaaacttacaaaatgcccgataacttcctcgggggtcattttagtatatctaggattaccacgaattaattgaacttgagtagggttaaggaaaataagtgatcttagaataaccttaaccacctcgtggtcgtcccactttatgctcccgaggttgcgcacttggttcaccaaggtcttgagccggttgtacatgtgttgtggctcctcccctttgcgaagccgaaaccgaccgagctccccctcgatcgtttcccgcttggtgatctttgtgagctcgtctccctcgtgcgcggttttgagcacatcccaaacctccttggcgctcttcaacccttgaactttgttatactcctctctacttaaagaggcgaggagtattgttgttgcttgagagttgaagtgctcgatttgggccacctcatcctcatcataatccttatcccctacggatggtacctgtgcaccaaactcaacaacatcccatatacttttgtggagtgaggttagatgaaatcgcattaaatcactccacctagcataatcttcaccatcaaaagttggtggtttgcctaacgggacggaaagtaaaggtgcatgtttagaaatgcgagggtagtgtaggggaatcttactaaacttcttacgctcttggcgtttagaagttacggagggcgcgtcggagccggaggttgatgttgatgaagtgtcggtctcgtagtagaccactttcctcatcctcttttgtttgtccccactccgatgaggcttgtgggaagaagatttttccttcttctctttgtggtgagaagaagatttcttctccttccctttgttggaggagctcttcttcttctccctccgtttggtgcgggactcttccaatgaagtgctctcgttgcttgtagtgggcttttcgccggtctccatctccttcttggcgtgatctcccgacatcacttcgagcggttaggctctaacgaagcaccgggctctgataccaattgatagtcgcctagagggggggtgaatagggcgaaactgaaatttacaaatataaacacaactacaagccgggttagcgttagtaatgaagaaacgagtccgcgagagagggcgcaaaacaaatcgcaagcaaatgaagagtgtgacacgtggatttgttttaccgaggttcggttctcgcaaacctactccccgttgaggaggccacaaaggcccgggtctctttcaacccttccctctctcaaacggtccctcggaccgagtgagcttctcttctctaatcaaagttgggaacaaaacttcccaacaagggccaccacacaattggtgcctcttgccttgattacaatgggtttttgatcacaagaacaagtgcgaaagaaaagaagcaatccaagcgcaagagctcaaaaagaacacggcaaatctctctctctaatcactaaagccttttgtggaattggagaggatttgatctcttttggtgtgtctagaattgaatgctagagctcttgtagtagttgagaagtggaaaacttggatgcaatgaatggtggggtggttggggtatttatagccccaaccaccaaacttgaccgttggctgggttgtctgttcgatggcgcaccggacagtccggtgcacaccggacagtccggtgcccctgccacgtcatcactgccgttggattctagccgttgaagcttctgacttgtgggcccgcctgggtgtccggtgcacaccggacatctactgttccttgtccggtgtgccggagtgggcgcgcctgacatctgcgcgcgcagagcgcgcattaaatgcgcggcagagagccgttggcgcggaaatagccgttgctctcgagtcgcaccggacagtccggtgcacaccggacagtccggtgaattatagtggacgggccgatggcttttcccgaagctggcgagttcctgaggccgacctcccttggcgcaccggacactgtccggtgtacaccggacagtccggtgaattatagcggagtcgcctctggcaattctcgaagggggcgagttggagcttgagtcctctggtgcaccggacgctgtccggtgtacaccggacagtccggtgctctcagaccagagggccttcggttcccactatgctcctttgttgaatccaaaaacttggtccttttattggctgagtgtgaaccttttacacctgtgtaatctataaacttgtgcaaacttagttagtccaattgtttgtgttgggcaattcaaccaccaaaattaattagggactaggtgtaagcctaattccctttcagttttcccgggcggtcatccatagaacaggtccttacggagaggcactcgagaaaccgctcgagcccccttgaagaccacaagcacaacatcataataagagaagggaaaacagcgtatcatagataatctcatcatgttcattgattagagttaagcaatagcataaagctaaacagtaataatccaacccaaataggtgaacaaggacatggataacaaaagctagtcaatccttaggcataaatgtgtaaagcgggaggtgaattaaataatgaataggacatagataggtcaagggacacttgcctccaccaaccgactgctgctcaggggcttctcctgcgggttcctcgggctcttcaaccggatcgttctctatgcgagcgcaaacatacacacatccacatatttaataccaaagaacagtacaccatacaatagaatgcaataagtaaacagacgttccacgcgggctcgcgagtacggttaagagagaaagaggaaaagacagtcgagaaacgatcacgttgcatgattataaattagccactagcttaatggaaggaaatttaatgtagacactatgtttagcgtaaagtaaagtcatgtttcatgtctaattattataagcaggtggagacaaataaaaggatagccgcgcggcgagacgcgcgacaaagctctctaaaacaaattaagaagttaacgactcgtcgcgcgactgagcacgcagcgagacacttcgccttagttaagaggagacgttaagcgtcgcgcgacgaagcgcacgacggcatacgtcgactaaactgagtccaaagtggaacgtcgcgtcaattcccacgcggcgttacaccttaaacaacctgaaacaaaatgaacgaatcaagcctgatcatccgccccccccnnnnnnnnnnnnnnnnnnnnnnnnnnnnnnnnnnnnnnnnnnnnnnnnnnnnnnnnnnnnnnnnnnnnnnnnnnnnnnnnnnnnnnnnnnnnnnnnnnnnaccgttcaacaaacaccgcccggggttccaaccgaccaggctccagatcgcccgaccgatcccccgtcccggcctcgcccccccccttcttcgctcgcccgcgctcgcggtgattgctcgttaagaagcgtgttgcgtcgcgcgcttcgccgcgcgacggatttatctaaaattcagattctatcctgtgttgcgtcgtgcgtttcgtcgcgcgacgatccattttgtttcaggttgtttaaggtgtaacgccgcgtgtgtattcacgcgacgttccactttggactcagtttagtcgacgtatgccgtcgtgcgcttcgtcgcgcgacgcttaacgtctcctcttaactaaggcgaagtgtctcgctgcgtgctcagtcgcgcgacgagtcgttaacttcttaatttgttttagagagctttgtcgcgcgtctcgccgcgcggctatccttttatttgtctccacctgcttataataattagatatgaaacatgactttactttacgctaaacatagtgtctacattaaatttccttccattaagctagtggctaatttataatcatgcaacgtgatcgtttctcgactgtcttttcctctttctctcttaaccgtactcgcgagcccgcgtggaacgtctgtttacttattgcattctattgtatggtgtactgttctttggtattaaatatgtggatgtgtgtatgtttgcgctcgcatagagaacgatccggttgaagagcccgaggaacccgcaggagaagcccctgagcagcagtcggttggtggaggcaagtgtcccttgacctatctatgtcctattcattatttaattcacctcccgctttacacatttatgcctaaggattgactagcttttgttatccatgtccttgttcacctatttgggttggattattactgtttagctttatgctattgcttaactctaatcaatgaacatgatgagattatctatgatacgctgttttcccttctcttattatgatgttgtgcttgtggtcttcaagggggctcgagcggtttctcgagtgcctctccgtaaggacctgttctatggatgaccgcccgggaaaacagtgcaaccatgagggtggaatggggtgcccttagctgaataattagaggatccggggtgtagttcacttagccgtcgtgccgtcaatggggctcggtgtatgcggctcgctctgccaagtttgggttcgccccttggggaggagtgcggtgcatttaggaaacctaacgggtggctacagtcccggggaatctttgtaaaggctatgtagtgatgccctgctgggtcaccttggtagtgatcaatggagagtcatgatctccgggtagaatgggaatcacggcttgtgggtaaagtgcacaacctctgcagagtgtttgaaaactgatatatcagccgtgctcacggttatgagcggccaagggagctccagtgattagtggtacttgatcagagatactttggtacaggtggttatgagatcgatgattctggttatgactatgatgctggtaagtggtactctttccgtttggaaaggagtacgtttgggttaataacttgggttaatgctaaaacttggctttctattagtaaataataatctgaccaactaaaagcaactgcttgacttatccccacataaagctagtccactacagccaaacaggatacttgctgagtatgttgatgtgtactcacccttgctctacacaccaaaccccccccccatccccaggttgtcagcattgcaaccactgctcagtcgaagatgaagctgtggaaggagacttccaggagttccaagattacgatgagttctaggtgtgggttagcggcaacccccagtcggctgcctgtgaaggccgcggttatctacgtttcttttccgcactttgatttattgtaagaactatatggacgtctcagacgtatgatgtaatcgactatttcccttagtaatactattttgagcactgtgtgatgatgtccatgttatgtaactgctgtgtacgtgaataactgatcctggcacgtacatggttcgcattcggtttgccttctaaaaccgggtgtgacataagtggtatcaaagccgtgctgactgtaggaccgctaacctagaatagaatggtcgctctaaggactatagacctctgtctctgccttgactttgatatcccttcaaaagttggtcataccgaccaaacctatgttctactatatattataccttgctgaaaatcatgttttattccagtccttcatttacttatgattcattatttgctggtcatattaattctgttctcacctttttgcttgcgatgtcttttgtagatggctcgacttagacacactgcacgaaagtcagtcatccccttcttaccctcccgccttgctgagcgtccgcttcgccgtcccgtggccggacagtccagccacttggagagactacaccaccgcctgcgtgaggagcaggagcgtcgacgacaggagcagcagagctcttccttctcgctccaccaggagatagagtctgtgaggagctgctcccctgtgcttcctctggagccgccccctccaccaccactgggcgccccagcttctggagtagctgctggaggagacccagacgatggagatggcgacgacagctcgagccacgacaccgacttctctgctaaccttgagccggaaggatgggttactcgacccatcactcgcgacgctgctcgcgggtgtcacttccacgatgcgctcgacaccctgctacgtcgggcatttaaccagcatacttggtctgtcgagtatcgctgtgtggtctaccagcacagtcgcggggtctacccggaccgctgggaggcaacctgcttggtgcgctgcccggagaacagtctccagggtgcggaggcctgctcagagcactattctatctctgagcgggactcagctgaggcagccatgcaagatgctgcacggcgtgcgctttcgcactactgctcggttttcggtggggcagctgacggtcttgacctgaagtattacccccgccgtccatctggcagcacaggaggcgtgattgtctcacctgtcggtgagggcaatcctaggttgagcagcacagtcaacctagccgccgtgctaaacacggagctggaccatgcattagacgagctgagtagggctcgtgctgagatcgccctgctgcgggctgagcgcgcggaacgtcgtcacctggatggtggttcccccgctcccgtcgggactcagcacccgtaccgctcacctcagcgtggacaccagtcttatggcaatcccgcctgcaagaccaagataactctagaaccatatatcgttagagttggatcttgtaattaatacgaaatatatacatagaagcttcagtcttagcgttagtctcggtcttagttagtcttagttaaacagggtagtttgctatatcctgtgcatttatgtttgtcatgatgaactatgtttggtttggatctttgtaatgattgtcaccagagtgtgggtaccccctgcattttggtttacctattatgttaatagagttagttatatagttgggaaaccttttattccactctcctctttatctgagaaactgtgtggtctgtgttggagatcagtgaagatgctcatctgttcagtgctgttgaagaattctattctcttttcttatgctgcaagatttgccagatcagtcctgatgtgtggttgcattctgcagatgtcagagaacaggcgcagaggaggaaggcgtgctcagcaggagcgagccgctcaacaggaggaggtgccccagcagcagcacctgccgcccccgcccccgatgtccatcgagcagatgtttctgatgcagactcaggcagttcaagccatcggtcagactctggccgccattcagcagcagcagcagcagcaggccccacctcaacctcagatgcctcagatgcccagagacaagcgtgctgaattcatgagaggtcatccaccaacgttcgctcattcttctgaccctatggatgctgaagattggctgcgcactgtggagcgggagttgcataccgctcagtgcgatgacagggagaaagtcctgtatggtccccgtctgttgagaggagcagcccagtcatggtgggagtcttacctcgccacccatgcccatcctgacgccatcacctgggaagagttcagaggtagctttcgtcagtaccatgttcctgcaggtctgatgacagtgaagaaggaggagttcctggccctcaaggaagggccattgtctgtcagtgagtaccgagacaggtttctgcaattgtctcgctatgctcctgaagatgtcaacaccgacgccaagcgacagtaccgtttcctgagaggcttggttgaccctctgcagtaccaactgatgaatcacaccttcccgacattccagcacctgattgacagagcaatcatgacagaaggaagcgtaaggagatggaagatcgtaagcgcaagatcagtggaccccagcctggaagcagcaatcgtcctcgtttctcaggcaatcaacctcagcagttcaggcagaaccagcgtccacctcagcagcagcagcaattccaaaggcagtatcctcagcaccagtaccagaaccgtcagagcaatcagtcaggaggtcagtttcagaggcagaatcagcaagcacctcgtcttcctgccccagcaaatcagcagaacagtcaggcagcaccagctcaggttggaaacagagcatgtttccactgtggagagcaaggccactgggtgatgcaatgtccgaagaaggcagcccagcagcagtcaggccccaatgccccagcgaagcagaatgtgcctcagcctggagcaggcaatcgctctcagccgcgctataatcatggaaggctgaaccacttggaggctgaagcagtgcaggagacccccggcatgatagtaggtatgttcccagtcgactcccatattgcagaagtgttatttgatactggagcaacgcattctttcattactgcatcatgggtagaagcacataaccttccaattactaccatgtcaacccccattcaaattgactcagccggtggtagaattcgagccgatagcatttgtttgaatataagtgtggaaataagggggatagcgtttcccgccaaccttatagtaatgggtactcaggcaatagatgtcatcctagggatgaattggctagataagtatcaggcagttatcagttgtgataaaaggaccatcaagttggtgtccccactaggagaggaagtggtgaccgagttagtcccgcctgagccaaagaaaggaagttgttatcagatagctgttgatagcagtgaagcagacccaatcgagaggatcaaggttgtgtccgagttcccagatgtgtttccaaaggacttaccgggtatgccaccagagcggaaagttgagtttgctatagagcttcttcccggaaccgcccctatctttaagagagcttacagaatatctggaccagagttggttgagcttaagaagcagattgatgagctgtcagagaaaggttacattcggccaagcacctcgccttgggccgcccctgtcctatttgtggagaagaaagatggcaccaagaggatgtgtatcgattatcgagctttgaatgaagtcacgatcaagaacaagtatcccttgcccagaatagaagatttgttcgaccagttgagaggagccagtgtgttctccaagattgatctgaggtcaggttatcatcagctcaggatccgaccttcggacattccgaagacggcattcatttccaagtatggtttgtatgagttcacagtgatgtcttttggtttgaccaatgcgccagcgttcttcatgaacttgatgaacagtgtattcatggattatctcgataagtttgtggtggtattcattgatgacattctggtttattctcaaagcgaagaagagcacgcagatcatttgaggttggtattgcagagattgcgagagcatcagttgtatgcaaagttgagcaagtgtgagttctggatcagtgaggtcctgttcttgggtcacataatcaacaaagaaggattggttgtggatccgaagaaagtggcagacattttgaactggaaagcgccaacagatgctagaggaatcaagagtttcattggaatggccggatactatcggcgattcattgaagggttttcgaagatcgcaaaaccaatgacagcgttgctaggcaacaaagttgagttcaagtggacccagaaatgtcaagaggcctttgaagcgctgaaagagaagttgactacagcgcctgtcctagtcttgcctgatgtgcacaagcccttctcagtgtattgtgatgcttgttacacaggtttgggatgtgtgttgatgcaagagggaagagttgtggcttactcgtcccgacaactgaaggttcatgagaagaattacccaatccatgatctagagttggcagcagtggttcacgcactgaagtcatggaggcactatctgtatggacagaaatgcgatgtttacacagatcacaagagtctgaagtacatattcactcagtcagagttgaacatgaggcaacgaagatggttagagttgatcaaagattatgagttggagattcattaccatccaggcaaagcaaacgtagtggcagatgctttgagcagaaagagtcaagtcaatctgatggtcgctcgtccgatgccttatgagttggccaaagagtttgacaagttgagtctcggttttctgaataattcgcgaggagtcaaagttgagttggaacctaccttggagcgcgaaatcaaagaagcgcagaagaatgatgagaaaatcagcgagatccggcgactgattctagatggcaaaggcaaagaatttcgagaagatgcagaaggcgtgatatggttcaaagaccgcttgtgtgttcctaatgtccagtctattcgggagttgattctcaaggaagctcatgagacgtcctattcgattcaccctggcagtgagaagatgtatcaggatctgaaaaagaaattctggtggtacggaatgaagagggagatcgcagagcatgtggctaggtgcgatagttgccgaagaattaaggcagagcaccagagacctgctggattgttgcaaccattgcagatccctcagtggaaatgggacgaaatcggtatggatttcatagtcggattgcctcgcactcgagccggctacgattccatctgggtagtagtggaccgcttgaccaagtcagcccacttcatacctgtcaagaccaactacagcagtgcagtattggcagaattgtatatgtctcggatcatttgtcttcatggtgtgccaaagaagatagtgtcagacagaggaacgcagttcacctctcatttctggcagcagttgcatgaagctttgggcacgcatctgaatttcagttcagcttatcatccacagacagatggccagaccgaaaggaccaaccaaattcttgaagatatgttgagagcctgtgcgttgcaagatcagtccggatgggataagagattgccttatgcagagttttcctgtaacaacagttaccaggccagcttgaagatgtcaccatttcaggcgctctatggaaggagttgtagaactccgttgcaatgggatcagcctggagaaaagcaagtgtttgggccagacattttgcttgaagccgaagagaacatcaagatggtccgagagaatctgaagatagcgcaatcgaggcagcgaagctatgcagacacaagaagaagagagctgagtttcgaagtcggagactttgtctatctgaaagtgtcaccaatcagaggagtcagaaggttcggagtgaaaggcaagctagcaccccgctacattggtccgtatcagattcttgcaagacgtggagaagtggcctatcagctcagtttgccagagaatttgtctgctgtgcatgatgtctttcatgtgtctcagttgaagaagtgcttgcgtgtgccagaagagcagttgccagtagaaggtcttgaagtccaggaggacttgacctacgttgagaagccagtgcaaatccttgaggttgcagaccgagtcacctggaggaagaccatcagaatgtgcaaagtcagatgggatcatcactctgaggaagaagcaacctgggagcgtgaagatgatctgatggccaagtaccctgagctctttgctagccaaccctgaatctcgagggcgagattcttttaagggggataggtttgtaacgccctgaatttgggggtagaatttttcttcttttctctcaccaaattcgggcgttactctcttttctctttccccgtttgctccttcttcccaatttcaaaccagtatagcggcaggtgtccgtgtcatgtataaaccaaaacctaagtgtcatgggtgttgcatcatgccgaagcacatttctttgtctgatgttgagtgttcgtctcgttccgttccggatttcggttcgcgatttaattccgtttagtggtccgcgctcgtcgcgggttttcgatccgcgaagtggcccgacccatcccaacctagtccagcccagcccagccggcccggcccgccccggcctgcgcgcccctggcgcccaaacccccccatgcgccccccctcctctctctctctcatttggatctcccgcgcaacaacctctcctctccctcttccacctctctctccccgtggtgccctaggatttggagacggcgatcaccggattttggaccccgaggtgagctcccctcccctccccttctcttctctctctctctccctcctcttcttctccccacgcgcgccccccttctccccctgctcacgcgcgcccctgcccgcccccgctcaccggcggcgcggcgccccccgcccctgcccggccccgcgcggcggcgcccgccctcccccggccgcggcggcgctcgtccgccctcacccccggccgcggcgcccgcccctccccctcgcgcgcggaggcggcgcccgccctcaccacgacccgcagcgaccccgccccgtccccgcctctccccccgcgcgcggcggcgcccgccccccgcccctccccgcggcggcgctcgcccgcccgcccctgcccctccccgcggcggcgcccgcccgcccctgctcgcgcgcagcgcggccccggcgcgcccccggcatggcccggcgcggccccggtggcccctgctcgccggcgcgaccccggcgtggcccccagcccccggcgcgtccccggcgcggccccggccggctcggccgcccctggccggttcaaccgccccccctggccggttcaaccgccctggccccagctcgcccgcccgttcccccgtcccggcctcgcccgaccgtatcttcgctcgcccgcgctcgcggtgattgctcgttaattagcgtgttgcgtcgcacgctacgccgcgcgacggatttatctaaaattcagattctatcctgtgatacgtagtacaactgacnnnnnnnnnnnnnnnnnnnnnnnnnnnnnnnnnnnnnnnnnnnnnnnnnnnnnnnnnnnnnnnnnnnnnnnnnnnnnnnnnnnnnnnnnnnnnnnnnnnntgggtcggcgctgagatcagcttgattcgtttttggttatacatgacacggacacctgccgctatactggtttgaaattgggaagaaggagcaaacggggaaagagaaaagagagtaacgcccgaatttggtgagagaaaagaagaaaaaattctacccccaaattcagggcgttacatcaggctacaaaggatgccaatggtattgctgctctctatattgttcttgttctaatgtaaaaactacaacacaactctttacttgatcccagaaattccttctgcctcaaatggagacaatgacgagtggtcataagtacagagattgcagacaaggtaaattttgcaatagaaataactaaccaaccattagtgcttgaaaaaaactggactggtgactggggcacgtggtttcatcaacatttggacctcaacggtctaatcagtataacttagaagttggctagctcttgaaaaacactgcatgacactaagcatttgtttattttcagctgcttacacccctatgatttcaagtaactacttgtctacttgtgataatcacctgaatatgattatttgaaatgcttatcatgtctcgtcaattgcatttcttttatgtgtacctgaagtctgctcttgcttcctaatagagttcgttttttaatacagaaaccactctgagatagccacaatatagtaaaagtggcagctaaggtactaaaaacacccatgcaaataagaaaaaaatgaatcttgtattttaattttgttaaatacctctatagtttggcgatatattatgttaccatcctgcttatagcctgtaggtcattttatatgagccatcaaattgcgatgacagttgccacaaatccagtttcatatgaaggtattagctgtgtaacaagctaattgttgctctctgcccaataagttattcaattggattagtaggttgcatccaaggttattcaattggatcagtaggttgcatccaaggtatactgctgctctctgcccaataagttattcaattcgatcagtaggttgcatgttcccttcattttattaaaaaatacataataatataataagtacttgtttgttctaaaaataatacttctgtaaatgaggatattaattttccttttggtaataatgcaggttgatgatactgaagtcatcagttttttgctgcaaactgaaataattcctctgtgcttgcgaaccatggagatgggtagtgagctatccaaaattgtatgtagctagccaaatattctcattcaaatatcataatttatctcttctgcttaatactggcaaaggtgtaatagtttttttagtattgatttgtcacctgaagtttatcttgtgcactactactttgccatcatcagttatctctagaatactcttgtcctgtaccattttctctctgataagcctaaatttgtacaattcataagcctaaaaggtgacttatataatatatacaaggaccctcaagagttgtttggcaattcagtgactgtcctgggtcctgttttggggagcttctggtagcttttgcttctccaaaagaaaagctagaagctccccccaaacagagcagcttcttcaagccggtaaaagcttcaaaagctgtaattatactaaaaacagtgaagctccctcagagcagcttcccagctctctaggagatgcttttggagaagctacagtttccccaaacagggccctgctctgttgaaccccccccttcctgatacatatttgaatatgagtttatagtgtgtgtgggggtgtaagtaggggggtaatgggttctaaattttatactataaaaattaaggatcggattagaattgagctctatttctattcatttttgaactaaaattaattaagggctcaaatgaattatgaagaagcattaggatcatgatccattaccacccctacgtgtaagatgttttttggtggttgtggttgattttgaattttaaggccgcatatgtctcatggaccacacaagctcatattcatctacatttgtagccgtcactaacttagccaaatatgcatatgtggcggctagcaacaggtccttggtttcttgggttatttattctctttttatcgtgtttgaatgttttcgtgttcatttgcataacatcttaggtctacattagtatatgaattgagatcaaatgtgaattggaccacacaagctcatattcatctacatttgtagtcgtcactaacttagccaaatatgcatatgtccgcttctgatttcattgtgtcttttcttcaggagtttggggatcaaggagaggactccattatcttgtcaccgcgactgaaggagattagtactcctgaccgccccactgccctccgtttcctaggtacacgcataacagccattggtatgaatacatgttttatacgtgaatggagttccagtttaatttaaagattcaagttcactacaacaagattttacagtactgagcccatttgactttccttgagaaatagtgaaagggaattaggcttacacctagttcctaaataattttggtggttgaattgcccaacacaaataattggactaactagtttgctctagtgtacaagttatacaggtgccaaggttcacaacaagccaattaaaaagaccaaagttgggttcaaaatagagagccaaaggcatcccgaaaggctccctggtttggcgcaccggactgtccggtggcgcaccggacagtgtccggtgcaccaggggacctcgcgcagaactcctcagcctcgggaatttttcggagccgccgcgctataattcaccggactgtccggtgtacaccggacagtgtccggtgctccaagaaaacgcggctccggaacttggcagcctcaggaaatcagaacggctgctccgctataattcaccagacatgtccggtgtacaccggactgtccggtgcaactgcggagcaacggctacttcgcgccaacggtcacctgcaggcgcattcaatgcgcgccagaagcgcgcagaagtcaggcacacccatgctggcgcaccggacactctacagtacatgtccggtgcgccaccggacatcaaggcgggcccagaagacagaactccaacggtcaaattccaacgactttggtgacgtggctggcgcaccggactgtccggtgcaccatatgacagacagcctccaccaacggtcatgtttggtggttggggctataaataccccaaccaccccaccattcattgcatccaagttttccagcttccaaccactatataagagctagcattcattgcaaagcacaccaaaagagatcaagtcctctcccaactccacacaaagccttagtgattagagagagtgatttgtagtgttcatttgagctcttgcgcttggatcgcttcttttctttggcattctttcttgtgatcaaacactcacttgtaattgaggcaagagacaccaattgtgtggtggtccttgcgggaagtttgattcccaagtgatttgagaagagaagctcactcggtccaagggaccgtttgagagagggaagggttgaaagagacccggcctttgtggcctcctcaacggggagtaggtttgagagaaccgaacctcggtaaaacaaatccacgcgtctcacttcattattcgcttgcgatttgttttcacgccctctctcggactcgttcttatttctaacgctaacccggcttgtagttgtgtttatatttgtaaatttcagtttcgccctattcaccccccctctaggcgactatcaattggtatcagagcccggtgcttcattagagcctaaccgctcgaagtgatgtcgggagatcacgccaagaaggagatggagaccggcgaaaagcccactacaagccacgggagcacttcatcggaagagtcccgcaccaagaggaaggagaagaaagactcctccaaagggaaggagaagaagaaggactcctccaaaggaaaggagaagaaatcttcttcacacaaagaaaagaaggagaagtcttcctcccacgagccgcaacggagtggggacaagaaaaagaggatgaggaaagtggtctactacgagaccgattcttcatcgacatccacctctggctccgacgcggcgtccgtcacttctaaacgccaagagcgtaagaagtatagtaagattcccctacgctaccctcgcatttctaaacatacacctttactttccgtcccattaggcaaaccaccaacttttgatggtgaagattatgctaggtggagtgatttaatgcgatttcatctaacctcactccacaaaagtatatgggatgttgttgagtttggtgcacatgtaccatccgtaggggatgaagactatgatgaggatgaggtgacccaaatcgagcacttcaactcccaagccacaaccatactcctcgcctctctaagtagagaggaatacaacaaggtgcaagggttgaagaatgcgaaagaaatttgggatctactcaagaccgcgcacgagggtgatgaactcaccaagattaccaagcaggaaacgatcgagggggagctcagtcgcttccgtcttcgccaaggggaggagccacaagatatgtacaaccggctcaaaaccttggtgaaccaagtgcgcaacctcgggagcaagaaatgggatgaccacgaggtggttaaggttattcttagatcactcatcttccttaaccccactcaagttcaattaattcgtggtaatcctagatatacactaatgacccccgaggaagttattgggaattttgtgagctttgaatgtatgatcaagggctcaaagaagatcaacgagcttgatgatccctccacgtccgaagcacaaccggtggctttcaaggcgacggaggagaagaaggaggagtctacaccaagtagacaaccaattgacgcttcaaagctcgacaacgaggagatggctttaatcatcaaaagctttcgccaaatcctcaagcaacggaaggggaaggattacaaatcccgttcaaagaaagtttgctacaagtgtggtaagcccggtcactttattgctaaatgtccattatcaagtgacagtgacagggataatgacaagaagggcaagaggagagaaaagaagaggtaccacaagaagaggggcggtgatgcccacgtatgccgcgagtgggactccaacgagagctccaccgactcctccgacgacgaggacgtcgccaacatcgccgacaccaagggactcctcttccccaacgtcggccacaagtgcctcatggcaaaggacggcaaaaacaagaaggataaatctaaatcctccactagatatgaatcctctagtgatgaaaatgttagtgatgaggaagataacttgcgatctctttttgccaacctcaacatgcaacaaaaagagaaacttaatgaattgattagtgtcattcatgaaaaggatgatctcttggacacccaagaggacttccttattaaagaaaataagaagcatgttaaggttaaaaatgcttatgctctaaaagtagaaaaatgtgaaaaattgtctagtgagctaagcacttgccatgagactataaacaaccttagaaatgagaatgctaatttgttagctaaggttgattctcatatttgtaatgtttcaagttccaatcctagagataataatgatgatttatttgctaggattaaagatttgaacatttcacttgctagccttagaaatgaaaatgaaaaattgcttgctaaggctaaagattttgatgtttgcaatgttactatttctaaccttagaagtgaaaacgacatattacatgctaaggttgtagaattaaaatcttgcaaacctcctacatctatagttgagcatgtatctatttgtactagatgtagagatattgatgttgatgctattcatgatcacatgactttaattaaacaacaaaatgatcatatagcaaaactagatgctaaaattgccgagcataacttagaaaatgaaaaatttaaatttgctagaagtatgctctatagtgggagacgccctggcatcaaggatggcattggcttccaaaggggagacaatgtcaaacttaatgcccctcctaaaagattatctaattttgtaaagggcaaggctcccatgcctcaggataacgagggttacattttgtaccctgccggttatcccgagagcaaaattaggaggattcactctaggaagtctcactctggccctaaccatgctttcatgtacaagggtgagacatctagctctaggcaaccaacccatgttaagttgcctaagaagaaaactcctagtgcatcaaatgaacatagcatttcatttaagacttttgatgcatcttatgttttgactaacaaatccggcaaagtagttgccaagtttgttgggggcaaacacaagggctccaagacttgtgtttgggtacccaaagttcttgtttctaatgccaaaggacccaaaaccgtttgggtacctaaagtcaagaactaaaattgttttgtaggtttatgcatccggaggctcaagttggatactcgacagcgggtgcacaaaccatatgacaggggagaagaagatgttctcctcctacgagaaaaaccaggatccccaacgagctatcacattcggggatggaaatcaaggtttggtcaaaggtcttggtaaaatagctatatctcctgaccattctatttccaatgtttttcttgtagattcattagattacaatttgctttctgtatctcaattatgcaaaatgggctacaactgtcttttcactgatataggtgtcactgtctttagaagaagtgatgattcaatagcatttaagggagtgttggagggtcagctatacttagtagattttgatagagctgaactcgacacttgcttaattgctaagactaacatgggctggctctggcatcgccgactagcacatgttgggatgaagaatcttcataagcttctaaagggagagcacattttaggattaaccaatgttcattttgagaatgacagggtttgtagcgcatgccaggcaggaaagcaagttggagcccatcatccacacaagaacatcatgacgaccgacaggccgcttgagctactccacatggatctattcggcccgattgcttacctaagcatcggcgggagtaagtattgtcttgtgatagtggatgattattctcgcttcacttgggtgttctttttgcaggaaaaatctcaaacccaagagaccttaaaaggattcttgagacgggctcaaaatgagttcgccttaaggatcaagaaaataagaagcgacaacggaacggagttcaagaactctcaaattgaaggcttccttgaggaggagggcatcaagcatgagttctcttctccctacacgtcacaacaaaatggtgtagtagagaggaagaatcgaactctattggacatggcaagaaccatgcttgatgagtacaagactttggatcggttttgggctgaggcggtcaacaccgcctgctacgccatcaaccggttatatctacaccgaatcctcaagaagacatcttatgaactcctaaccggtaaaaagcccaatatttcatattttagagtctttggtagcaaatgttttattcttgttaaaagaggtagaaaatctaaatttgctcctaagactgtagaaggctttttactaggatatgattcaaacacaagggcatatagagtctttaacaagtccactggacaagttgaagtttcttgtgacgttgtgtttgatgagactaacggctctcaagtagagcaagttgatcttgatgaaataggtaatgaagaggctccatgcatcgcgctaaggaacatgtccattggggatgtgtgtcctaaggaatccgaagagcctccaaatgcacaagatcaactatcctcctccacgcaagcatctccaccgactcaaaatgaggatgaagctcaagttgatgaagtagaagatcaagcaaatgagacacctcaagatgacgacaatgatcaagggggagatgcaaatgatcaagacaaggaggatgaagagcataggccgccacacccaagagtccaccaagcaatccaacgagatcaccccgtcgacaccatcctcggcgacattcataagggggtaactactagatctcgtattgcacatttttgtgagcattactcttttgtttcctctattgagccacacagggtagaggaagcactccaagattcggattgggtggtggcgatgcaagaggagctcaacaacttcactaggaatgaggtatggcatttagttccacgtcctaatcaaaatgttgtaggaaccaaatgggtcttccgcaacaagcaagatgagcatggtgtggtgacaaggaacaaagctcgacttgtggccaaaggatactcccaagtcgaaggtttggatttcggtgaaacctatgcacccgtagctaggcttgagtcaattcgtatattattggcctatgatacttaccatggctttaagctttatcaaatggacgtgaaaagtgccttcctcaatggaccaatcaaggaagaggtctatgttgagcaacctcccggctttgaagacagtgagtaccctaaccatgtctataagctctctaaggcgctttatgggctcaagcaagccccaagagcatggtatgaatgccttagagatttccttattgctaatggcttcaaagtcggaaaagccgatcctacactctttactaaaactcttgaaaatgacttgtttatatgccaaatttatgttgatgatattatatttggatctactaacgagtccacttgtgaagagtttagtaggatcatgacacagaaattcgagatgtctatgatgggggagttgaagtattttctaggattccaagtcaagcaactccaagagggcaccttcattagccaaacaaaatacactcaagatattctaagcaagtttggaatgaaggatgccaagcccatcaagacacccatgggaactaatgggcatctcgacctcgacacgggaggtaagtccgtggatcaaaagctataccggtcgatgataggttctttactctatttatgtgcatctcgaccggacattatgctttccgtatgcatgtgtgcaagattccaagccgaccctaaggaagcccaccttacggccgtaaaacgaatcttgagatatctggcttatactcctaagtttgggctttggtatcctaggggatccacatttgatttgattggttattcggatgccgattgggcagggtgcaaaatcaataggaagagcacatccgggacttgccagttcttgggaagatccttgggtgtcttgggcttcaaagaagcaaaattcggtcgctctttccaccgccgaagccgagtatattgcccgcaggccactgttgcgcgcaactgctttggatgaggcaaaccctgcgggactatggttacaaactaaccaaggtccctttgctatgtgataatgagagtgcaatcaaaatggtcgacaatcccgtcgagcatagccgcactaagcacatagccattcggtatcactttttgagggatcaccaacaaaagggagatatcgagatttcatacattaatactaacgatcaattagctgatatctttaccaagcctcttgatgaacaatcttttaacaaacttaggcatgagctcaatattcttgattctaggaacttcttttgttaaattgcacacattgttcttttatatacctttgatcatatctcttttatatgctatgactaatgtgttttcaagtctatttcaaaccaagtcataggtatattgaaagggaattggagtcttcggcgaagacaaaggcttccactccgtacctcatccttcgccatcacttcaagcaactctccgttctcgggggagataagcatgagcatcaaagaaaaggactttgggggagaaatgagcccaaagccaaaggaccggacttcgtctttggtataatcttaactcatttatttatgaccaaaagggaaaatagcacttcgagggctctaatgattccgtttttggcgattcatgccaaaaagggggagaaatgagcccaaagcaaaaggaccgcaccaccaccaatttcaaaaacttagtgttgaatatttttcaatttgtatcttattttcaattggtatcttattgtgttcaaaagggggagaaagtagtattttaaaatgatatatcaaaaaccctcttgaatactaagaggaggatctcttttagggggagttttgtttaagtcaaaggaaaagcatttgaaacagggggagaaaatttcaaatcttgagaatgctttgcaaaaatcctattcatttacctttgactatttgcaaaagaactttgaaaaggatttacaaaataatttgcaaaaacaaaactcgtggtgcaagcgtggtccaaaatgttatataaagaaagaaacaatccatgcatatcttgtaagtattcatattggctcaattccaagcaacctttacacttacattatgcaaactagttcaattatacacttctatatttgctttggtttgtgttggcatcaatcaccaaaaagggggagattgaaagggaattaggcttacacctagtccctaattaattttggtggttgaattgcccaacacaaacaattggactaactaagtttgcacaagtttatagattacacaggtgtaaaaggttcacactcagccaataaaaggaccaagtttttggattcaacaaaggagcatagtgggaaccgaaggccctctggtctgagagcaccggactgtccggtgtacaccggacagtgtccggtgcaccagaggactcaagctccaactcgcccccttcgggaattgccagaggcgactccgctataattcaccggactgtccggtgtacaccggacagtgtccggtgcgccaagggaggtcggcctcaggaactcgccagcttcgggaaaagccatcggcccgtccactataattcaccggactgtctggtgtgcaccggactgtccggtgcgactcgagagcaacggctatttccgcgccaacggctctctgccgcgcatttaatgcgcgctctgcgcgcgcagatgtcaggcgcgcccactccggcacaccggacaaggaacagtagatgtccggtgtgcaccggacacccaggcgggcccacaagtcagaagcttcaacggctagaatccaacggcagtgatgacgtggcaggggcaccggactgtccggtgtgcaccggactgtccggtgcgtcatcgaacagacaacccagccaacggtcaagtttggtggttggggctataaatacccccaaccaccccaccattcattgcatccaagttttccacttctcaactactacaagagctctagcattcaattctagacacaccaaaagagatcaaatcctctccaattccacaaaaggctttagtgattagagagagagatttgccgtgttctttttgagctcttgcgcttggattgcttcttttctttcgcacttgttcttgtgatcaaaaacccattgtaatcaaggcaagaggcaccaattgtgtggtggcccttgttgggaagttttgttcccaactttgattagagaagagaagctcactcggtccgagggaccgtttgagagagggaagggttgaaagagacccggcctttgtggcctcctcaacggggagtaggtttgcgagaaccgaacctcggtaaaacaaatccacgtgtcacactcttcatttgcttgcgatttgttttgcgccctctctcgcggactcgtttcttcattactaacgctaacccggcttgtagttgtgtttatatttgtaaatttcagtttcgccctattcaccccccctctaggcgactatcaaaaacagtgcaaccatgagggtggaatggggtgcccttagctgaataattagaggatccggggtgtagttcacttagccatcgtgccgtcaatggggctcggtgtatgcggctcgctctgccaagtttgggttcgccccttggggaggagtgcggtgcatttaggaaacctaacgggtggctacagtcccggggaatctttgtaaaggctacgtagtgatgccctgctgggtcaccttggtagtgatcaatggagagtcatgatctccgggcagaatgggaatcacggcttgtgggtaaagtgcacaacctctgcagagtgtttgaaaactgatatatcagccgtgctcacggttatgagcagccaagggagctccagtgattagtggtacttgatcagagatactttggtacaggtggttatgagatcgatgattctggttatgactatgatgctggtaagtggtactctttccgtttggaaaggagtacgtttgggttaataacttgggttaatgctaaaacttggctttctattagtaaataataatctgaccaactaaaagcaactgcttgacttatccccacataaagctagtccactacagccaaacaggatacttgctgagtatgttgatgtgtactcacccttgctctacacaccaaaccccccccccatccccaggttgtcagcattgcaaccactgctcagtcgaagatgaagctgtggaaggagacttccaggagttccaagattacgacgagttctaggtgtgggttagcggcaacccccagtcggctgcctgtgaaggccgcggttatctacgtttcttttccgcactttgatttattgtaagaactatatggacgtctcagacgtatgatgtaatcgactatttcccttagtaatactattttgagcactgtgtgatgatgtccatgttatgtaactgctgtgtacgtgaataactgatcctggcacgtacatggttcgcattcggtttgccttctaaaaccgggtgtgacacctgattactctcaagcaaagcctataggtagtttaagaggttgagtacaatgagaaacatttcaatcattatttgcaaaagaaacattttgatcatattaaggaaaatcataggagtgaaagaaaaacaatgtgtgcaaataactgaacctcctgcagctccatcatgctggccaaagtatgcttcgacgaattcaaaatatcatcatatgcttgctctatctgcttatcatgattgcaaccttgttcggatgggttcctggcttcctgcaacagcacagtagaaaacaaactggagtttagaattcaacttgagacttcagagttgaaacaaaacctgtattcacatatgtagcaccgatgcatatacaaatacctttatcagaaacatgaagatatgtgaatacattattttctcaataaaagtcatgatagaattcatgcaaatttttttagaaataaataaatgatgaggcatactacaattctaaaagcagtagcagtgcaacacgaacgaacattcaaattgccccacattcttgaaactgtgctgctttgctctcgttccaaaaaaactccgctaaagtaaaacttggaaaggtctggttttgcgtgagccaccaacaccaaccaaactttacgtcactatgacagtttcagcctttcggtcccggcgacagccatggcggacgcgggggtgacagggggtgctggccaagctgggtgagctgacggaggaggaggcgacgacgctgctgcgcgtggacgccgagatacgggcattgtggcagaagctggcctacctgcaggcgctcgtacgcggggccggccgccagcgccgcgaccgcgcaagcgagctgctcctgctctggctacgcgagaccagagaggttgctttcgcgggtggttctgccatacatagcggcgatggctcttcctcccaggactaccatatctacacataacaatcatgctctcatgaagttgtgatgtaataggtcacacgattttaatgtataagattgtgaagagtaaattaattcaaatgaattcatggacatgggacaactatgtgttaaaaacagaatctcctatgtatcctaaccatgtgtaatgacatgacaaaatgacacttgtatatgagcaattaaagcatcatactaccttgtagagttctcttcggcgaatacgttgaatgatttcttttgctttcttcagtttattgttaggagcagtctcgtagacacagtcaagtcctagcattagctcactgcgagagtatcagccattccagactccaggagctcctcccgggtagcctgcctggcaatgggcgcagatatcctcttgagctcactcttaatgctaggttgtaggctccttgcttccaggtccatcttccgaatctgcagacacaaaacaaaaacataaaattacttttcccccaacccccaaattgaagactaaggcacataaacatctcgcaactccgttggaacaccaaaactgcaccgacggaaacgaaaaatccctaatctctgcttttctacccattccccaaatgtcgtatgtcccgttagccaaggggatccccaaaacagaacgtgtcacgacatctatttaccagcgattcagcttcctcaacgccggattggatctcagagagcttctgcttcttcctctctgcggacagacccaccgaaatcagaccaaaacaaacggtcaacaaaagaaggctttccaagcggcgctactgacgctcggctgcctggccggcgagcctcgcagtcggccctcgatgaaggaggtggtggagacgctggagcgggtggaggcgatgaagagccgggcacgcggcgcgcgtacaccgcccggttcctgcccccccccccccccgacgacgaccatggcgcttcgccgatggcccacttgcctggtcgccccgccgtcgcgtcagcgagcgcgctcagcagctccgtgacccgctcgtcgaaccgcgtggccacggcgagcggcacgaggcctgggttcgtgacgttgaccggggggcggcgggggtgaaagggaattaggctcacacctatttcctaattgattttggtggttgaattgtctaacacaaataattggactaactagtttgctctagtctataagttttacaggtgccaaaggttcataataagccaataaaaagaccaagaaagggttcaaacaaaaagagcaaaagacatcccggaaggcaccctggtctggcgcaccggactgtccggtgtgccaccggacagtgtccggtgcaccagggcactcgaagctgaactcgctaccttcgggaaaatcagagggcgctccgctataattcaccagactgtccggtgaagcaccggactgtccggtgtgccagcggagcaacggctacttcgcgcgcaacggtcgactgcaacgcattcaatgcgcgcctgcgcgcgcagagggcagagcactcacagttggcgcaccggacagtctacaggacctgtccggtgcaccaccggacagcccagaggccccacaagtcagagctccaacgatcgaaccccaacgatctgctgacgtggctggcgcaccggactgtccggtgcgccatgcgaccgcagccttccaacggccatttttggtggtttagggctataaataccccaaccaccccacattcaatggcatccaagtttcccaccttcaacacattacaagagctataacattcaattctagacactccaaaagatcaaatcctctcccaagtccggaatcactccaaatcaaatagtgactagagagagcgacatttgtgttcatttgagctcttgcgcttggatcgcttcttttctttctcattcttcttgtgatcaaactcaattgtaaccaaggcaagagacaccaattgtgtggtggtccttgcaggaactttgtgttccgtttgattgagaagagaagctcactcggtctaagtgaccgtttgagagagggaaagggttgaaagagacccggtctttgtgaccacctcaatggggagtaggtttgcaagaaccgaacctcggtaaaacaaatcatcgtgtctcgctctttatatttctaacgttaacccggcttgtagttgtgcttaagtttgtaaatttcagattcgccctattcaccccccctctaggcgactttcaattggtatcggagccggtgcttcattagagcctaactgctcgaagtgatgtcgggagcatccgccatgagggatctcgggaccggcgacaagaccgcatgctcgggaagaactcactcaagggagtccgcccacaagcataaggaggaatcgtcttcctccatcaagtcccatcggatgggtgacaaaaagaagaagatgaggaaggtggtctactacgagaccgactcttcgtcaccctccacctccggctcggaatcggcctccaccacttcaaagcgccatgagcgcaagaagtatagtaagatgccccttcgctatcctcgcatttctagacgcactccatcactcttcgttccattaggcaaaccacctatatttgaaggtgaagattattctatgtggagtgataaaatgaggcatcacctaacctcactccacaaaagcatatgggatattgttgagtatggagtgcaggtaccaaagaagggagataaagattacgactcggaggaggttgaacaaatccaacatttcaaatccaagtcgagaggagtataataaggtgcaagggttgaagagtgcaaaggatatctgggacgtgctaaagaccgcgcacgaaggagacgaggtaaccaagatcaccaagcgggagacgatcgagggggagctcggtcgcttccggcttcgccaaggggaggagccacaagatatgtacaaccggctcaagaccttggtgaaccaagtgcgcaacctcgggagcaaaaaatgggatgaccatgaaatggttaaggttattcttagatcacttgtgttccttaaccctacgcaagttcaattaattcgtggtaatcctagatatacactaatgactcccgaggaagtaataggaaactttgtgagctttgagttgatgatcaaaggctcaaagaaaattatcgagcacgacggtccctccacgcccgaagcacaaccggtcgcattcaaggcgacagaggagaagaaagaggagtctacatcaagtagacaacccatcgacgcctctaagctcgacaacgagaaaatggcgctcatcatcaagagcttccaccaaatcctcaaacaaaggaaggggaaagattacaagccttgttccaaaagggtgtgctacaagtgtggtaagcccggtcatttcattgttaaatgtcctttatctagtgatagtgacaggggcgacgacaagaagggcaagaggagagaaaagaggaggtattacaagaagaagggcggcgatgcccatgtgtgccgcgagtgggactccgacgagagttcctccgactcctcatccgacgaggacgccgccaacatcgccgtcaccaaagggctcctcttccccaacgtcggccacaagtgcctcatggcaaaggacggcaaaaagaagaaggtaaaatcaaaatcctccactaaatatgcatcctctagtgatgaagataatgctagtgatgaggaggataatttgcgtaccctttttgtcaacctaaacatgcaactacaggaaaaactaaatgaattaattagtgctattcatgagaaagatgatctcttggactttcaagaggacttcctaattaaggaaaataagaagcatgttaaggttaaaaatgcttatgctctagaagtagaaaaatgtgaaaaattatctagtgagctaagcacttgccatgatactattaccatccttagaaataaaaatactaaactaattgctaaggttgattctaatatttgtgatgtttcaattcccaatcttagagatgataatgttaatttgcttgctaagattgaagaattgaatgtctctcttgctagccttagggttgaaaatgaaaaattgattgctaaggctaaagaattagatgtttgcaatgcttccatttctgatcttagaaataacaatgatattttacgtgctaagattgttgaacttaattcttgcaaaccctctacatctgccattgagcatgtcattatttgcactagatgtagagatattaacattgatgctattcatgatcatatggctttaattaaacaacaaaataatcatatagcaaaattagatgctaaaattgccgagcatgacttaaaaaatgaaaaatttaaatttgctagaagcatgctctatagtgggagacgccctggcatcaaggatggcattggcttccaaaagggaaacaatgtcaaacttaatgcctctcctaaaagattgtcaaactttgttaagggcaaggctcccatgcctcaggataatgagggttacattttgtaccctgccggttatcccgagagcaaaattaggagaattcattctaggaagtctcactctggccataatcatgcttttatgtataagggtgagacatctagctctaggcaatcaacccgtgcaaaattgcctaagaagaaaactcctgctgcatcaaatgatcataacatttcattcaaaacttttgatgcatcttatgttttaactaacaaatccgacaagatagttgccaagtatgttgggggcaaacacaagggatcaaagacttgtgtttgggtacccaaagttcttgtatctaatgtcaaaggacccaaaaccatttgggtacctaaaatcaagaactaaacttgttttgtaggtttatgcatccgggggcccaagttggatcatcgatagcgggtgcacaaaccatatgacaggggagaagaaaatgttctcctcctatgagaaaaaccaagatccccaaagagcgatcacattcggggatggaaaccaaggtttggtcaaaggattgggtaaaattgctatatctcctgaccattccatttccaatgtgtttcttgtagattctttagattacaacttgctttcagtttcgcaattatgtaaaatgggctacaactgtctttttacagatataggtgttactgtctttagaagaagtgatgattcagtagcatttaagggagtgttagagggtcagctatacttggtagattttgatagagctgaactcgacacttgcttaattgctaagactaacatgggctggctctggcatcaccgactagcacatgttggaatgaagaatcttcacaagcttctaaagggagaacacattttgggactaacaaatgttcactttgagaaagataggatttgtagcgcatgtcagacagggaagcaagttggtactcatcatccacacaagaacatcatgatgactgacaggccactcgagctcctacatatggacctattcggcccgatagcttacataagcatcggcgggagtaagtactatctagttattgtggatgattatactcgcttcacttgggtattctttttgcaggaaaaatctcatacccaagagaccttaaagggattcttgggacgggctcaaaatgagttcggcttaagaatcaaatttgttttaagcgacaacgggacggagtcaagaatctcaaatcgaaggcacgatctcctagatccggcccaaaannnnnnnnnnnnnnnnnnnnnnnnnnnnnnnnnnnnnnnnnnnnnnnnnnnnnnnnnnnnnnnnnnnnnnnnnnnnnnnnnnnnnnnnnnnnnnnnnnnncgctgatgaatcagcttgattcgtgacacgggaggtaagtccgtggatcaaaaggtataccggtaagataataggctctttactctatttatgtgcatctcgaccggatattatgctttccgtatgcatgtgtgcaagattccaagctgaccctaaggaagctcaccttacggccgtaaaacgaatcttgagatatttggcttatactcctaagtttgggctttggtatcctaggggatccacatttgatttgattggttattcggatgctgattgggcggggtgtaaaatcaatagaaagagcacatcagggacttgccagttcttgggaagatccttggtgtcttgggcttcaaagaagcaaaattcggtcgctctttccaccgccgaagccgagtacattgccgcaggccattgttgcgcgcaattgctttggatgaggcaaaccctgcgggactatggttacaaattaacctaagtccctttgctatgtgataatgagagtgcaatcaagatggcggataatcccgtcgaacatagccgcactaaacacatagccattcggtatcattttcttagggatcaccaacaaaagggagatatcgagatttcttacattaacactaaagatcaattagccgatatctttaccaagcctcttgatgaacaaacctttaacaaacttaggcatgagctcaatattcttgattcgcgcaatttcttttgctaaattgcacacatagctcatttatatacctttgatcatatctctttcatatgctatgactaatatgttcttcaagtctatttcaaaccaagtcataggtgtattgaaagggaattggagtcttcggcaaagacaaaggcttccactccgtaactcatccttcgtcgtcgctctgggccactctccatctttgggggagagagcaaaagacttcgtctttggtacaatcttaactcatttatttatgaccaaaggggaagaaagtacttcgagggctctaatgattccgtttttggcgattcatgccaaagggggagagagtatgagcccaaagcaaacggaccgcaccaccaccaatttcaaaaacttagtttttcaaagagtattttcaattggtatcctattgtgttcaaaagggggagaaagtagtattttcaaaaatgatatatcaaaaccctcttgaacactaagaggtggatctcatttagggggagttttgtttagtcaaaggaaaagcatttgaaacagggggagaaaatttcaaatcttgaaaatgcttcataaaatcgtattcatttacctttgactttttgcaaaagaactttgaaaaggatttacaaaatagtttgcaaaaacaaaacatgtggtgcaagtgtggtccaaaatgataaaaacaaaggaacgatccatgcatatcttgtaagtatttatattggctcaaatccaagcaacctttgcacttacattatgcaaactagttcaattatgcattttatacttgctttggtttgtgttggcatcaatcaccaaaaagggggagattgaaagggaattaggcttacacctagttcctaaataattttggtggttgaattgcccaacacaaataattggactaactagtttgctctagtgtacaagttatacaggtgccaaggttcacaacaagccaattaaaaagaccaaagttgggttcaaaatagagagccaaaggcatcccgaaaggctccctggtttggcgcaccggactgtccggtggcgcaccggacagtgtccggtgcaccaggggacctcgcgcagaactcctcagcctcgggaatttttcggagccgccgcgctataattcaccggactgtccggtgtacaccggacagtgtccggtgctccaagaaaacacggctccagaacttggcagcctcgggaaatcagaacggctgctccgctataattcaccggacatgtccggtgtacaccggactgtccggtgcaactgcggagcaacggctacttcgcgccaacggtcacctgcaggcgcattcaatgcgcgccagaagcgcgcagaagtcaggcacgcccatgctggcgcaccggacactctacagtacatgtccggtgcgccaccggacatcaaggcgggcccagaaggcagaactccaacggtcaaattccaacggctttggtgacatggctggcgcaccggactgtccggtgcaccatacgacagacagcctccaccaacggtcatgtttggtggttggggctataaataccccaaccaccccaccattcattgcatccaagttttccagcttccaaccactatacaagagctagcattcattgcaaagcacaccaaaagagatcaaatcctctcccaactccacacaaagccttagtgattagagagagtgatttgtagtgttcatttgagctcttgcgcttggatcgcttcttttctttggcattctttcttgtgatcaaacactcacttgtaattgaggcaagagacaccaattgtgtggtggtccttgcggggagtttgattcccaagtgatttgagaagagaagctcactcggtccaagggaccgtttgagagagggaagggttgaaagagacccggcctttgtggcctcctcaacggggagtaggtttgagagaaccgaacctcggtaaaacaaatccacgcgtctcacttcattattcgcttgcgatttgttttcacgccctctctcggactcgttcttatttctaacgctaacccggcttgtagttgtgtttatatttgtaaatttcagtttcgccctattcaccccccctctaggcgactatcaaatagccagtgctttttggtctgcgagttcctgcacttggttaatcaactgtgtcgcttgatcttctacttgtttgcacgagaaggtcaaagccactttcgaagctattagttcagaacacacaacatctagctaaatacatcaccagtttgaagtcattgattgtattcttgatatcatctttattcttgaatgtcatttgtgccagttcatttaactcttgtgctgcaaaccaacctgacatcgtcaattcatttaatctctcaatctcagtttcctttttttgtttcacattgaagctccctaattgttgcttctcgatgtgcagtggcctgattagctacaagaagctcttgttccatggactcgatctctggaccgcactatcgttgcctcagcccctaggtcgtgctgccctctggcctcctcatcgtacaattcaccaacatctccaatgtaagtgcagcaggttcagtaatgaactcagaagtggcatcagaatactccaagagttttttgatctttttgcctggatatataccaagggaaatgcattcaaaactcctatagatgacgaatcccatctctccctcttttctcggacacggatccccaggtccgtctccgtgctttactcatttgttttttacaagttcagatccacttgcgtactcacacggtggacatctgttatgcacatgtgtaaaccagcataagtccttacactcgaaaatgcatgtgttatttagcttgagaataaataaaattattagcaaggagaaaacaaaaaaataggactaaacaatagagtcacattggtttaaattagtacctagaagtaaaaaaagatgatctaaattagatacatcataccaaataccatattactattccagttaccccgtctactatgcctagatatcaaattcttgaaggttggccttctcattttcagtaatagcctgacgaaagtagagtatgtttgtatgagcaattatgctgctcactactgccttgcgctataataggccactactgattttacatgctttttctacattagatagctcacaaacatgctacctcaaaaaaatgatggcaaaggggagccacaaaatgtcaattattttgtcaagtattagcagttttcttgtgtatgtgatcagactaacactgcatgtctttgttttcctgtaaaactatgtatgatgaaaccatggtgtgattgtattggctggccttaccctgttttgttgcaatgcattcgttgttgtacaggtaatatgttgaaacacaattcattgcatatgacaattctgttttttctttctagaatattgacatattgtttgatcattattttctaagcaataatcatggctattcttatagtattgcataatacctttttcttttcgaaccctagcgcattgattctttagtgaagtgattatagtgattccagcgggagagtagggtggggagcagagggttgattctggactgatttcggtggagattaaatggggagcagtgaggagcatgtttttttagatcccaccagaatatgtgcgccattttgctatttggctgaggagtgatgctcagggagaatccgttctcaggagctgtgccaaatgtcgccttaggttttatgatatgacctgacttctgtgttaatatttgttagatctttattttatttgaggttacaaaggtggtgttctcaagctagaaacaaagttgtggctaggtcaaaactagatgatgctcttgaaccgtgtcttttgactctgttacttgttgcaggtttgatgttcactaatatgttgttcaactttgagcaggtcagcaattgactggtgttgctggtagcctggcatatctggcacctgaggttctactaggaaattactcccaaaaggtagatgtatgggctgccggggtgcttctgcatgttctgttgatgggcactcttccgttccaaggaaaatctatcgaagctatctttgatgttataaagactgctgaacttgactttcacaatagtcagtgggcatctgtgtcacttcttgcttatgatctcattggtcgaatgcttaatcgagaggtctcttcaaggcccgatgccgaagatgttctccgtaagttcaagcacccttgtaacttgtgctttatatatatatataatatatatatatatatgattctcaatttatcattgacttttcctaatggctttcaacacagggcacccatgggtcttattctacactgattgcctgcagaaagctgaattctctaacctatgggatactaacaaaactgcagctcccatgattcatcgggagatagtcaggtttggttactgcgagtcttcatcttcaaaatcctcaagtgacaactctgaagagcgagatgaatgcggtatagttgatgcactggcgacaacaataacacaggtgaggatctcagagcccaagaggagtcggctgttcagcctacccaacgggttgttgccgccaagcaggaacagtctccgaacatgaagatgatgaatccgtgtgtggctttctaacttgacctacctagctcccatccccatgcatgtataaacgagataaacgagctctgtgattttatagatggaaaattttcaccgtggttgatgttttgcgattgctagctcgctgagcctgcaatcctctgtaaatatatcattgttgtcatcatttttgtacatcgatgacaccgtaattgattcgatt

SEQ ID NO: 2 - DNA, 1524 bp, Artificial Sequence
  cDNA
atggggagcagtgaggagcatgtttttttagatcccaccagaatatgtgcatccgtgtcacttcttgctcatgatctcattggccgaatgcttaatcgagaggtctcttcaaggcccaatgccaaagaagttctccctcccatgattcatcgggagatagtcaggtttggttactgtgagtcttcatcttcaaaatcctcaagtgacaactctgaagagcgagatgaatgcggtatagttgatgcactggtgacaacaataacacagattcggaagatggacttggaggcaaggagcctacagcctagcattaaggctggtttgcttgcaaagctgagggagtataaatctgacctcaacaacgtcaagatgggtctatccgcagagaggaagaagcagaagctctccgagatccaatccggcgttgaggaagctgaatcgctgattcagaaaatggacctggaggcaaggagcctacagcctagcattaaggctggtttgcttgcaaagccgagggattataaatctgacctcaacaacgtcaagagtgagctcaagaggatatctgcgcccaatgccagtggcctgattagctacaagaagctcttgttccatggactcgatctctggaccgcactatcgttgcctcagcccctaggtcgtgctgccctctggcctcctcatcgtacaattcaccaacatctccaatgtcagcaattgactggtgttgctggtagcctggcatatctggcacctgaggttctactaggaaattactcccaaaaggtagatgtatgggctgccggggtgcttctgcatgttctgttgatgggcactcttccgttccaaggaaaatctatcgaagctatctttgatgttataaagactgctgaacttgactttcacaatagtcagtgggcatctgtgtcacttcttgcttatgatctcattggtcgaatgcttaatcgagaggtctcttcaaggcccgatgccgaagatgttctccggcacccatgggtcttattctacactgattgcctgcagaaagctgaattctctaacctatgggatactaacaaaactgcagctcccatgattcatcgggagatagtcaggtttggttactgcgagtcttcatcttcaaaatcctcaagtgacaactctgaagagcgagatgaatgcggtatagttgatgcactggcgacaacaataacacaggtgaggatctcagagcccaagaggagtcggctgttcagcctacccaacgggttgttgccgccaagcaggaacagtctccgaacatgaagatgatgaatccgtgtgtggctttctaacttgacctacctagctcccatccccatgcatgtataaacgagataaacgagctctgtgattttatagatggaaaattttcaccgtggttgatgttttgcgattgctagctcgctgagcctgcaatcctctgtaaatatatcattgttgtcatcatttttgtacatcgatgacaccgtaattgattcgatt

SEQ ID NO: 3 - DNA, 1082 bp, Artificial Sequence
  cDNA
cctgcccttccattcttcccccgctgcccccggtcaacgtcacgaacccgggcctcgtgccgctcgtcgtggccacactgttcgacgagcgagtcacagagctgctgagcgtgctcgctgatgcggcggtggggcgaccaggcaggtggtccatcggcgaagcgccatggtcgtcgtcggggggcacgaaccaggcggtgtacgcgcgccgcgcgcccggctcttcatcgcctccacccgctccagcgtctccaccacttccttcatcgagggccgactgcttggctcgctggccaggcagccgagcattagttgcgccgcttggaacgcctgcttttgttgatcgtttgttttggtctgatttcagtgggtctatccgcagagaggaagaagcagaagctctccgagatccaatccggcgttgaggaagctgaatcgctgattcagaaaatggacctggaggcaaggagcctacagcctagcattaaggctggtttgcttgcaaagccgagggattataaatctgacctcaacaacgtcaagagtgagctcaagaggatatctgcgcccaatgccagattcggaagatggacctggaagcaaggagcctacaacctagcattaagagtgagctcaagaggatatctgcgcccattgccaggcaggctacccgggaggagctcctggagtctggaatggctgatactctcgcagtgagctaatgctaggacttgactgtgtctacgagactgctcctaacaataaactgaagaaagcaaaagaaatcattcaacgtattcgccgaagagaactctacaagatatggtagtcctgggaggaagagccatcgccgctatgtatggcagaaccacccgcgaaagcaacctctctggtctcgcgtagccagagcaggagcagctcgcttgcgcggtcgcggcgctggcggccggccccgcgtacgagcgcctgcaggaagccaggaacccatccgaacaaggttgcaatcatgataagcagatagagcaagcatatgatgatattttgaattcgtcgaagcatactttggccagcatgatggagct

SEQ ID NO: 4 - DNA, 2321 bp, Artificial Sequence
  cDNA
tgaggagcatgtttttttagatcccaccagaatatgtgcatccgtgtcacttcttgctcatgatctcattggccgaatgcttaatcgagaggtctcttcaaggcccaatgccaaagaagttctccgtaagttcaagcacccttgtaacttgtgctttatatatatgattctcaatttatcattgacttttcctaatggctttcaacacagggcaccatgggtcttattctacactgattgcccgcagaaagctgaattctctaacatatgggatactaacaaaactgcagctcccatgattcatcgggagatagtcaggtttggttactgtgagtcttcatcttcaaaatcctcaagtgacaactctgaagagcgagatgaatgcggtatagttgatgcactggtgacaacaataacacaggtgaggatctcagagcccaagaggagtcggctgttcagcctacccaacgggttgttgccgccaagcaggaacagtctccgaacatgaagatgatgaatccgtgtgtggctttctaacttgacctacctagctcccatccccatgcatgtataaacgacatttggggaatgggtagaaaagcagagattagggattttcgtttccgtcggtgcagttttggtgttccaatggagttgcgagatgtttatgtgccttagtcttcaatttgggggttgggggaaaagtaattttatgtttttgttttgtgtctgcagattcggaagatggacttggaggcaaggagcctacagcctagcattaaggctggtttgcttgcaaagctgagggagtataaatctgacctcaacaacgtcaagagtgagctcaagaggatatttgcgcccaatgccaggcaggctacccgggaggagctcctagagtttggaatggctgatactctcgctgtgagctaatgctaggacttgactgtgtctacgagactgctcctaacaataaactgaagaaagcaaaagaaatcattcaacgtattcgccgaagagaactctacaaggtagtatgatgctttaattgctcatatacaagtgtcattttgtcatgtcattacacatggttaggatacatacttaagtttctaacgtaggcgtccacacaacggattggtgcacggttctgccgatgtatcccacgcacgtgcatggaaggaggcaggcacccttccccgccgccccggatctcgcgccagcccccgccctaccccgcctgcccttccattcttcccccgctgcccccggtcaacgtcacgaacccgggcctcgtgccgctcgtcgtggccacactgttcgacgagcgagtcacagagctgctgagcgtgctcgctgatgcggcggtggggcgaccaggcaggtggtccatcggcgaagcgccatggtcgtcgtcggggggcacgaaccaggcggtgtacgcgcgccgcgcgcccggctcttcatcgcctccacccgctccagcgtctccaccacttccttcatcgagggccgactgcttggctcgctggccaggcagccgagcattagttgcgccgcttggaacgcctgcttttgttgatcgtttgttttggtctgatttcagtgggtctatccgcagagaggaagaagcagaagctctccgagatccaatccggcgttgaggaagctgaatcgctgattcagaaaatggacctggaggcaaggagcctacagcctagcattaaggctggtttgcttgcaaagccgagggattataaatctgacctcaacaacgtcaagagtgagctcaagaggatatctgcgcccaatgccagattcggaagatggacctggaagcaaggagcctacaacctagcattaagagtgagctcaagaggatatctgcgcccattgccaggcaggctacccgggaggagctcctggagtctggaatggctgatactctcgcagtgagctaatgctaggacttgactgtgtctacgagactgctcctaacaataaactgaagaaagcaaaagaaatcattcaacgtattcgccgaagagaactctacaagatatggtagtcctgggaggaagagccatcgccgctatgtatggcagaaccacccgcgaaagcaacctctctggtctcgcgtagccagagcaggagcagctcgcttgcgcggtcgcggcgctggcggccggccccgcgtacgagcgcctgcaggaagccaggaacccatccgaacaaggttgcaatcatgataagcagatagagcaagcatatgatgatattttgaattcgtcgaagcatactttggccagcatgatggagct

SEQ ID NO: 5 - DNA, 1082 bp, Artificial Sequence; identical to SEQ ID NO: 3
  cDNA

SEQ ID NO: 6 - DNA, 3646 bp, Zea mays
atggcacactttgatgaactagaggataaaacaacagattatgttgatttatcggttcaagaatttgctcttaagcaacctcaatgtggcatggcttataattactatggaaatttaaggctttatgtagtagccaataaagctgaattggcctcttcaatatttgaaatcgataaggtaaacaaaggcggagttaatgcatctatgccagtgaccacttccactcctaattcgaatcaaaattcatgaaccggttatggaacaaatagagaatcaagtttcggtgaggtataatacgattcccctaacccatggaatttacctagtaaaaatcctgtagttaatagtgtactagtaacttctgtcaccgacttgaataaagctttgaatgagtataaaaatgagatgtctaaatttattgagaatagcttggtgtatagattaagcctagtagaaacacttataacaagttgtatgcttcaattttttttgatttttttggaagctactcatagttggagggtaccaaatttacaaaaaaaaattggtgattataatagtaaatctaccatagaacatgttagcttgtttcttgctctgagaggtgaagctagtagcatgaaaattgaatgtgcgttatttttctttttcacttactggtacaatttttgcatggtttatgttgttgccctgcttgttgtattggttcatgggctggtctgtgaaataatttggcgatagccattttcttttttgagatacattgcttttgctatatatatctagatatggtgcatatttaaatgcataataaaaatgtaaaaatctaaaacgtcttataatttaggacagatgaaagtactagatattagacatttttagtgtttttattaaaatggaatatgtaccgcctttgatgctacaacttttacttagcttttaaaacacaccattctaaattgtaaaaaaatattaaaaatgtgttttgcaagatgaatatactaacctttgttatgataatagttttcatatgttaatggaacaagctaaaaagtttggcaaagtatagtcctatagcttccatttcgactcagagagagtatgttgtatccactaaccgtgtacacaagatagcccaactaattaattattttgtgagctatcacccaaccttctgtttatcatggattcatggaaaaatgtaattgccatcattacactaaaaactaaaacttatgaaggagaaccattgtcttgctatatatgagatgacaaaattttccaaagaagagagaagccggcagaacccatcctgtttcaaatctcttctactacttaagtttctaacgtaggcgtccacaaaacggattggtgcacggttctgccgatgtctcccacacacgcgcatggaaggaggcaggcacccttccccgccgccccggatctcgcgccagccccagccctaccccgcctgcccttccattcttccccagccgccccccggtcaacgtcacgaacccgggcctcgtgccgttcgccgtggccacgcggttcgacgagcgggtcacggagctgctgagcgcgctcgctgacgcggcggcggggcgaccaggcaggtgggccatcggcgaagcgccatggtcgtcgtcggggggcaggaaccaggcggtgtacgcgcgccgcgcgcccggctcttcatcgcctccacccgctccagcgtctccaccacctccttcatcgagggccgactgcgaggctcgccggccaggcagccgagcgtcagttgcgccgcttggaacgcctgcttttgttgatcgtttgttttggtctgatttcggtgggtctatccgcagagaggaagaagcagaagctctccgagatccaatccggcgttgaggaagctgaatcgctggtaaatagatgccgcgacacgttctggtttggggatccccttggctaacaggacatacgacatttggggaatgggtagaaaagcagagattagggatttttcgtttccgtcggtgcagttttggtgttccaacggagttgcgagatgtttatgtgccttagtcttcaatttgggggttgggggaaaagtaattttatgtttttgttttgtgtctgcagattcagaaaatggacctggaggcaaggagcctacagcctagcattaaggctagtttgcttgcaaagctgagggagtataaatctgacctcaacaacgtcaagagtgagctcaagaggatatctgcgcccaatgccaggcaggctacccgggaggagctcctggagtctggaatggctgatactctcgcagtgagctaatgataggacttgactgtgtctacgagactgctcctaacaataaactgaagaaagcaaaagaaatcattcaacgtattcgccgaagagaactctacaaggtagtatgatgctttaattgctcatatacaagtgtcattttgtcatgtcattacacatggttaggatacataggagattctgttttttaacacatagttgtcccatgtccatgaattcatttgaattaatttactcttcgcaatcttatacattaaaatcgtgttacctattacatcacaacttcatgagagcatgcttgttctgtgtagatatggtagtcctgggaggaagagccatcgccgctatgtatggcagaaccacccgcgaaagcaacctctctggtctcgcatagccagagcaggagcagctcgcttgcgcggccgcagcgctggcggtcggccccgcgtacgagcgcctgcaggtaggccagcttctgctgcaatgcccgaatctcggcgtccacgcgcagcagcgtcgtcgcctcctcctccgtcagctcacccagcttggccagcacccccgtcacccccgcgtccgccatggctgtcgccgggaccgaaaggctaaaactgtcacaatgacgtaaagtttggttggtgttggcggctcacgcaaaaccagacctttccaagttttactttagcggagtttttttggaacgagagcaaagcagcacagtttcaagaatgtggggcaatttgaatgttcgttcctgctgcactgctactgcttttagaattgtagtatgcttcatcatttatttatttctaaaaaaacttgcatgaattctatcgtgacttttattgagaaaataatgtattcacgtatcttcatgtttctgataaaggtatttgtatatgcatcggtgctacatatgcgaatacaagttttgtttcaactctgaagtctcaagttgaattctaaactccagtttgttttctactgtgctgctgcaggaagccaggaacccatccgaacaaggttgcaatcatgataagcagatagagcaagcatatgatgatattttgaattcgtcgaagcatactttggccagcatgatggagctgcaggaggttcagttatttgcacacattgtttttctttcactcctatgattttcctcaatatgatcaaaatgtttcttttgcaaataatgattgaaatgtttctcattgtactcaacctcttaaactacctataggctttgcttgagagtaatcaggctacaaaggatgccaatggtattgctgctctctatattgttcttgttctaatgtaa

SEQ ID NO: 7 - DNA, 3646 bp, Artificial Sequence; identical to SEQ ID NO: 6
  cDNA

SEQ ID NO: 8 - DNA, 10605 bp, Zea mays
aggaatcttaaacatgtggaacaggtgctcaacacatttagcaactagttgttgatgacccataactttgcagccttcataatgcacacaattgatgcatcaattgcatacctcctgtctttgtcaacattttcaacaccttttttcttctcatcaacaggaggcgatggaatccaaaaagagtgacaacaaaaatattagtataataactaaactctaagtctaccaaacagtgaaagaatagtgaaacaggaaataccttaattcttatcattatgttaataaatttaaaattgaactaaaaaacatcattaggtgagatggatctatttgtcggttccctgttaaggatcttgtatttcacacaagaaagtgaatggagcaaacacacactacatcatctgacatgtttagttgtgttgcaatttcaaaatatctaagcctgtcggatccattgaacaatagtagtaatgtggcatgtcaaaaaatgtcaaacatgttaatatagcaccattttttgtgatgcagaaatgacccgagattacctgatatgtcataacaacgagctcaatagggttagcatcaaacttcgcacttacgttgcaggttcccatccatgtcagcttcatgtgcttcgttcttgtttgatggaactccttgaaaacatctacacatttcagtgcctcatgagactcgccatagcgagcggggtggaggatggtgacaatttcggcagcctcgccgggggcagcactgcgacgagcgaggcgggaggggtggcaatctcgtgggggaggggccaggcacgaccgtccaaccacggcgggcggagacacggtatccatgtgagatatagccacctcatctagccttatctccaagattttaaatcactgatcatcataagcgatcagatggaggccagttcacatcgaccgacaggactgatactaacaggaccatccacacttgcacatactataaagattaataagagattacataagaactaagtagtgaatcagacacccattgctgaccttgttaatcagcccatcgccaatgaaggtgctgctgatcttcttgaacaacctgtacaatgcctcgaccttgttcacgctgactgcaagaatgacaagcagaggaaacccaaccaggcaggaaaatgatgaccaacactgaatagaaaaagtaaatgaacacctccagctatcaaaattttaaagcaatgtgaagtcctcaaagaaccaggacaacactcatgattttttataactaagggaattgtttatcatcaattcattctaaaatacaagacaatcaaaagaactaagcaaagcatgagatacaaaaattcaaagcacatgtatagtgtcttggtaaaaaatttacaagatggtgaatgaattcaactcaggttgtctacttcagcattagtttgcactgtccagaaaaagaacaacagcaagattggaataatgctatggccaccagaataaaaggtcagagctgtcttttaatgctaatattgttcatgccaaacatttctttgttagcttgtgaatttatacttggacactggactgggccttgatcgacgctggcaatatcatgctgaactctgaaggcaccaaaactgttagctccttccctcgtcaatttgtcaattcaacatgtctgcttcaaaatggttatgcgtaggttgaagaaaagttgggagtttacaaaataatacaatgggatgcctgttctatcatctaacttaagccatgtatcaaggttgcaagttacataaaatacgcttatattctgatggttggaaccacacattctacacgtttcccaaaacaatgaaaaaggtagttgtcgaaagatttaagcatctaaagtgtccactctctctgagagcatcaaaataaagtagtacgtcttatgttttaaactatttattgaagtaccaaactatacggctactaaagatttatttagatgagtaaacgaaataatttatggtatataaattaagaaggggtgattagtcatgaaaaataaaatgtcacaattaccagcagcacgtgattttctaaataatttaagcatgtgcggtgctcttccagataaaacttaggggacgaccacctagttcattgaaagaggggaataaaccaagctccaactttcaagcttgtcaaggcttgtcattattaatttaaacaggacagccaattctcagacatgatgttccaaactgctaatgaatatataatgctcaaaataaacaactaggttcttaactgtcaattacacccacaagatgcacataattagaaaaggtaaaagagaaggcaaatggaataccaggaattatatgactactaaatcatttatttagataagtagatgaaataatttatggtacataatataagaacgggtgattagttatgagaaataaaaggtcaccattaccagcagcatgtgttgttctaaataatttaagcctgtgtggtattctttgagataaaacataggagacgaccacctaattcattggaagaggggaacagacgaagctccaaccttcgagcttgtcaaggcttggcattattaatttaaacaggacagacaatgctcaatctgaactgccattgtatctacaatactcaaaataaacaactagattctgaacaaccagattatttgtactcattccatgtctcataaacaaggaaaaaataacaaccagattatttgtactcattccatgtctcataaactttgggcaccatccatccaacacatccaatctaaacacaccaaacgatggggaatggaaagagcagtattcgattcaacaatggcaaacaaatatcactgaattagaccaagaataaacctaattagacaacgacctcccaaccatcattcgtcaggctgtaaagaagataaagctgccatggggcatggatcaagcagaacaccagagatgaatccaaacacacagaaaatcacgcgcgctgtctacaatgacaacaagccccacatttcattgcagtacactgggctacaaaggcacgtacaacaaagagctagggaaacattgcggagggcacgagagagcagctaacttgacaatatagcagactgagcttgcactgttagcaggcgaggaagggaatcatggggacggagaatggggtccatgcccgcgaaggagaaggcggacgccgccacggtggcaccggcgcacgcgcacacagggaacccgcacaggcagccatggatgctgcctcgccattgcgccggtcgtctctgccacgctcctctctctctcccgctgcatcgccgtggatggggcaagcagagagcagggactgcgacgatctgggcggaggactcgccttggagagcgcggacgcagacgggattctagggagagagcgaagacggggcgcgcgcggcgctcgcgcggcgtggtggcggcgagattagcgggggtggggggagggcggagccgtggtgagggtgtggacgccctccttaccctcttaagtagtagtagagatataatccgttccaaaatatccatccgttcaatttatatttcgtttgatctttttaccctaaatttgattgactcatcttattaaaaaagttcataactattattaatctttattgagatatcatttagcatataatatactttaagtgtggttttagattttttttaaaaaaaaaaattcgcaaaaattaaatgaaacgacccaatcaaacttgaaaagtaaaactaattataaatttgaacggaaggagtaagaggatgtttgaatgtactagagctaatagttggttgctttaaaatttgctagtagaattagctagctaataaatatctagataactattagctaatttgctaaaacagctaatagttgaactattagctagattgtttggatgtattcggctaattttaatggctaactattagctatagtacaatattcaaacacctcctaattaaaatggacaaatatctcttcttttggtcccttgcgttagatttttcatatctccttatttagtataaaagaatcatcaaaaagtggacaacccctagtggaacaccattttagtagtggttgcatgaaacctttcgcgcaccagtttctatgtgtcactctaaaaatgggacagcatgtacgtagtgcctatatatatacaagtcatctatcgttgcctcctcagttcatcactaatcacacttattgtgccctcgacgagtatctatagctagctcattaatcgattcgggggtgtgttgtcgaaggcggcaatggcgagctactcgtcgcggcgtccatgcaatacctgtagcacgaaggcgatggccgggagcgtggtcggcgagcccgtcgtgctggggcagagggtgacggtgctgacggtggacggcggcggcgtccggggtctcatcccgggaaccatcctcgccttcctggaggccaggctgcaggagctggacggaccggaggcgaggctggcggactacttcgactacatcgccggaaccagcaccggcggtctcatcaccgccatgctcaccgcgcccggcaaggacaagcggcctctctacgctgccaaggacatcaaccacttttacatgcagaactgcccgcgcatctttcctcagaagtgagtccgatgctgccgccattgttcttgcatccatccagcatcgtacgtacgtcctctatacatctgcggatcatcatgtgcgcatgtttgtggcatgcatgcatgcatgtgagcaggagcaggcttgcggccgccatgtccgcgctgaggaagccaaagtacaacggcaagtgcatgcgcagcctgattaggagcatcctcggcgagacgagggtaagcgagacgctgaccaacgtcatcatccctgccttcgacatcaggctgctgcagcctatcatcttctctacctacgacgtacgtacgtcgtcacgaatgattcatctgtacgtcgtcgcatgcgaatggctgcctacgtacgccgtgcgctaacatactcagctctttcctatctgctgcgccaatttgcaggccaagagcacgcctctgaagaacgctctgctctcggacgtgtgcattggcacgtccgccgcgccgacctacctcccggcgcactacttccagactgaagacgccaacggcaaggagcgcgaatacaacctcatcgacggcggtgtggcggccaacaacccggtaactgactagctaactggaaaacggacgcacagactccatgtccatggcggcccacaaggtcgatgctaattgttgcttatgtatgtcgcccgattgcacatgcgtagacgatggttgcgatgacgcagatcaccaaaaagatgcttgccagcaaggacaaggccgaggagctgtacccagtgaagccgtcgaactgccgcaggttcctggtgctgtccatcgggacggggtcgacgtccgagcagggcctctacacggcgcggcagtgctcccggtggggtatctgccggtggctccgcaacaacggcatggcccccatcatcgacatcttcatggcggccagctcggacctggtggacatccacgtcgccgcgatgttccagtcgctccacagcgacggcgactacctgcgcatccaggacaactcgctccgtggcgccgcggccaccgtggacgcggcgacgccggagaacatgcggacgctcgtcgggatcggggagcggatgctggcacagagggtgtccagggtcaacgtggagacagggaggtacgaaccggtgactggcgaaggaagcaatgccgatgccctcggtgggctcgctaggcagctctccgaggagaggagaacaaggctcgcgcgccgcgtctctgccatcaacccaagaggctctagatgtgcgtcgtacgatatctaagacaagtggctttactgtcagtcacatgcttgtaaataagtagactttattttaataaaacataaaaatatatatatgttcttgaatataaaattgataaccaaattaaaattcgaaccatcacttatacataattttactttattttttataaaacgtgaacgggaaggactaccgtgaatgactatagaaccaatcatactagtataaaatatatgatgacactacgggagagacaaactttgtctggcgctaaatattttgccgagtgtgaattcacgggcactaggcaaagatcttctttgccgagtgttacgctgggcaaagtaagacactaggtaaatcagtcatttgccgagtgtccgccactaggcaaagcaaaacactggcaaatcaaaagtttacctagtgccagacactaggcaaaaaaaaaacgctcggcaaatcggaagtttccctagtgccagacactagacaaagaaaaacacttgataaactagcgtcgtcagctaacaccatccaccaaccgttaacgttgccgagtatctgacttcgacactcggcaaagaaggtctctttgcctagtgtcggtctggaacactaggcaaagaggcactttacctagtgtcgtattttgacactcagtaaaataattttttttctttctgcttccaaactttttatgatgtgttcctatagcacctagaactacatgtcaagttttggtaaaatttttgaagtttttgctatatttacttaatttattttatttaattgaatttcttttgataattcaaatttgaactcggcaaggtaagaagcgagggtagcctggaaacacactttgcctagtgttacactcggtacaggagcctcccctgcctagtgctgcactcgacaaaagattcgcctttgcctagcgctgcactcggcacaggagtcgcctttgcctagtgctgcactaggcaaagcctccgttaccgtgccttccatcgtcatggaaacttttcttcgccgagtgacgtgtggcactaggcaaagtttttgccgagtgcccgagaaatggcactcggcaaggactctttgccgatcccttcgttgccgacttctttttgccgagtgcaacactaggcaaaccatttgccgagtgtaaaagaggctttgcctagtgtctgtggcactaggcaaagaagacgagtcctgtagtgaacctagtaggccagtgcgggaccattccaaaaaatacctataaaaataaatttaatattaaattaaacatatggtccacgtaccaagatattaaactcaaaagaacaattattacaatttatcttagctaaaaggccgagaaaaagtatatgttaaaaaggagtgtgatcccatttttatagctcgctcggtcgatcgcccgtccacttttaggtaacgaggtggtaccatgtaggagtgttgcgttgcgtgcgacttcctatcatgttgggcttaggtggcttctcacgacccaatgataggcgagaagtgtggaagatgaacaaacctacttgtttcgtgcacgacgcatgtgtttgaacaacgagttagattagaaaaaaaatataatgacttttttttttgcaaaagtgaggataatgaaaaccagaaaaactggtgcttcataagagtagagatttgatggtaaatatagtagtaatgcaatggctatactacacgcgagagtccaatggcaagccggtgtgttggggcgaaggcgaagacgctacccttcgctccaggcctttgtcaactcgctgcaccaacagaggcaagatgaccggcgcggcccacccttcgtcctcttcactgcaagacgaaggcctacgacgaagtctctccatcccacgtcctcgccttacctggaggcccacgtgggattcggcccatcgtaacaggccccgcacggacaggcgtgttacgggtttgatttgtaatagcttttctgtaatgacagtttgtaaccctcccttatgggaatattctggggataatccaggtgtctgagggcataagcgtccttacatcgggacgttgggcgctcgggcacctataaatacccccgtacagtgcccttgagaggctggattaacatagcaattgccatctcgagttaaaccttgcttgcatcctttccactctcccgttggatcaacttgcccaagagagctagttccaacatttggcgcccaccgttcgtgctacgagcaaaccacccgcgatggcacccaaaagagctagttcgaaggcagccccatccgtcgacgaagcggcgaaggcagcactgctagctgagaaaaagggcaaggccctcgcagacaacacccaccaagaagctggcgaagacgaagcactcagtaagagacagcgcaacgatcaacacactctcgaaggcaccctccgcacctacagctccggaggccaaccacaagtaccacccctaggcttcgctccactagagggcgaggacacaacagaggacggcgaagtcatcggcgtctcagcagaagaacaactacagttatgggccctgcgcctcaagaaccgcaacctccaaaagcagaaagaaatcctcgaagccaagcgccaacgcgtctccgcgcaagccaaagtgcgttagatgatacgagacgaggagcagagggcccgggaactagagcaagagattgcgctcatgcagagcgaaggacagcatgatctacagcatggcccacccctccagcagcgcgcgccagctagagatttattcattccccagcgcgggcccttcatcccacacgccgcagctttccaaggcatcaactaccttgatgagcgaagccccctggcgccgcaactccaagtgtcaccttggcccgccaacttcagggcagggagctaccccaagtacaatggcagcaccgacccagcacaatacatcatgagctatcaagtcgctgtcgcatcatccggaggggacgacgccacaatggccaagtccttcatcatcgccctcgaaggtccggccttgacctggtacaccaggttgcccccactgtccatcgactcctggcgaagtctccgggacaagtttctgcttaactttcaagggtaccgcccagacatcgatgccttggccaagctgtcactctacaaacaacaagagaaagaaaccctacgggagtactaccgcaagttcctggctctcaagtcgcaactgccctcggtcgacgaccaaatcgccatacactacgccatcagtggccttcgggctggcgtcctatacagtcactgcatcaggtacccacccaaaaacctccaagagctctatcagttgtttgaaaagtacgccagatccgaagagctccatcagcgcaaggtcgagtctcaaagaaagcccaaggaccctccgcagtctagccaaacatggacaagaccttcacagtcagactccggtcgggacaaccgcagtcagcagcaggtgcataacattgccaaccagcaccccgccagcgaagcccctcgccgccaagattatccccccagggccgcggcaatggcacgcgtggtcggggctggggacgggcgcaacagccgtgcagatattactgcctgttttcacggcgaagactgcacgcacccaaccaaggattgtccggaaacgaaggccaccagggacaggatgtctcgggcacaacccgccgacaacccaagagttgtcgcgcacacataccaacaccaccacccacaaccatacaaccacggccccgcccagcatctacccaaccacgcatatcaacaccaccaggagttacaagtcataccacctccacccccgcctccgcatcaaccaaacatccaccaccaaaatcaccccaagcaccaaaacaggaagacttcgctgatcagccgtatcgcggagtcattcacatgatcaccggaggggtccagcattgactttgacacgaagcgacaaaagaggaatcactaccgaagcatcaaccacgtcgccatcaccggctcggtcgtgcaaacgaagtggtcacatgtgccgctaaccttcgacgccagagatgttgatctgcgcagcgcaccccacattgatgccatggtaatcaactgcagtgtggcaggctgggacctgcacaaagtcctagttgacaacggcagccaggcggacatcatcttcctccatgccttcgaccgcatgggcatcagccacagccctctcaagccttcgaacaatcccctatatggcttcggcggcaagggcaccttccctgtgggcaagatagagctacccctatccttcggcgtagcacccaatgcgcgaagcgaataggtcacctttgacatcattgacatggtctatccctacaacgccataatgggtcggggctctatcaacaaatttgaagcggcaatccacggattatacctctgcatgaaaattccgggtccacaatgcgtaataacggtgtacgggaaccagcagactgcgcataacattgagagagatttcgttcccgatcaacggaacgtacactgccttacgacgcagcgcgaagtccccgaggctacctgcctagctgccaacaaaaatgaaaaggcacagctaaaaagcaac

SEQ ID NO: 9 - DNA, 11001 bp, Zea mays
aaatggccgaagctattttggatgaagccatctctcgactattaaacgaagctgcggaagcagttttaaaagaagaatagttgttattgtaaaaacatttggaatgtaatatttgctgaacaaagtgtgtaatatttttataatttgaatgtaatatataagctgctcgtaactcaattctttacgatgcatgaaactttacgtacataccgtttttgagccttcggcgaaaaaacaccttcccttcttttcatgcttcgtgaagaatatccatacttcgtaaaaacattatgcttcataagcaatagatctctttttcatattagagttgatgaagttgtacttgttcaaaacttattgtgccttggcactgcttcttcgaaacaatctcgaagatcaacattgtatccccttcttgtgttattgatgcaatatgatgttatgctatgcaaaatgatgtgatgatgttatgctatgcaaaatgatatttatgtcgaagatacataaacattcccacagtagagcacacaatctttttgccgtttatttttcggcttcaccgcttatttttcggtgtatcagcgctgacttttcgctgtaagcctcccttaggtgcttcttcgccttttacttcggcggtatttgcgttgactttttgcgcttcgccttatacttcggtggaatcagcgtttatttctcgctgtaagctctgcattccctttggaacgacttttgagcagaaaacttacgctgcgctcccttagaaatgactttttgtaacttcggcaaacttacgctgcgtttcatagaacgacttttttgtagtttcggagatactttctgtagccacaagttcttaagaacgagttttcatgcttcatcaactttttgaattccgtaagtctgtggagaagatatattttcactatgacaaaaacaaagctgttacaagaaattgaaaacaacaagaaaaacttaggctttcaatgattgttctttattaaaaagaaaaatgataactaatgcaagaactatttcagaagtaggatatctgttagtagatgtgctttgactctggcacaatactgttgactgtgcgagcttcggactcctctctgaagtctcgttgctgatgagtgtgctggctcccttctggctgctggcctcgttgtattggtggtggaggtggaagctgttgccaagatgcctgaggttggcttgccgaagcaacagaagctgcaggatggttacccttacccacatactctggaatgtacggtgagtggtacgaagcagtatgcataacttgcttcggctggctctgttgggctgcagtttctgctatctctttctgtttctggatggtgacatggcacatcctggtagtatggcccttgtcctcaccgcagaatagacaataaattttcctgggctgatccccaaaccttcctccgaagcccctggctcctctgccccttggggctggaggccgaggataactctgttgctgccccgaagcctaggaggaatattgcggcctctgttgctgacttcccctgtcgtcattctgagtggaatgaattgatctgacatgtctagggtgtactctccctccgaagcccctggtcatctcggagaatctgtaagaaggcccccaacacctctctttcccattcgtttaggtgagaaaacacattggggagcactagggagttctttcctagtgaggcgtctgtgatttgataatcacaagattaaggatttcattagtgcatgtgtagtagcaagtgtgcatccaccttcctcattaagcttgtttaggataagccagagtttgtgccggttactcttgatgttcaacaacaccaagatggcttggtggtaattaagagcttggtgatctctcagtggtgctcgtgagagtcccaactcattgtgtaataaaagattataggtgattcaccatgccggagtggtgaataatcaacccgtagagagcattgagtccttgaatggatcgatggggggctacacccttgtgtgggtcaagtcagagttttagcagttcttgcacccatgatctcatcgtgaagcatagataaatttaaattcttttgaattatttatatatgacaacactattcgtcgctctaggtgactatcacctaccctaaaatgacttaacaaatctttattaattgttaagtcattcacatttttgttaatccactccaaagtcagggtgtttagtgtttttacatccatgtctccttagactcacggtgtctctcccagattctctctcaccctcacctctctctcactagccactagggaacgcaacacccatcgatggctcttcgccccatgaaacgttcacacaatcgcaattgtcgaggcatgcatggctgggagagcagacatggaggcatacgtgctagggttgcacatgggcaagagggtgggtgtggctattcagatatgcatggtgagcaagatgggtgaggttgtgggcatgatgaggggataaggaagaataagatctcttttgttaggctgtctccagcagctatcgtatcccattccctatcgcatcccctattttaaactttactatgcaaacaatgtaatatatagtgcagattccctattttacacaatgtgttgtagacaaccttggagctcttgcataaaagctctagttttggctctagctcctctgagaaaacaatccccaccatgtttttaggaagaatccctgaagggcaccccatttggttggaaatacatctcctcctacaggattatgtttgacttttttttgcaatgtgggacccacaggggagaggaggacgagaaggaaccggagagcctattttttgggctcctggcttcgcttggtttctaggggcggctccttcctattttcacaaaggagctagtagaggagcctcccatttcatgattttttgaaggatctatttaaggagccttgaaagagccctaccaaggtaggcctagaaataataaaggaggaaaaagagaaggtatcacaacttttgtctacaacgtgaaaatgtttggctaaatagataaaacagtttgaattttatcgattcaattgtttattgagggcatgtttgggagggctttagttctagcttctttcgcgaaaaatccagagccctacaaaatgacgtttggtaaaacgacttcttccgaaaaacacccaaaaacccaagatattttatactacgaaggaaaggtcacacatcctagttagcttcactggttctagctccttccaattttgcaaaaaagtcacaaaggataagccattttttcaaatgatttgtgaaatgcctacgctaaaaagtctacttttccaaaaaaactagagctagagccgtttttggcaagtcagaaccctaccaaatagtccctcagtttaagcaaagtgaggctatactgaagctaaattatgccaaattgggcctacatctccatattttcaaccaaatgctttagggtttcttgtaatcgacatgatttgtttcttcataaatagtatatggaccgctccaaaatactccatccgtttcaatttatattacgtttgatctttttaccctaaatttgatcgactcgtcttattaaaaaagttcataactattaataatctttactgtgatatcatttagcatataatatactttaagtgtagctttgattttttttttgcaaaaattaaatgaaacgacccaatcaaacttgataaaaaagtaaaactaattataaatttggacataaggagtaggagggtgtttgaatacactagagttaatagttagttgtcttaaaatttgctagtacaattagctagctaacaaatatttaggtaactattagctaatttgctaaaaacagctaatagttgaactattagttgaactattagctagactgtttggatgtattcaactaattttagcagctaactattagttatagtataatattcaaacacctcctaattaaaatggacaaatatctattcccttggtcccttgcgttagattttccatatatcctcatttagtataaaaagaatcatcaaaaagtggacaacccctagtggaacaccattttagtagtggttgcatgaaacctttcgcgcatcagttactatgtgtcactctaaaaatggggcagcatgtacgcagtgcctatatttatacaaggcatctatcgttgcctcctcagttcatcactaatcacacttattgtgccctcgacgagtatctagctagctcattaatcgatcaatcggggtgtgcggtcgaaggcggcaatggcgagctactcgtcgcggcgtccatgcaatacctgtagcacgaaggcgatggccgggagcgtggtcggcgagcccgtcgtgctggggcagagggtgacggtgctgacggtggacggcggcggcgtccggggtctcatcccgggaaccatcctcgccttcctggaggccaggctgcaggagctggacggaccggaggcgaggctggcggactacttcgactacatcgccggaaccagcaccggcggtctcatcaccgccatgctcaccgcgcccggcaaggacaagcggcctctctacgctgccaaggacatcaactacttttacatggagaactgcccgcgcatcttccctcagaagtgagtccgatgctgccgccattgttctcgcatccatccagcatcgtacgtcctctatacatctgcggatgatcatttgcgcatgtttgtggcatgcatgtgagcaggagcaggcttgcggccgccatgtccgcgctgaggaagccaaagtacaacggcaagtgcatgcgcagcctgattaggagcatcctcggcgagacgagggtaagcgagacgctgaccaacgtcatcatccctgccttcgacatcaggctgctgcagcctatcatcttctctacctacgacgtacgtacgtcgtcacgaatgattcatctgtacgtcgtcgcatgcgaatggctgcctacgccgtgcgctaacatactcagctctttccgatctgctgcgccaatttgcaggccaagagcacgcctctgaagaacgcgctgctctcggacgtgtgcattggcacgtccgccgcgccgacctacctcccggcgcactacttccagactgaagacgccaacggcaaggagcgcgaatacaacctcatcgacggcggtgtggcggccaacaacccggtaactgactagctaactgcaaaacgaacgcacagactccatgtccatggcggcccacaaggtcgatgctaattgttgcttatgtatgtcgcccgattgcacatgcgtagacgatggttgcgatgacgcagatcaccaaaaagatgcttgccagcaaggacaaggccgaggagctgtacccagtgaacccgtcgaactgccgcaggttcctggtgctgtccatcgggacggggtcgacgtccgagcagggcctctacacggcgcggcagtgctcccggtggggcatctgccggtggctccgcaacaacggcatggcccccatcatcgacatcttcatggcggccagctcggacctggtggacatccacgtcgccgcgatgttccagtcgctccacagcgacggcgactacctacgcatccaggacaactcgctccgtggcgccgcggcaaccgtggacgcggcgacgccggagaacatgcggacgctcgtcgggatcggggagcggatgctggcacagcgggtgtccagggtcaacgtggagacagggagcgaggtacgaaccggtgaccggagaaggaagcaatgccgatgccctcggtgggctcgctaggcagctctccgaggagaggagaacaaggctcgcgcgccgcgtctctgccatcaaccccagaagctctagatgtgcgccctacgatatctaagacaagtggctttactgtcaatcacatgcttgtaaataagtagactttattttaataaaatataaatatatatatattctgataaccaagattcgaaccctcacttatacacaattttatcttattttttataaaatgagaatggaaaggactaccgtgaacgactatagaaccaatcatactagtttaaaatgctcgtaagctatgacgaacctagtaggccggtgctggaccattccaaaaaacctataaaaataaatttaatattaaattaaacatatggtctatatatcagatattaaactcaaaagaataattattataatttatcttagctaaaaggttgagaaaggtatgcgttaaaaaagagttttaacccatttttatagcttatttgatcgcccgtccacttttagggagcgaggtggtactatgcagaagtgttgcgctgtgtgcgacttactatcatgttgggtttaggtggattctcacgacccaatgatagacgagaagtgtgggagatgaacaaacctacgcatttcgcgtacgacacatgtgtttgaacaacgagttagattggaaaaaatataatgaccttttttgcaaaaatgactacaatgaaaaccaggaaaaccggtgcttcataggagtagagatttgacggtaaattgttacgatctactggtatttgctgcgaggatgtattcgcttggtgaaaacagaattacagagtagcagtagcagggaagacagtagcgagaggagaagaagaaacttgaggaagaagaagataaatgtagttgttacatcctgccttcgccgtaggtctcagcgagcatatatcttcaggtcctccattctgggccctggaatctcacattggccttacgctggcgtgttcctcttctcggcccaactgtagtcttctcttgaggcccaccagtctccacattcctttgttgctgctatagctcctcggacacggctgcttccgcctgctgctgcacctggatgtcttctgaagtcgacttgcgtggagggacagtgctgccattcccctcccgataacacgctgcttgtccccaagcaggcgctcgagggaacctctgacgaagtggaatcaggtcctcccaagttgccagagatggatgcaactcagaccacagaatcaaccgttgtgatgctccattaggcccccatcggcattgtagtactcgttcaggaatttggtggttgtcaaggcgatcaggaagctgtgccaccaccactaaagaacccactgccttcttgagttgtgaaacatggaacacgggatggatagtagaagtaactggaagctccagcctgtaagcaacagatcccaacttagcagcaactggaaatggcccaaaaagcgaaaatctagcttctgatttgcccgaggtgcaagcgatgactgcacataaggctgcataacagccttctcttgcagccactctccgaggataggcacaggagtggaatccaaaatgtcaatgccaaaatgcttgggtgcataaccatatagcacctcaaatggagacattttcaatgctgaatgccaactagaattgtaccaaaattctgccaagtacaaccagtcaatccatttgtgaggacaagcatgcacaaaacatctcaaaaaggtctcaaggcactgattaactctctttgtttgtccatcggattgagggtgataggaagaactcatattcagtgatacaccagccagggtaaacaatgatttccagagctgactagtaaagattttatcgcgatcagagaccatagcagatggcataccatgcaggcgataaatgtgttgcataaaggccttggccaccactgcagctgtgaaggggtgtttaaggggaatgaaatgtccaaacttggagaatttgtcaaccacgacaagaatacaatttttacctccggacacaagcaagccttcaacaaaatccatagtgatcgtttgccaagctcctgaaggcacatgaagaggttggagtaggcctgggtatttcactctctcaggtttagcttgctgacaagtggcacatgctgcaatgaactggatgacagatttcttcatgttcggccaggcaaacaactgcttcagccgatggtaagcgactgctatacccgagtgacccccaacagcagaactatggagagcagacaatatagactgttgaagtgtatgattgttaccaacccaaatacggcctttaaacttaagcaacccttcttgaagagtaaaatgaggaacaacatcttggtcaacaaccaacttagataacaaggtcttagccgaagggtccaacaaatatccatccattaccaaacgagtccactatggtgaacagactgagagagcatgtaatgtgatagcatgttgtcttctcgacaaggcgtcagcaactctattttcatgtccatgcttgtatacaatcttatattgcaaccccaaaagtttagtaaagacttttgctgccatggagtgttaagccattgctcattcaaatgcaccaaactcttttggtcagtataaataacaaactccccatgaagtaagtaagctcgccattgttccaccgcgaccaatatggctaagtactccttctcataggttgataagccttgagtcttaacaccaagaggtttgctgagaacgctaatggatgaccattctgcaaaagtacagctcccaccccattcttgcaagcatcggtctcaatagcaaaaggttggtgaaagttggataatgctaacaccggggctgagatcacagcttgcttcaaggtattgaaggagatttcttgatcttgagtccaaacatagaacacccctttctttcacagtgcatttagaggtttggcaataatagcaaaatgactgacaaatcgcctataataacccgccaaaccaaggaagctccttaactctttaacattggagggcacaggccagttcaacacagcatcaacctttgcaggatcagtatccactccagcagcactgatcacatgacccaagtaagcaatagatgtttgagcaaatttacacttagacttcttgacaaaccagtggtctttttggagaatggtgagaacttgggccaagtgagatacgtgatcgtcaaatgacctgctgtagactaagatgctatcaaagaagactacaacacacttcctcaacaaaagggccaaagaagagttcatagcgccctgaaaggtaccaggtgctcccgacaatccaaaaggcatgactcaaaactcaaattgaccatgatgtgtctagaacgctgttttaaactcttccctaggcttcaacctcacccgatgataccctgaagccaagtccaatgtggtgaaccaacatgcaccatgcaactcatccattaactgttcaaagatggggatggaaaacgggctttgaccgttaaagcattcaaatagcgataatccacacaaaactgaaaagtgccatccttctttctcaccaacagcacaggagaattaaaagatgatgcactgggtctgataatccccgactgaaccatttctgccacctgacgttcaatttcatctttcggagctggtgggtatcgatagggtctgatattaactgggctggcaccagcaaccaatggtatactatgatcacaacttctttctagaggtaaggacataggtttagcaaaaaccgactgaaactggttcaacagctgaacaatttcaggaggaagggtagcctcatcagtcagagcaacagacacttgagatagggaaatctgaaccaacaattcgtcaaccggctctacagtttccccttgcaagagcacttgcacaccatgataagggatcaacatccatcgttgtttccaatgcacttccataggactgaaagtctctaaccaatcaagtcccaatatcacatcaaaggattgtaatggcaacaccttcagatcaaaggaaaacccatacccctaaattgtccattgagcttgagtaaacacttgggagcaagtcataacaccttcattagccactttaacctggagacaagttggtaccaaagtaatgtcggttaacctggaaatcatagtgtgactgataaaagagtgtgaactgcttgaatccacaagaataacgatttcatactcctgtatagaccctctcaacaaaatggatcctttggcccttgatcttgaaacagcctcagcagatagagccaagaagagttgttcctcgtggactgaatcttctgatggagaagactcattcagaaatgcaggcataagatcccagacttcctgcagggcatgaagttgaactgtagtattgcagacatgtcccctatgccatttttcagcacaacggtcacaaagaccacgtgcatgacgataagcacggagtgcagccagtttttcatcagtgcttcgatcagtctgcatgagacgctgcttaggtaaggatctcggcgcactggcacttgctgcagcagtagttggttgaggaagaggcagggtcgtcttgtgctgggatttcgaccaaataccacgatcacccttgcagaattcactccgcataggtggagcagcgacctcatcctgcaaaaaagcgagggaacaggcaatatccagatccatcgacctttgaagcataacaacagcacgcatatcatcgcaaagaccatccacaaaccgtgtaacaaaatataacggatcaaccccagactcatacacagagagttgatctacgagagaagaaaattgttcaatatattgagttaaactacctaactatttgatgcgaaataagtggtgcaacaacagctgatactggtccttaccaaaccgttcgttcatcaattgacacaagagaggccaagacaaacggggatgacgaaacataactgacagaaaccagcacgctactgtaggcgacaagtgcatagaggcaattttgacccatgaattcagatcaacttgatatatatcaaagtaattctt

SEQ ID NO: 10 - DNA, 1284 bp, Artificial Sequence
  cDNA
atggcgagctactcgtcgcggcgtccatgcaatacctgtagcacgaaggcgatggccgggagcgtggtcggcgagcccgtcgtgctggggcagagggtgacggtgctgacggtggacggcggcggcgtccggggtctcatcccgggaaccatcctcgccttcctggaggccaggctgcaggagctggacggaccggaggcgaggctggcggactacttcgactacatcgccggaaccagcaccggcggtctcatcaccgccatgctcaccgcgcccggcaaggacaagcggcctctctacgctgccaaggacatcaaccacttttacatgcagaactgcccgcgcatctttcctcagaagagcaggcttgcggccgccatgtccgcgctgaggaagccaaagtacaacggcaagtgcatgcgcagcctgattaggagcatcctcggcgagacgagggtaagcgagacgctgaccaacgtcatcatccctgccttcgacatcaggctgctgcagcctatcatcttctctacctacgacgccaagagcacgcctctgaagaacgctctgctctcggacgtgtgcattggcacgtccgccgcgccgacctacctcccggcgcactacttccagactgaagacgccaacggcaaggagcgcgaatacaacctcatcgacggcggtgtggcggccaacaacccgacgatggttgcgatgacgcagatcaccaaaaagatgcttgccagcaaggacaaggccgaggagctgtacccagtgaagccgtcgaactgccgcaggttcctggtgctgtccatcgggacggggtcgacgtccgagcagggcctctacacggcgcggcagtgctcccggtggggtatctgccggtggctccgcaacaacggcatggcccccatcatcgacatcttcatggcggccagctcggacctggtggacatccacgtcgccgcgatgttccagtcgctccacagcgacggcgactacctgcgcatccaggacaactcgctccgtggcgccgcggccaccgtggacgcggcgacgccggagaacatgcggacgctcgtcgggatcggggagcggatgctggcacagagggtgtccagggtcaacgtggagacagggaggtacgaaccggtgactggcgaaggaagcaatgccgatgccctcggtgggctcgctaggcagctctccgaggagaggagaacaaggctcgcgcgccgcgtctctgccatcaacccaagaggctctagatgtgcgtcgtacgatatc

SEQ ID NO: 11 - DNA, 1140 bp, Artificial Sequence
  cDNA
atggcgagctactcgtcgcggcgtccatgcaatacctgtagcacgaaggcgatggccgggagcgtggtcggcgagcccgtcgtgctggggcagagggtgacggtgctgacggtggacggcggcggcgtccggggtctcatcccgggaaccatcctcgccttcctggaggccaggctgcaggagctggacggaccggaggcgaggctggcggactacttcgactacatcgccggaaccagcaccggcggtctcatcaccgccatgctcaccgcgcccggcaaggacaagcggcctctctacgctgccaaggacatcaactacttttacatggagaactgcccgcgcatcttccctcagaagagcaggcttgcggccgccatgtccgcgctgaggaagccaaagtacaacggcaagtgcatgcgcagcctgattaggagcatcctcggcgagacgagggtaagcgagacgctgaccaacgtcatcatccctgccttcgacatcaggctgctgcagcctatcatcttctctacctacgacgccaagagcacgcctctgaagaacgcgctgctctcggacgtgtgcattggcacgtccgccgcgccgacctacctcccggcgcactacttccagactgaagacgccaacggcaaggagcgcgaatacaacctcatcgacggcggtgtggcggccaacaacccgacgatggttgcgatgacgcagatcaccaaaaagatgcttgccagcaaggacaaggccgaggagctgtacccagtgaacccgtcgaactgccgcaggttcctggtgctgtccatcgggacggggtcgacgtccgagcagggcctctacacggcgcggcagtgctcccggtggggcatctgccggtggctccgcaacaacggcatggcccccatcatcgacatcttcatggcggccagctcggacctggtggacatccacgtcgccgcgatgttccagtcgctccacagcgacggcgactacctacgcatccaggacaactcgctccgtggcgccgcggcaaccgtggacgcggcgacgccggagaacatgcggacgctcgtcgggatcggggagcggatgctggcacagcgggtgtccagggtcaacgtggagacagggagc

SEQ ID NO: 12 - DNA, 16619 bp, Zea mays
atcttttattggtttgagttgaacctatatgcacctgtagaatataatctagagcaaactagttagtccaattatttgtgttgggcattcaaccaccaaaattatttataggaaaaggttaaaccctatttccctttcatccgggcccttgcggcggaccgtccgcgacaccagggtgagccttggacaggaacactgcaaaaacacaagttaacactacggatcgtccgatggagaagcgagcaccgtccgagaccaagcacggaccgtccggcctcaggcgcgaatcgcccggtcgttgaaaaaccagaaaaacccgaaggtgacgggttcggtaaaatgcatttttagcgtccttgcggatcgtcctgggtgcacggtcggaccgtccacgactgctttatctgacatttgacgacgcattaaaagctctatagccgttactcctgaccgttgtgatttcagtcgttgatgtgcaggggtacggaccgtccgcggtcggtagaaaatgagcaacgactaggaagtggttggaggctataaatacaagagaaaattcctggtatgccatcagattttatactcatcccttgtgtgccactgagtggcatataagtatatttttttgtgtctatgacatgtggggccagtggcatacaaggaatgagtatatttttcagtggcatacagggaattggccctaaatacaaccccaaccacctccattcaaatgatccaagcactccactcattcacattcaatacaggagctagcaatacattccaagacacactcaaagctttcaatctctcaaagtcccacaatttagacaagtgatcattagtgcttagtgacttgagagagtgtgatctatgtgttatttgtcgctcttgttgcttggctttcacaattgggctttcttcatctctttctcaaccttctaagtgaattataaagcaagcaagagacacctaattttgtggtgatccttgtggggtcttagtgacccgtgtgattaagaagaagcactcgaccggtctaagtgaccgactgagagagggaaagggttggaatagacccggactttgtggcctccttaacggggactaggttctttggaatcaaacctcggtaaacaaatcgctgtgtttatttgtgttgattttcactcgatttgtttcccctcccttcctctctctaaaattcccttgctcatattgttgtgagttggctctcaaagttatctgcattgattgggcaactacttgcaaggataactatcttccgcactccgaattatttctgacattaaccccgggcataatgtgtgttttaagtgtataattttcatgtttcgcctatttacccccctctaggcgactttcaaatgttctccttcacttgtgatgtctacaaccataatcagctcaacatttggactatcacccttgaacacttatgttgaactttaaaagttgtgcactaagcacttgtccaacacttaacacacttgtcagtcctttaattgggttgtcatctaaaccaccaaaaaccacaaagagatctttcaccggggtccgtggttcatggccgtactgctcggtctcaagatttttattataaaatcactagagctctactatttatggttcggtgtgccatcgaaccgtctccaacgggtacatccaacgagcgccagcacaccaacgactagttgacgtggtctacggtccagaggctcatcagacttgtcaggaggctcgtcgactggtctggtgccacacccgtcgacttgggatcgaacaagaatgatggcaagaggacgaagcgcatcaagaagatcatctactacgactcctcttacccttcacacaaggacgacgattccacctcctccaagaaaaatacggttaaacaaggttactctaagacatcttttatttattctcgcattccttacaatttcaatgctcatttgctttctattcatcttggcaagcctgctcgctttgatgggaggactattcttggtggagccataaaatgcgtagccatatttttttgctccaccctagcatttgggatgtcgtagacaatgtaatgcaattgctaggtagcgatgataaaaattataatactattattgcccaataatctattcataatagcgcccaagctaaagaggtgcgctaagggatcctttttatagcccaaagaggtccataggcgttgctccttccttctaaacatcgatgaaattgtgttgtctgcgaggacatcaaaccgggtctgtgcacaccttctccgggatctgatttggtgctttccttaactgattcacagcggaccgatccgatgcaccaccggaccgtctgccacatcagctagtcgttggccttcaaactccaccgggaagtagccgttggaggcggtccggtgcgccattggaccgtgcaaagtgaagggtcgatgatttttataaataaaatctcgagacctcaaagttcagctctgtaggcggtccggtgcacatggacctggttcgatgcattaggtcgcctaacactaagttctatgccctgcggacttgatccggtgcaccaccagacgagtccgatgaggcctagaacaacccaagtaaggctgttttgagcctaacttcttcaaatccttttggctattcttgggagctttccaacaacttagacaaacataattagcacatattccaattgattaggtgtggagaactcaccttttactttgtcgttcaccatgatttgcattttggcttaatctaagtattcgaaccacttttctcacaggatagagttagagttcaaataaagtgctaaacacatagtattagacacatgcaacttatctaagtaatcaaacctcatgattttacccttttgtccaaagctgcacactttagccttcattttagttctttaggatctagtactttcaaattgacttcaagtgcttgtgctcgtactcatatcaaattagttagtccatgttgttgtgctaaacacttaatcactaaaacatgtagaaatggttatctaacacatttttctttcataagtaaaacaggagatttatattgtagatgttattgtttgttgatgaaatttgaaataagagatataagagcaactcgaaaagcctagctaaatcgatttgtatcggtaaaaatagaaaactgatgattaaaataggatccaacaaactctctttgctcctctctatgctatcctgctcagcatcacgtcgaggtctctagccatatttgctgagctcacctgcctcgccatcttcattctctcgtgcatcctcaccgtccctgcgccttgccgtcgttgcagctcactgtcccacgccctgctgtcgccatgcctcgccgaccctgcggctcaccttaccgcgcctcgtcatcgtcgcggctcgccgtctcgtgcctcgccaaccccgctccttgacgtcctcacggcttacagtccccatcgtcctcgtggctccacgcctcgccatatttgcggttcactgtccacgtgccctgccatcctagagcccgacatcgatatgtcaaatgagacaggagaaaaagaaatgaacatgtgattataatcagtgatttgaatattgatagataagatttgaagagtctgttgtgtcatatcacctttttatgaaactctttattttttagagtttttataaaactctaaatttagctaaaattatatctagtcttttagagttactctaacaagagatgagatagcgagctggcgagctgctggagacagccgagagtagagatagtagaggagactagaaactccattaggcctagcccagagtcagctagggatgccgcccgatccactacgtactgaaagcgatcccggcccatgaacgctagtgggttgtaattcggcttacccaagtacccagccgttcctccacacctctgcactacccgaaacccacgcccaacggccgtttcccgcaccccctatccgggaaggaagaaagccagaactcacccctgcttcgtctggcggcgccgtttcccgcacgcgatgccgtcgacggcggaggatttcccggcgataaggaagctggggaagctcttccggcttaccgaagtgtacctctggtaagtctcctgtctcccctacccgcttctcagcgtagggtttgccgtttgcgaggagtacgtctcctcaaactactctctcttcctgcagggacgattcgtatggcgctggacctcacgatggacagaagaacgggcgctcggcggaggctgctctcgtggtacggtctctgacccgctttggtgtagctcactcttaagctttctgagttgggggtgcgcttgtgcttcgactagtagatggctaatttcgtcgggctactggtaatttcttggtatctgcattgtcgagaaagaaggcccgacgcataatttcatgcttgcccaagagtctacttaacacaaggaattggttttgtggcgtggtttgtgcattgcgcccaaactgtagcctgtacaaaatgttaatcgtcgcgtgcattttaaacaaagttttgtattatacgacaaaataccctcggcacatttgttacagactaccgataagtgcatacctatttctcctagttctatcaggaaataatcctggacctcgaaatgacagcctcgtctggctagaaccctactaaacattttgagtgatcacttttcattactcattttcttgatgaaagcacattactgacatggaagtttgctacataagacataacacttccttgtagtgctttatttaattattgaccgatgatctttttggaaaattaagctgtattaaacaattgtagcttcggtgatgattgttggattaagcattagtctgctgcagtcctcttcttgattctgatatgacagttatttgttgattaaaataatgatggtttgctttacacttcgatctcctttgagaggaaaacatgtgaaggtgtggactagatcatgtatagaccaacagcattatcttattaaaacacttctaaataacttagcaatttcataaccatttttacacttctgaggaattcatcttgtcgtgaaagagtcaattaacttagctgcttagcagactgtgtcaagcttattacttgtatgttgtgccctacaaattactatgaggtttataatgtacatagcaatttgacgaccttcaacttttcaggactctcatacagataaaacatgcaatgaagcatccaatagcactgacaaaggttagatgtatttttcttgtattctagtatcttccttggtcaattttctttacagaggatgttacaatgtactctactttttttgtgtggaaacaacccactagagaaaaaaaatcacttcatttgagaaatcttaagaatctgaactctgaagctcagcatgcttccacaccaccacttttcaggccactgtctcttcattggagtaaatgacgcttcttttagagagaaagagaggggggggggtctgtttataattgaatcaagagattttattggtcacctgatttctgttgcatgacgtgggacctggatagacttcagatttgccttagttgataagttcaccggcactagtgaaagaaaagtatatggtacaggtactcttatgaacaggcaaccacttagcaattcagcatctaatagagaaggaccaagtcttcaactaaagtcacaatatacctttagtactattagaggggctgaccctccttgtctagtgcttgtgagatcataggagatggggcgtggtggttaagattgtggatcatattcgccaagctcccagggtcaatgtgattgagggatgtggtatgctacttgtgaaagggttcaaaaaggccaggatgacattgttcctacattcctggaatggggatgacacccccaggacaaggaaggtggcacagttccacgttcctggtgacatgttgtgtatcaaatgggaggccaaatcaccacgggattactctaggaagggaagatgatgttgataatttgagtcattgttgcaacatctgttcatggtttcatgcctcattttataagtcatattgcccacacataacattgtaatagtaaaatcaacaccagttattttacgttttcccttgtatgtcaaccgatttcttactgtgtatatgatctgtctatcaataggccatttctttgttgaagatttggaattggtcaatctcatgggttctttggggcttcctgtttcattcagcacaagtaaagtggtcagttgctcacatagtgtgacaccatgttactgttccctaccggttccattgcttaattcctttatgcattgcagaacaagaacacatgcaacaagggaaagaaaaaaggaagacaagcaccgctcaaagcagcaaacactcaaatcaatgatgctgtgaggatatgtatcaatactgaagatagagaaaattctgttgaatcattggatgctatggagcaaacgcactcatgcaatttatttgtgacaccactgggtcaaaatgaaccctcccgtgatgacactgacaagaggcttagggaagacagctcttgtgttgaagaacaagaagagtctggctgtagcaccatctactctgctggcaaagcccctggctgtgatgctaaaaatcatctcactgaacttggggcttttgagctttctgataacttggccaactcagcaaaagaagaatactcaattcaagaaaatcaagcttatgaaagtgtgttgctagattctgaagagatgtcaaggaatgactgtgttgatgatgaatctacacattcctgtgttggcatttatcaggatgaaagagtgtccacaaggggagatcaaacatctgaagaaactctatcagtaccccatgattacaatgatgttggcagagaagctagtctaagtttggcagagccatcatctattgatgagcatgcacaaagctctgccaacaacttttactatgactatggtgaatggagggttatctgggatccattctataatcggtattatttttacaacatccagacacaagagtccacatggtgtcctcctgaaggactggaggattttgcatcatattgtagcccagataccactaaagagctagctgaactgggatctcagtgttcaagcatggcaccacaagagaacagtaaaaaccctagtctcgtcctttgcagttgacattacgaatagttatatgcactacgataaaaactttctacaatatgtaacacttgagcatgtggcaatgggtgtaaacatttaataataaggtagtgaaatccattacacacagtattgaattttgcactacaaatgctgaaggagaaacctaaattgtcaatgctttttggtgacattaattattgccattgatttcctgcttgtaggtgcttcatttatctgtctccaatttactcatatgctagcttcttgtttgggactaaaggctttgctgttgttttagtatgtcacacatttctctttaatctcaccatcacagatctggctactcatgtcaatcatttagaagcacaggagcaagatcactgcattcatgatttatctgacattcctgttgaaaagccaatatatcaaaggtagggaataccaaactgtacaatgttgaacaagttattgtttttttttgttaattctgttcatctatgcagtatgataactacctctgacaaagcacagcacactgaaaataagtacagcgattcaacaactactgtgttagagatgaaccaggaagttgctagcaccaaaacgaaaaagagagtaaggagatctcgatcgtgtaaggcgataatatatggcatctgctttctaggagtttgttcctgttacaattttaggttgcgcatttacacaatagtttcttggtttctttgagcaaatgcagctttgcatgactgctacattgcctacttatgtctaggtaacttttctttgcaaactgcaaagttatgtctaggtaactatgccttctagaaaacctccttgttagctatgtattagtgagacttgcctaatatttattttcttgtggtccgttcttgtgctctttgtacatatttgccaataaccattttaattgttctacagatcattcatgccaagacatggcagggaacgtctctaatgacatcatcaagtactgggctcagcggtattcacttttctcactttttgatagtggtataaagatggatgaagtagggtggttttcagttacgccagagccaattgcaaagcatcatgcatctcgtgtgggtgcgggagtaatgattgattgtttcacaggagttggtggaaatgccatccaatttgccaaaaagtacgtcaatgttatcttgcaattgagttatgtgatggtctaatgtatcatttgcttgaacacttcctgtttagtagcaactgttatttttcttatgtcacgagaatgcaatggctatatcaccttaagcagtatgctatgtccactgtccagtttaactaaggcatctgcttccagtaatatgcaaggctcttcttacttttgctgttatttaatatatggaagtgtccttacggaggtgttattgtggacattttgagcatgttcatcatgtcacttgagttagtagagccagccttagttgtttgcagtgtaggtggatttattttatgttatcaatgtttcttctacagtactaagactattgttccacattaactatgtctccttttccaggtgcaagcatgtaattgcagttgatattgatccacaaaagattgattgcgcgcatcataatgcatccatttatggagtaaatgatcacatagatttcattgtaggtgattttatacatatagctcctcatctgaaggtaatgcctttttcttggaattattacttttaagtttctcaacacgtcacttctattagctatatgtttttgtagctgtttgcgagagtgaatttattgttgacattgttctcatttgcccacccattttaggataggggcttggtactacaaatatcttgatacttcaagtcctacaaaaagaaatttatgtttcatattttttccatttgaacgtcgagattttatggtcccatggagttctccctatttttcgatgatgcccatcttttggcagtaccttctttgtgtacacaataaatgggaggatattttctgcagggagaaactgctttcatgtcgcctccttggggtggccctgactatgccaaagttgatgtttatgatatgaaaagcatgcttattccttgtgatgggttagttccttgtttctattttaagagagtaatttctttcagtttgcactcactgatgtttacttactttgtgagtaaaacgcaccagagatccattaacctttaaggaggtgttatctatgtccatcaacactcaaactgcatttttgggttcctaaactttttaagtgattcaccggagttccgtaccccttcgtttatatttgtattttgcagaaacctcactctgttttatttctccttcgcatgtaggggtggtaatggatcacgattcaaacgtttctccacgattcgtttgagcccttaattaattttagtacaaaaataaatagaaatagagatagagcctgatcctaatatgatttgatcctcaaattttatagcgtagaatttagagcccattaccatttaccacccctattcacatgcctacccctctccatcttctggattgaatgttccaacctaatttacactcgtagtttctttgatctgccaatcaaatccagagcctaattgctataacattagaacgaacacgccatattaccagaatactcgatgcagatatggatagaagcgaggcgctaagcgcagccagccttggcttcttgctctgcaggccgatcagggcgccagccaaagccaaccatgcgcgcacgtgactgcaatgctactctctcttcgcctttgccatcgtcgtcgcaggatgttacgttgtgcttatgctggctcccacgagtgccgccgcccagagcgagctgagcgcacgcagccactgcttgtggttcacgagcgtgagcatgccctcaccacctgctgctgcgcccttgctgcttgcttgcttgccggtggtgtacattatggacggattaaattgaatggatttacctgttccagaaaaagatctgatcgacgatgggatgctatcttgtatggctccggatcaatgaagattaatggaacaaccaatcgaaggctcagagcaggctagttggtgcccggaagactctggccagaagatggaaatgggtaagcgtgtgaaggaaaaaagaaatagagggggatttctacaaaaaacaaacataatgaagaggtatggatttcaggtgaaccacttaaaaaataaaaagggcatacccagtgccgtaggcttcccgcactgtgcggggtcgtctggggaagggtatctttaagcgtcaagtcttacccgcataatatgcagaggctggggctcgaacccgggacctttcggttatagacggtaggctctaccgccgcaccaagcccgcccttgaaccatttaaaaaatttaggactcaaaaatacagtttgacagttgatggacctagatgacacctccttaaaaaatttaatggacctatggtgcattttaatcttttgttgatcgactatactcaatgttgaactctttaggtactctctttttaaactcggaaccatgatagcttcaagagtagtgatgtttcttcctcgcaacattgacctaaaccaattggcggacatgtccttgtctgtggatcccccgtgggcagttgaggtaagcccatttttgctgattttgtgccaagctgacgtttcctatagatgtcacagtggtctctctctctgcaggtcgagaagaacttcctcaacggaaagctgaaagccataacagcttactttgaagaacaggatcgttgaaccaagcatcggcgctggtgatacaaatcatcttgttagctatgactcacgacaaatttttgtggtgaccctaaacagaacctttgtgttcggagacagaaagaagcggtttatcatcttcaccgagcatagataatttatttgcagagatgagtcattggtatcatacaaaagcagctcagcttatctcaattcacagcaagtgaaactgtcgaaggaaaactacaaggctgacagtcgaacgcgtgggagttagcttaattttgccttatgataagcaagcatgcttcctggtttatttcatacagctactagtagtttcagctgcaacagttgtgcgttggtgtgcgtgtgattctcacatatctggtcctgcggatgtgagtgatgcaaatgtatgtgtcatcatcccatgtaagggtttgtttgtttgctctcaatctatgtagattgagtgggattaagtgagtttaaatctcagacaagtcaaaaaaaaatgttttcaatctcatccaatccacatatgatagtaatacccgagtaaggcttagatgtaatagttggaataagaaaaacaagtcagccattttgaagttttgtccttggagttctattaaaaggcattactgataaatctccaacagatttgcagttgaagcaacatgtgaaacatatttatcatgttaaaacaatttgccttagtattcgattatgccatgaaatctgacatttccttacacatcccagtttatcattgtcaactgtctttaggaatgtattgtatctgctgtttttacttgtatatgtatgttattttttgtcgttgtatgtatatgttttattataaacatggccactaaggttgttctattcgttaaaataacacagatctataaacgactaaacaagcttcttgggataaagaatcatatggaggctggattttcgaggagtctggtgcactgttttgctaatgatcagccccccccccccccccctctaaaaataaagaaaatactggatttcctgttcatttattacattcatatgtaaatgcttctgtccttttctatatctgggctggactttttgtgtgctcgtcactcaagttggttagtgtggttaattttattatgctccgtgctctttcctaccgaacttggtctttgttagtatcattatcagtcagttatattttctcctcttgatgcttcatctaatctatttttgcaaagttgtcatgttatgtactatatgatcttttacaaggtttttgacttttcaaattattgtgtcgtatattatttgtactcagattgtgcttacaactttagtttatctatactttaaggggtgtttggtttctatgggctaatttataatcccttcattttattctattttcgtacctaaattgtcaagcacgaaaacgaaaataaagttttaacttttatatttagcagtttatacactaaaatagaataaaatagatgaagtaaaaattagtcctcagaaaccaaacatctcctaaatgtctagtaatagtcgcctgaactgtagagcgcccaacacgcgccaccctgatttggtgtcttaaaatggcatgtgtatataggtggaatgggtttgacgagactgtaactactttttcttaattaaattatagatggacttaacttttctatatgcattttaaatatatttttctatatttttggtgggctgagttacagtttatgtcaatataaattacaacagaccgaatctaaaattttattataaaatgtatgcaccaaccgttgactaaaaagataaaatttggacacctacattttagcaagtcacctgctaatatatatctatactaggtaagtgtccgtgcgttgcaacgaaaacatataataatacgataacttatatataaaatatgtgttatactgttatgagaaaaagtttcacctgtcctatttttatcaatatgacaacagaggatcaatataaggccttggcatggcttcagaagttcagattaacgaattatggagcaagagcaactatttctggtgtttcagtagaaagaatggggatatgtgtttatctctctcatacatgttacacaatgtgctatagaatgacacctctaggccgctgctacaactacagagaataaattatggatcatgggtgccctactaagttagctacacgtaaaatctggggcgattgaccccctaatgcttcatcttggagatctcactaaaatacaccttccgcacaaaccgagccttgataaagctcgcgatcttcgtgtcctgatctttagtgcagacaactgcaagggaaattattgtgccggtcagcaagagtggaaaatgtcagcagaaacacaagaatggaaaattatatgatgtgcaagtaggacggcaccctatttaactaaaggtgtgtttggttcagttttctgaaccaattcgttgccaaaaaatctaaaatctcacacaaacggtacaacatcagaatagatttttaaaagtttatagatttctcaagttcaattcaaaatcaccatctaccccaaatttttcagattactattattcatgttacaactatcactcttgtagtatctaccattgatagttgttttaatcaaatatattttagctttctcacaatcctcagctcgaaacagattttcatggctcacagttggattcatattttcataaatctataggtgtgaaccaaatagaccctaaaacatcatgttgtaatgttccaaaaaaatcatcacaaaaaacatgtatgcaacacacctaagtgcaacaacactaacctgcaggagcgttggcgtaggctggactcttgtgtgtctgcaatgtggaaacctgcattgtaaatggttaggtaaatgcttcgcttaaaaatggcagtaaatgcttcactaaaaatgcttccacgtgctcatgatcaagtaggttttatgttcaatctgcagttctacacaagtgcgattcattttgatactcatttctatttactttcagagctcgtgctaactgtcataaagtgcaatgcatctatgactgccaattgatattgtgctcctgccataaagtgcactgcatcgtgctaactgtacactaatctgtgaggatctaagaccaatatttgtttacgttttctcctttagtatcctataaaaacaacacgcctagacaacccaaaaaatgtgtcccaataggaatatcagattctgacgctggcagcaatctcgaatgataatattttttccaaacaagcgaggtccctaaatagaagcggcaacagataaaaactaaagataaaaactaaagagtacagatgattggcatcacatcgggaatgaaatatgcctaacatatcaatttgcatattagattatttgctgagaacaataacgaaaacatatttagttgttcatcacaagttaccttagattttgctgttcaaggtcctttgggtcttctttctgctagaacatacaagggtatttcagatttgcaaacaaggaaaagcaagaacttcaatgatacatcattgtaaaaccaagtttccgatttaaataaagatgatgcttgcggtcaacacattcacaaatgtaaatgtgtgaaatcgttcaaacataaggcttatgtggtcatgctcaggtagtatgtacagacctaaaaacaaggtatatgacaacagtaccagccactaaacacacatggttaatcactaaaacaattctccgattaaccaggaaaactatagcagccactagaactatacaggtttctaccagtaattgcttcactaaaaaatgcccccatgtgtaaattttcaggtggtttgtacagacataaaaacaagggtataggactacttcttgtgctaaaataaaagctggcactaaacagtgtatccagttcatcaggaaaacagttttagtgattaatcactaaaacaatacccatggtgcaaattatctgattaaccatgtacataccagtaattgcttcataaaaaatgcccccaatttgctcatgtttaaggaatatgtatagaactaaaaacaagggtatatgataacaataccagccactaaacacacatggttaatcactaaaacaattctctgacaactcctataaaaagatagcaaccaccagaaataaaccgcccacgacatccctaattgtagtcactaaaaactggtagcagtaattggttcactaaaaaatgaccataatcacgaaaactataacagtcaccagaactatataggtttcattagtaattgcttcactaaaaaatgtccccatgtgtaaattttcatgtcgtatgtatagacctaaaaacaagggtatatgactacttgctatgctaaaacaatagctagcactaaacagtgtattcagttaatcatccaaacaattttgtgattaatcactaaaacaatacccatggagcaaattatatgagaataagatctcgtcgttcctattgtgaagaatatactactacctccagtttcaaattacaatttcaaattacaagttgtttagaacatccacaaggtaattgcgaagaatatactaattgctctagtttcaaattagaagttgtttagagaaaaggtgttccttaatagtctagttttagaagctacatccaactggtaaacataaattgcagaaaccttttatgtggaagcctccgtcattgagtctgtcccctttagctgtaagtagttttctaaatattgttagtcaggcttagttgtttgagactctgtttccattcgtgaccatgggaactgtgaaatgtgtagaagatgctcatgctcatgcatatgcatcgaattgttttgtaaagtcatcttaatgctcaaacagtttttttatctgccccagctgtacactgctttctgaattatgtcatttaggcttagctgtccgagataatttcatttgtgatgaaggtaaccggagcatctgtccttttgttttaaacataaatattttgatagcttaacttgtgcgtcattttatcatgtactaacatggtatatagatggcacttagcagtaacattcctgacttatgtgattgtcctgttagaatgcttctgcaatataatgggcttatgctaatctgtttggaatcccatgatgaataacaattatggatgttgggcattttgtatttttatgatgtaggcttaacatattttcttctctgctcagccctgccggtggagacctctatttatagctataatccagccatatctagtgaactaacagatctattcctatctctagtgcttatccccttaacagatttattttcctatctctatttctttgatgttacttgctgcaggtgctatcccccactgatgcattatatgacaatcactcgaagaatcagatgctaattaattgttttatacttgaccattgctaattaagtactccatttttt

SEQ ID NO: 13 - DNA, 17274 bp, Zea mays
caaccctttccctctctcaaacggtcacttagaccgagtgaggcttcttccttaatctcatgggtcacttagaccccgcaaggatcaccacacaattggtgtctcttgcctcgcttacaaagcacttgagagtaagaagtgagaaagaaaagaaagccaagccaagcaaacaagagcaacaaagaaacacaaatgatcctttaacaagttctaatgcgctagagttgaatcgagaactttgagtggatcgatcacttgaattgtgtctttgcagtggagtctattgctcttgtattgaatgcaatgtgttgaatgcttggatggttagagtggaggtggttgggggtatttatagccctcaaccaccaaacaactgttggggaggggttgctgtcgatgggcgcaccggacagtccggtgcgccagcaacgtcacccaaccgttagggttcgagcgcagacgactgttggagctttgtcttcttgtgccaccgaacagtcaggtgccgcaccggacaggcactgttcactgtccggtgcgcctctgacggctgctctaacttctgcgcgcactggtcgcacactgtagcgttcgcaggtgtccgttgcagtcgaccattgtgctggaagccgttgctccgtttggtgcatcggacagtctggtggcacaccggacagtctggtgaattatagcggagtgcggcctgagaaacccgaaggtggagagttcggagttgtacggtcctggtgcatcggacactgttcggtgcgccagaccagggcacctttggtttctttgttcctttgcttttgaaccctaactttgatcttttattggtttgagttgaacctatatgcacctgtagaatataatctagagcaaactagttagtccaattatttgtgttgggcattcaaccaccaaaattatttataggaaaaggttaaaccctatttccctttcatccgggcccttgcggcggaccgtccgcgacaccagggtgagccttggacaggaacactgcaaaaacacaagttaacactacggatcgtccgatggagaagcgagcaccgtccgagaccaagcacggaccgtccggcctcaggcgcgaatcgcccggtcgttgaaaaaccagaaaaacccgaaggtgacgggttcggtaaaatgcatttttagcgtccttgcggatcgtcctgggtgcacggtcggaccgtccacgactgctttatctgacatttgacgacgcattaaaagctctatagccgttactcctgaccgttgtgatttcagtcgttgatgtgcaggggtacggaccgtccgcggtcggtagaaaatgagcaacgactaggaagtggttggaggctataaatacaaccccaaccacctccattcaaatgatccaagcactccactcattcacattcaatacaggagctagcaatacattccaagacacactcaaagctttcaatctctcaaagtcccacaatttagacaagtgatcattagtgcttagtgacttgagagagtgtgatctatgtgttatttgtcgctcttgttgcttggctttcacaattgggctttcttcatctctttctcaaccttctaagtgaattataaagcaagcaagagacacctaattttgtggtgatccttgtggggtcttagtgacccgtgtgattaagaagaagcactcgaccggtctaagtgaccgactgagagagggaaagggttggaatagacccggactttgtggcctccttaacggggactaggttctttggaatcaaacctcggtaaacaaatcgctgtgtttatttgtgttgattttcactcgatttgtttcccctcccttcctctctctaaaattcccttgctcatattgttgtgagttggctctcaaagttatctgcattgattgggcaactacttgcaaggataactatattccgcactccgaattatttctgacattaaccccgggcataatgtgtgttttaagtgtataattttcatgtttcgcctatttacccccctctaggcgactttcaaatgttctccttcacttgtgatgtctacaaccataatcagctcaacatttggactatcacccttgaacacttatgttgaactttaaaagttgtgcactaagcacttgtccaacacttaacacacttgtcagtcctttaattgggttgtcatctaaaccaccaaaaaccacaaagagatctttcaccggggtccgtggttcatggccgtactgctcggtctcaagatttttattataaaatcactagagctctactatttatggttcggtgtgccatcgaaccgtctccaacgggtacatccaacgagcgccagcacaccaacgactagttgacgtggtctacggtccagaggctcatcagacttgtcaggaggctcgtcgactggtctggtgccacacccgtcgacttgggatcgaacaagaatgatggcaagaggacgaagcgcatcaagaagatcatctactacgactcctcttacccttcacacaaggacgacgattccacctcctccaagaaaaatacggttaaacaaggttactctaagacatcttttatttattctcgcattccttacaatttcaatgctcatttgctttctattcatcttggcaagcctgctcgctttgatgggaggactattcttggtggagccataaaatgcgtagccatatttttttgctccaccctagcatttgggatgtcgtagacaatgtaatgcaattgctaggtagcgatgataaaaattataatactattattgcccaataatctattcataatagcgcccaagctaaagaggtgcgctaagggatcctttttatagcccaaagaggtccataggcgttgctccttccttctaaacatcgatgaaattgtgttgtctgcgaggacatcaaaccgggtctgtgcacaccttctccgggatctgatttggtgctttccttaactgattcacagcggaccgatccgatgcaccaccggaccgtctgccacatcagctagtcgttggccttcaaactccaccgggaagtagccgttggaggcggtccggtgcgccattggaccgtgcaaagtgaagggtcgatgatttttataaataaaatctcgagacctcaaagttcagctctgtaggcggtccggtgcacatggacctggttcgatgcattaggtcgcctaacactaagttctatgccctgcggacttgatccggtgcaccaccagacgagtccgatgaggcctagaacaacccaagtaaggctgttttgagcctaacttcttcaaatccttttggctattcttgggagctttccaacaacttagacaaacataattagcacatattccaattgattaggtgtggagaactcaccttttactttgtcgttcaccatgatttgcattttggcttaatctaagtattcgaaccacttttctcacaggatagagttagagttcaaataaagtgctaaacacatagtattagacacatgcaacttatctaagtaatcaaacctcatgattttacccttttgtccaaagctgcacactttagccttcattttagttctttaggatctagtactttcaaattgacttcaagtgcttgtgctcgtactcatatcaaattagttagtccatgttgttgtgctaaacacttaatcactaaaacatgtagaaatggttatctaacacatttttctttcataagtaaaacaggagatttatattgtagatgttattgtttgttgatgaaatttgaaataagagatataagagcaactcgaaaagcctagctaaatcgatttgtatcggtaaaaatagaaaactgatgattaaaataggatccaacaaactctctttgctcctctctatgctatcctgctcagcatcacgtcgaggtctctagccatatttgctgagctcacctgcctcgccatcttcattctctcgtgcatcctcaccgtccctgcgccttgccgtcgttgcagctcactgtcccacgccctgctgtcgccatgcctcgccgaccctgcggctcaccttaccgcgcctcgtcatcgtcgcggctcgccgtctcgtgcctcgccaaccccgctccttgacgtcctcacggcttacagtccccatcgtcctcgtggctccacgcctcgccatatttgcggttcactgtccacgtgccctgccatcctagagcccgacatcgatatgtcaaatgagacaggagaaaaagaaatgaacatgtgattataatcagtgatttgaatattgatagataagatttgaagagtctgttgtgtcatatcacctttttatgaaactctttattttttagagtttttataaaactctaaatttagctaaaattatatctagtcttttagagttactctaacaagagatgagatagcgagctggcgagctgctggagacagccgagagtagagatagtagaggagactagaaactccattaggcctagcccagagtcagctagggatgccgcccgatccactacgtactgaaagcgatcccggcccatgaacgctagtgggttgtaattcggcttacccaagtacccagccgttcctccacacctctgcactacccgaaacccacgcccaacggccgtttcccgcaccccctatccgggaaggaagaaagccagaactcacccctgcttcgtctggcggcgccgtttcccgcacgcgatgccgtcgacggcggaggatttcccggcgataaggaagctggggaagctcttccggcttaccgaagtgtacctctggtaagtctcctgtctcccctacccgcttctcagcgtagggtttgccgtttgcgaggagtacgtctcctcaaactactctctcttcctgcagggacgattcgtatggcgctggacctcacgatggacagaagaacgggcgctcggcggaggctgctctcgtggtacggtctctgacccgctttggtgtagctcactcttaagctttctgagttgggggtgcgcttgtgcttcgactagtagatggctaatttcgtcgggctactggtaatttcttggtatctgcattgtcgagaaagaaggcccgacgcataatttcatgcttgcccaagagtctacttaacacaaggaattggttttgtggcgtggtttgtgcattgcgcccaaactgtagcctgtacaaaatgttaatcgtcgcgtgcattttaaacaaagttttgtattatacgacaaaataccctcggcacatttgttacagactaccgataagtgcatacctatttctcctagttctatcaggaaataatcctggacctcgaaatgacagcctcgtctggctagaaccctactaaacattttgagtgatcacttttcattactcattttcttgatgaaagcacattactgacatggaagtttgctacataagacataacacttccttgtagtgctttatttaattattgaccgatgatctttttggaaaattaagctgtattaaacaattgtagcttcggtgatgattgttggattaagcattagtctgctgcagtcctcttcttgattctgatatgacagttatttgttgattaaaataatgatggtttgctttacacttcgatctcctttgagaggaaaacatgtgaaggtgtggactagatcatgtatagaccaacagcattatcttattaaaacacttctaaataacttagcaatttcataaccatttttacacttctgaggaattcatcttgtcgtgaaagagtcaattaacttagctgcttagcagactgtgtcaagcttattacttgtatgttgtgccctacaaattactatgaggtttataatgtacatagcaatttgacgaccttcaacttttcaggactctcatacagataaaacatgcaatgaagcatccaatagcactgacaaaggttagatgtatttttcttgtattctagtatcttccttggtcaattttctttacagaggatgttacaatgtactctactttttttgtgtggaaacaacccactagagaaaaaaaatcacttcatttgagaaatcttaagaatctgaactctgaagctcagcatgcttccacaccaccacttttcaggccactgtctcttcattggagtaaatgacgcttcttttagagagaaagagagggggggggggtctgtttataattgaatcaagagattttattggtcacctgatttctgttgcatgacgtgggacctggatagacttcagatttgccttagttgataagttcaccggcactagtgaaagaaaagtatatggtacaggtactcttatgaacaggcaaccacttagcaattcagcatctaatagagaaggaccaagtcttcaactaaagtcacaatatacctttagtactattagaggggctgaccctccttgtctagtgcttgtgagatcataggagatggggcgtggtggttaagattgtggatcatattcgccaagctcccagggtcaatgtgattgagggatgtggtatgctacttgtgaaagggttcaaaaaggccaggatgacattgttcctacattcctggaatggggatgacacccccaggacaaggaaggtggcacagttccacgttcctggtgacatgttgtgtatcaaatgggaggccaaatcaccacgggattactctaggaagggaagatgatgttgataatttgagtcattgttgcaacatctgttcatggtttcatgcctcattttataagtcatattgcccacacataacattgtaatagtaaaatcaacaccagttattttacgttttcccttgtatgtcaaccgatttcttactgtgtatatgatctgtctatcaataggccatttctttgttgaagatttggaattggtcaatctcatgggttctttggggcttcctgtttcattcagcacaagtaaagtggtcagttgctcacatagtgtgacaccatgttactgttccctaccggttccattgcttaattcctttatgcattgcagaacaagaacacatgcaacaagggaaagaaaaaaggaagacaagcaccgctcaaagcagcaaacactcaaatcaatgatgctgtgaggatatgtatcaatactgaagatagagaaaattctgttgaatcattggatgctatggagcaaacgcactcatgcaatttatttgtgacaccactgggtcaaaatgaaccctcccgtgatgacactgacaagaggcttagggaagacagctcttgtgttgaagaacaagaagagtctggctgtagcaccatctactctgctggcaaagcccctggctgtgatgctaaaaatcatctcactgaacttggggcttttgagctttctgataacttggccaactcagcaaaagaagaatactcaattcaagaaaatcaagcttatgaaagtgtgttgctagattctgaagagatgtcaaggaatgactgtgttgatgatgaatctacacattcctgtgttggcatttatcaggatgaaagagtgtccacaaggggagatcaaacatctgaagaaactctatcagtaccccatgattacaatgatgttggcagagaagctagtctaagtttggcagagccatcatctattgatgagcatgcacaaagctctgccaacaacttttactatgactatggtgaatggagggttatctgggatccattctataatcggtattatttttacaacatccagacacaagagtccacatggtgtcctcctgaaggactggaggattttgcatcatattgtagcccagataccactaaagagctagctgaactgggatctcagtgttcaagcatggcaccacaagagaacagtaaaaaccctagtctcgtcctttgcagttgacattacgaatagttatatgcactacgataaaaactttctacaatatgtaacacttgagcatgtggcaatgggtgtaaacatttaataataaggtagtgaaatccattacacacagtattgaattttgcactacaaatgctgaaggagaaacctaaattgtcaatgctttttggtgacattaattattgccattgatttcctgcttgtaggtgcttcatttatctgtctccaatttactcatatgctagcttcttgtttgggactaaaggctttgctgttgttttagtatgtcacacatttctctttaatctcaccatcacagatctggctactcatgtcaatcatttagaagcacaggagcaagatcactgcattcatgatttatctgacattcctgttgaaaagccaatatatcaaaggtagggaataccaaactgtacaatgttgaacaagttattgttttttttgttaattctgttcatctatgcagtatgataactacctctgacaaagcacagcacactgaaaataagtacagcgattcaacaactactgtgttagagatgaaccaggaagttgctagcaccaaaacgaaaaagagagtaaggagatctcgatcgtgtaaggcgataatatatggcatctgctttctaggagtttgttcctgttacaattttaggttgcgcatttacacaatagtttcttggtttctttgagcaaatgcagctttgcatgactgctacattgcctacttatgtctaggtaacttttctttgcaaactgcaaagttatgtctaggtaactatgccttctagaaaacctccttgttagctatgtattagtgagacttgcctaatatttattttcttgtggtccgttcttgtgctctttgtacatatttgccaataaccattttaattgttctacagatcattcatgccaagacatggcagggaacgtctctaatgacatcatcaagtactgggctcagcggtattcacttttctcactttttgatagtggtataaagatggatgaagtagggtggttttcagttacgccagagccaattgcaaagcatcatgcatctcgtgtgggtgcgggagtaatgattgattgtttcacaggagttggtggaaatgccatccaatttgccaaaaagtacgtcaatgttatcttgcaattgagttatgtgatggtctaatgtatcatttgcttgaacacttcctgtttagtagcaactgttatttttcttatgtcacgagaatgcaatggctatatcaccttaagcagtatgctatgtccactgtccagtttaactaaggcatctgcttccagtaatatgcaaggctcttcttacttttgctgttatttaatatatggaagtgtccttacggaggtgttattgtggacattttgagcatgttcatcatgtcacttgagttagtagagccagccttagttgtttgcagtgtaggtggatttattttatgttatcaatgtttcttctacagtactaagactattgttccacattaactatgtctccttttccaggtgcaagcatgtaattgcagttgatattgatccacaaaagattgattgcgcgcatcataatgcatccatttatggagtaaatgatcacatagatttcattgtaggtgattttatacatatagctcctcatctgaaggtaatgcctttttcttggaattattacttttaagtttctcaacacgtcacttctattagctatatgtttttgtagctgtttgcgagagtgaatttattgttgacattgttctcatttgcccacccattttaggataggggcttggtactacaaatatcttgatacttcaagtcctacaaaaagaaatttatgtttcatattttttccatttgaacgtcgagattttatggtcccatggagttctccctatttttcgatgatgcccatcttttggcagtaccttctttgtgtacacaataaatgggaggatattttctgcagggagaaactgctttcatgtcgcctccttggggtggccctgactatgccaaagttgatgtttatgatatgaaaagcatgcttattccttgtgatgggttagttccttgtttctattttaagagagtaatttctttcagtttgcactcactgatgtttacttactttgtgagtaaaacgcaccagagatccattaacctttaaggaggtgttatctatgtccatcaacactcaaactgcatttttgggttcctaaactttttaagtgattcaccggagttccgtaccccttcgtttatatttgtattttgcagaaacctcactctgttttatttctccttcgcatgtaggggtggtaatggatcacgattcaaacgtttctccacgattcgtttgagcccttaattaattttagtacaaaaataaatagaaatagagatagagcctgatcctaatatgatttgatcctcaaattttatagcgtagaatttagagcccattaccatttaccacccctattcacatgcctacccctctccatcttctggattgaatgttccaacctaatttacactcgtagtttctttgatctgccaatcaaatccagagcctaattgctataacattagaacgaacacgccatattaccagaatactcgatgcagatatggatagaagcgaggcgctaagcgcagccagccttggcttcttgctctgcaggccgatcagggcgccagccaaagccaaccatgcgcgcacgtgactgcaatgctactctctcttcgcctttgccatcgtcgtcgcaggatgttacgttgtgcttatgctggctcccacgagtgccgccgcccagagcgagctgagcgcacgcagccactgcttgtggttcacgagcgtgagcatgccctcaccacctgctgctgcgcccttgctgcttgcttgcttgccggtggtgtacattatggacggattaaattgaatggatttacctgttccagaaaaagatctgatcgacgatgggatgctatcttgtatggctccggatcaatgaagattaatggaacaaccaatcgaaggctcagagcaggctagttggtgcccggaagactctggccagaagatggaaatgggtaagcgtgtgaaggaaaaaagaaatagagggggatttctacaaaaaacaaacataatgaagaggtatggatttcaggtgaaccacttaaaaataaaaagggcatacccagtgccgtaggcttcccgcactgtgcggggtcgtctggggaagggtatctttaagcgtcaagtcttacccgcataatatgcagaggctggggctcgaacccgggacctttcggttatagacggtaggctctaccgccgcaccaagcccgcccttgaaccatttaaaaaatttaggactcaaaaatacagtttgacagttgatggacctagatgacacctccttaaaaattttaatggacctatggtgcattttaatcttttgttgatcgactatactcaatgttgaactctttaggtactctctttttaaactcggaaccatgatagcttcaagagtagtgatgtttcttcctcgcaacattgacctaaaccaattggcggacatgtccttgtctgtggatcccccgtgggcagttgaggtaagcccatttttgctgattttgtgccaagctgacgtttcctatagatgtcacagtggtctctctctctgcaggtcgagaagaacttcctcaacggaaagctgaaagccataacagcttactttgaagaacaggatcgttgaaccaagcatcggcgctggtgatacaaatcatcttgttagctatgactcacgacaattttttgtggtgaccctaaacagaacctttgtgttcggagacagaaagaagcggtttatcatcttcaccgagcatagataatttatttgcagagatgagtcattggtatcatacaaaagcagctcagcttatctcaattcacagcaagtgaaactgtcgaaggaaaactacaaggctgacagtcgaacgcgtgggagttagcttaattttgccttatgataagcaagcatgcttcctggtttatttcatacagctactagtagtttcagctgcaacagttgtgcgttggtgtgcgtgtgattctcacatatctggtcctgcggatgtgagtgatgcaaatgtatgtgtcatcatcccatgtttgtttgtttgctctcaatctatgtagattgagtgggattaagtgagtttaaatctcagacaagtcaaaaaaaaatgttttcaatctcatccaatccacatatgatagtaatacccgagtaaggcttagatgtaatagttggaataagaaaaacaagtcagccattttgaagttttgtccttggagttctattaaaaggcattactgataaatctccaacagatttgcagttgaagcaacatgtgaaacatatttatcatgttaaaacaatttgccttagtattcgattatgccatgaaatctgacatttccttacacatcccagtttatcattgtcaactgtctttaggaatgtattgtatctgctgtttttacttgtatatgtatgttattttttgtcgttgtatgtatatgttttattataaacatggccactaaggttgttctattcgttaaaataacacagatctataaacgactaaacaagcttcttgggataaagaatcatatggaggctggattttcgaggagtctggtgcactgttttgctaatgatcagaccccccccccccctctaaaaataaagaaaatactggatttcctgttcatttattacattcatatgtaaatgcttctgtccttttctatatctgggctggactttttgtgtgctcgtcactcaagttggttagtgtggttaattttattatgctccgtgctctttcctaccgaacttggtctttgttagtatcattatcagtcagttatattttctcctcttgatgcttcatctaatctatttttgcaaagttgtcatgttatgtactatatgatcttttacaaggtttttgacttttcaaattattgtgtcgtatattatttgtactcagattgtgcttacaactttagtttatctatactttaaggggtgtttggtttctatgagctaatttataatcccttcattttattctattttcgtacctaaattgtcaagcacgaaaacgaaaataaagttttaacttttatatttagcagtttatacactaaaatagaataaaatagatgaagtaaaaattagtcctcagaaaccaaacatctcctaaatgtctagtaatagtcgcctgaactgtagagcgcccaacacgcgccaccctgatttggtgtcttaaaatggcatgtgtatataggtggaatgggtttgacgagactgtaactactttttcttaattaaattatagatggacttaacttttctatatgcattttaaatatatttttctatatttttggtgggctgagttacagtttatgtcaatataaattacaacagaccgaatctaaaattttattataaaatgtatgcaccaaccgttgactaaaaagataaaatttggacacctacattttagcaagtcacctgctaatatatatctatactaggtaagtgtccgtgcgttgcaacgaaaacatataataatacgataacttatatataaaatatgtgttatactgttatgagaaaaagtttcacctgtcctatttttatcaatatgacaacagaggatcaatataaggccttggcatggcttcagaagttcagattaacgaattatggagcaagagcaactatttctggtgtttcagtagaaagaatggggatatgtgtttatctctctcatacatgttacacaatgtgctatagaatgacacctctaggccgctgctacaactacagagaataaattatggatcatgggtgccctactaagttagctacacgtaaaatctggggcgattgaccccctaatgcttcatcttggagatctcactaaaatacaccttccgcacaaaccgagccttgataaagctcgcgatcttcgtgtcctgatctttagtgcagacaactgcaagggaaattattgtgccggtcagcaagagtggaaaatgtcagcagaaacacaagaatggaaaattatatgatgtgcaagtaggacggcaccctatttaactaaaggtgtgtttggttcagttttctgaaccaattcgttgccaaaaaatctaaaatctcacacaaacggtacaacatcagaatagatttttaaaagtttatagatttctcaagttcaattcaaaatcaccatctaccccaaatttttcagattactattattcatgttacaactatcactcttgtagtatctaccattgatagttgttttaatcaaatatattttagctttctcacaatcctcagctcgaaacagattttcatggctcacagttggattcatattttcataaatctataggtgtgaaccaaatagaccctaaaacatcatgttgtaatgttccaaaaaaatcatcacaaaaaacatgtatgcaacacacctaagtgcaacaacactaacctgcaggagcgttggcgtaggctggactcttgtgtgtctgcaatgtggaaacctgcattgtaaatggttaggtaaatgcttcgcttaaaaatggcagtaaatgcttcactaaaaatgcttccacgtgctcatgatcaagtaggttttatgttcaatctgcagttctacacaagtgcgattcattttgatactcatttctatttactttcagagctcgtgctaactgtcataaagtgcaatgcatctatgactgccaattgatattgtgctcctgccataaagtgcactgcatcgtgctaactgtacactaatctgtgaggatctaagaccaatatttgtttacgttttctcctttagtatcctataaaaacaacacgcctagacaacccaaaaaatgtgtcccaataggaatatcagattctgacgctggcagcaatctcgaatgataatattttttccaaacaagcgaggtccctaaatagaagcggcaacagataaaaactaaagataaaaactaaagagtacagatgattggcatcacatcgggaatgaaatatgcctaacatatcaatttgcatattagattatttgctgagaacaataacgaaaacatatttagttgttcatcacaagttaccttagattttgctgttcaaggtcctttgggtcttctttctgctagaacatacaagggtatttcagatttgcaaacaaggaaaagcaagaacttcaatgatacatcattgtaaaaccaagtttccgatttaaataaagatgatgcttgcggtcaacacattcacaaatgtaaatgtgtgaaatcgttcaaacataaggcttatgtggtcatgctcaggtagtatgtacagacctaaaaacaaggtatatgacaacagtaccagccactaaacacacatggttaatcactaaaacaattctccgattaaccaggaaaactatagcagccactagaactatacaggtttctaccagtaattgcttcactaaaaaatgcccccatgtgtaaattttcaggtggtttgtacagacataaaaacaagggtataggactacttcttgtgctaaaataaaagctggcactaaacagtgtatccagttcatcaggaaaacagttttagtgattaatcactaaaacaatacccatggtgcaaattatctgattaaccatgtacataccagtaattgcttcataaaaaatgcccccaatttgctcatgtttaaggaatatgtatagaactaaaaacaagggtatatgataacaataccagccactaaacacacatggttaatcactaaaacaattctctgacaactcctataaaaagatagcaaccaccagaaataaaccgcccacgacatccctaattgtagtcactaaaaactggtagcagtaattggttcactaaaaaatgaccataatcacgaaaactataacagtcaccagaactatataggtttcattagtaattgcttcactaaaaaatgtccccatgtgtaaattttcatgtcgtatgtatagacctaaaaacaagggtatatgactacttgctatgctaaaacaatagctagcactaaacagtgtattcagttaatcatccaaacaattttgtgattaatcactaaaacaatacccatggagcaaattatatgagaataagatctcgtcgttcctattgtgaagaatatactactacctccagtttcaaattacaatttcaaattacaagttgtttagaacatccacaaggtaattgcgaagaatatactaattgctctagtttcaaattacaagttgtttagagaaaaggtgttccttaatagtctagttttagaagctacatccaactggtaaacataaattgcagaaaccttttatgtggaagcctccgtcattgagtctgtcccctttagctgtaagtagttttctaaatattgttagtcaggcttagttgtttgagactctgtttccattcgtgaccatgggaactgtgaaatgtgtagaagatgctcatgctcatgcatatgcatcgaattgttttgtaaagtcatcttaatgctcaaacagtttttttatctgccccagctgtacactgctttctgaattatgtcatttaggcttagctgtccgagataatttcatttgtgatgaaggtaaccggagcatctgtccttttgttttaaacataaatattttgatagcttaacttgtgcgtcattttatcatgtactaacatggtatatagatggcacttagcagtaacattcctgacttatgtgattgtcctgttagaatgcttctgcaatataatgggcttatgctaatctgtttggaatcccatgatgaataacaattatggatgttgggcattttgtatttttatgatgtaggcttaacatattttcttctctgctcagccctgccggtggagacctctatttatagctataatccagccatatctagtgaactaacagatctattcctatctctagtgcttatccccttaacagatttattttcctatctctatttctttgatgttacttgctgcaggtgctatcccccactgatgcattatatgacaatcactcgaagaatcagatgctaattaattgttttatacttgaccattgctaattaagtactccatttttta

SEQ ID NO: 14 - DNA, 1767 bp, Artificial Sequence
  cDNA
atgggttctttggggcttcctgtttcattcagcacaagtaaagtgaacaagaacacatgcaacaagggaaagaaaaaaggaagacaagcaccgctcaaagcagcaaacactcaaatcaatgatgctgtgaggatatgtatcaatactgaagatagagaaaattctgttgaatcattggatgctatggagcaaacgcactcatgcaatttatttgtgacaccactgggtcaaaatgaaccctcccgtgatgacactgacaagaggcttagggaagacagctcttgtgttgaagaacaagaagagtctggctgtagcaccatctactctgctggcaaagcccctggctgtgatgctaaaaatcatctcactgaacttggggcttttgagctttctgataacttggccaactcagcaaaagaagaatactcaattcaagaaaatcaagcttatgaaagtgtgttgctagattctgaagagatgtcaaggaatgactgtgttgatgatgaatctacacattcctgtgttggcatttatcaggatgaaagagtgtccacaaggggagatcaaacatctgaagaaactctatcagtaccccatgattacaatgatgttggcagagaagctagtctaagtttggcagagccatcatctattgatgagcatgcacaaagctctgccaacaacttttactatgactatggtgaatggagggttatctgggatccattctataatcggtattatttttacaacatccagacacaagagtccacatggtgtcctcctgaaggactggaggattttgcatcatattgtagcccagataccactaaagagctagctgaactgggatctcagtgttcaagcatggcaccacaagagaacaatctggctactcatgtcaatcatttagaagcacaggagcaagatcactgcattcatgatttatctgacattcctgttgaaaagccaatatatcaaagtatgataactacctctgacaaagcacagcacactgaaaataagtacagcgattcaacaactactgtgttagagatgaaccaggaagttgctagcaccaaaacgaaaaagagagtaaggagatctcgatcgtatcattcatgccaagacatggcagggaacgtctctaatgacatcatcaagtactgggctcagcggtattcacttttctcactttttgatagtggtataaagatggatgaagtagggtggttttcagttacgccagagccaattgcaaagcatcatgcatctcgtgtgggtgcgggagtaatgattgattgtttcacaggagttggtggaaatgccatccaatttgccaaaaagtgcaagcatgtaattgcagttgatattgatccacaaaagattgattgcgcgcatcataatgcatccatttatggagtaaatgatcacatagatttcattgtaggtgattttatacatatagctcctcatctgaagggagaaactgctttcatgtcgcctccttggggtggccctgactatgccaaagttgatgtttatgatatgaaaagcatgcttattccttgtgatgggtactctctttttaaactcggaaccatgatagcttcaagagtagtgatgtttcttcctcgcaacattgacctaaaccaattggcggacatgtccttgtctgtggatcccccgtgggcagttgaggtcgagaagaacttcctcaacggaaagctgaaagccataacagcttactttgaagaacaggatcgt

SEQ ID NO: 15 - DNA, 1767 bp, Artificial Sequence; identical to SEQ ID NO: 14
  cDNA

SEQ ID NO: 16 - protein, 434 aa, Zea mays
MGSSEEHVFLDPTRICASVSLLAHDLIGRMLNREVSSRPNAKEVLPPMIHREIVRFGYCESSSSKSSSDNSEERDECGIVDALVTTITQIRKMDLEARSLQPSIKAGLLAKLREYKSDLNNVKMGLSAERKKQKLSEIQSGVEEAESLIQKMDLEARSLQPSIKAGLLAKPRDYKSDLNNVKSELKRISAPNASGLISYKKLLFHGLDLWTALSLPQPLGRAALWPPHRTIHQHLQCQQLTGVAGSLAYLAPEVLLGNYSQKVDVWAAGVLLHVLLMGTLPFQGKSIEAIFDVIKTAELDFHNSQWASVSLLAYDLIGRMLNREVSSRPDAEDVLRHPWVLFYTDCLQKAEFSNLWDTNKTAAPMIHREIVRFGYCESSSSKSSSDNSEERDECGIVDALATTITQVRISEPKRSRLFSLPNGLLPPSRNSLRT

SEQ ID NO: 17 - protein, 143 aa, Zea mays
MLNREVSSRPNAKEVLRKFKHPCNLCFIYMILNLSLTFPNGFQHRAPWVLFYTDCPQKAEFSNIWDTNKTAAPMIHREIVRFGYCESSSSKSSSDNSEERDECGIVDALVTTITQVRISEPKRSRLFSLPNGLLPPSRNSLRT

SEQ ID NO: 18 - protein, 162 aa, Zea mays
MEGGRHPSPPPRISRQPPPYPACPSILPPLPPVNVTNPGLVPLVVATLFDERVTELLSVLADAAVGRPGRWSIGEAPWSSSGGTNQAVYARRAPGSSSPPPAPASPPLPSSRADCLARWPGSRALVAPLGTPAFVDRLFWSDFSGSIRREEEAEALRDPIRR

SEQ ID NO: 19 - protein, 87 aa, Zea mays
MDLEARSLQPSIKAGLLAKPRDYKSDLNNVKSELKRISAPNARFGRWTWKQGAYNLALRVSSRGYLRPLPGRLPGRSSWSLEWLILS

SEQ ID NO: 20 - protein, 279 aa, Zea mays
MAHFDELEDKTTDYVDLSVQEFALKQPQCGMAYNYYGNLRLYVVANKAELASSIFEIDKASTKRIGARFCRCLPHTRMEGGRHPSPPPRISRQPQPYPACPSILPQPPPERKKQKLSEIQSGVEEAESLIQKMDLEARSLQPSIKASLLAKLREYKSDLNNVKSELKRISAPNARQATREELLESGMADTLAPEQEQLACAAAALAVGPAYERLQEARNPSEQGCNHDKQIEQAYDDILNSSKHTLASMMELQEALLESNQATKDANGIAALYIVLVLM

SEQ ID NO: 21 - protein, 428 aa, Zea mays
MASYSSRRPCNTCSTKAMAGSVVGEPVVLGQRVTVLTVDGGGVRGLIPGTILAFLEARLQELDGPEARLADYFDYIAGTSTGGLITAMLTAPGKDKRPLYAAKDINHFYMQNCPRIFPQKSRLAAAMSALRKPKYNGKCMRSLIRSILGETRVSETLTNVIIPAFDIRLLQPIIFSTYDAKSTPLKNALLSDVCIGTSAAPTYLPAHYFQTEDANGKEREYNLIDGGVAANNPTMVAMTQITKKMLASKDKAEELYPVKPSNCRRFLVLSIGTGSTSEQGLYTARQCSRWGICRWLRNNGMAPIIDIFMAASSDLVDIHVAAMFQSLHSDGDYLRIQDNSLRGAAATVDAATPENMRTLVGIGERMLAQRVSRVNVETGRYEPVTGEGSNADALGGLARQLSEERRTRLARRVSAINPRGSRCASYDI

SEQ ID NO: 22 - protein, 401 aa, Zea mays
MASYSSRRPCNTCSTKAMAGSVVGEPVVLGQRVTVLTVDGGGVRGLIPGTILAFLEARLQELDGPEARLADYFDYIAGTSTGGLITAMLTAPGKDKRPLYAAKDINHFYMQNCPRIFPQKSRLAAAMSALRKPKYNGKCMRSLIRSILGETRAKSTPLKNALLSDVCIGTSAAPTYLPAHYFQTEDANGKEREYNLIDGGVAANNPTMVAMTQITKKMLASKDKAEELYPVKPSNCRRFLVLSIGTGSTSEQGLYTARQCSRWGICRWLRNNGMAPIIDIFMAASSDLVDIHVAAMFQSLHSDGDYLRIQDNSLRGAAATVDAATPENMRTLVGIGERMLAQRVSRVNVETGRYEPVTGEGSNADALGGLARQLSEERRTRLARRVSAINPRGSRCASYDI

SEQ ID NO: 23 - protein, 380 aa, Zea mays
MASYSSRRPCNTCSTKAMAGSVVGEPVVLGQRVTVLTVDGGGVRGLIPGTILAFLEARLQELDGPEARLADYFDYIAGTSTGGLITAMLTAPGKDKRPLYAAKDINYFYMENCPRIFPQKSRLAAAMSALRKPKYNGKCMRSLIRSILGETRVSETLTNVIIPAFDIRLLQPIIFSTYDAKSTPLKNALLSDVCIGTSAAPTYLPAHYFQTEDANGKEREYNLIDGGVAANNPTMVAMTQITKKMLASKDKAEELYPVNPSNCRRFLVLSIGTGSTSEQGLYTARQCSRWGICRWLRNNGMAPIIDIFMAASSDLVDIHVAAMFQSLHSDGDYLRIQDNSLRGAAATVDAATPENMRTLVGIGERMLAQRVSRVNVETGS

SEQ ID NO: 24 - protein, 589 aa, Zea mays
MGSLGLPVSFSTSKVNKNTCNKGKKKGRQAPLKAANTQINDAVRICINTEDRENSVESLDAMEQTHSCNLFVTPLGQNEPSRDDTDKRLREDSSCVEEQEESGCSTIYSAGKAPGCDAKNHLTELGAFELSDNLANSAKEEYSIQENQAYESVLLDSEEMSRNDCVDDESTHSCVGIYQDERVSTRGDQTSEETLSVPHDYNDVGREASLSLAEPSSIDEHAQSSANNFYYDYGEWRVIWDPFYNRYYFYNIQTQESTWCPPEGLEDFASYCSPDTTKELAELGSQCSSMAPQENNLATHVNHLEAQEQDHCIHDLSDIPVEKPIYQSMITTSDKAQHTENKYSDSTTTVLEMNQEVASTKTKKRVRRSRSYHSCQDMAGNVSNDIIKYWAQRYSLFSLFDSGIKMDEVGWFSVTPEPIAKHHASRVGAGVMIDCFTGVGGNAIQFAKKCKHVIAVDIDPQKIDCAHHNASIYGVNDHIDFIVGDFIHIAPHLKGETAFMSPPWGGPDYAKVDVYDMKSMLIPCDGYSLFKLGTMIASRVVMFLPRNIDLNQLADMSLSVDPPWAVEVEKNFLNGKLKAITAYFEEQDR

SEQ ID NO: 25 - protein, 589 aa, Zea mays; identical to SEQ ID NO: 24

SEQ ID NO: 26 - DNA, 13229 bp, Zea mays
  misc_feature (10689)..(10788): n is a, c, g, or t
ccccgcgcggccaaccctctctaagagggccctggtccttccttttatagtcgtaaggagtggatccaggtgtacaacgggggtgtagcagagtgctacgtgtctagcgggggagagctagcgccctaagtacatgccgatgtggcagccggagagatcttggcacccagcgagtgtgatgtcgtggccatcggaggagcgacggagcctggcggagggacagctgttggagcggttgagtccttgctgacgtcctcctgcttccgtaagagagctgagagccgccgtcgtcacagagcttgcggggcgccatcattgcctatctggcggagctagccagataggacaccggtcttgttctctgcggcccgagtcggctcggggcagggtgatgatggcgcttcctgttgacgtgactggcctgcgccctaggtcgggcgacgtggaggctcctccgaagccgaggtcgagtctgtcttccatggtcgaggccgagcccgagcccctgggtcgggcgaggcggaggtcgttcggcagaggccagggcggagtccgagccctggggtcgggcgaagcggagttcgtcgtcttctggggctgagcccgagtccgagccctgggtcgggcggagcggagttcgccgtcttccgggactttagcccgagtccgagccctgggtcgggcggagcggagttcgccgtcttccggggcttagcccgagtccgagccctgggtcgggcggagcggagttcgccgtcttccgggacttaccccgagtccgagccctggggtcgggcggagcttcctatggtgcctttggcagggcctgactgcccgtcagtctcactctgtcgagtggcactgcagtcggagtggcgcaggcggcgctgtccttctgccaggccggtcagtggagcggcgaagtgacggcggtcacttcggctctgccggagggcgtgtgtcaggataaaggtgtcaggccacctttgcgttaaatgctcctgcgattcggtcggtcggtgcggcgatttagtcagggttgcttcttagcgaaggcaaggcctcgggcgagccggagatgtgtccgccgttggaggggggcctcgggcgagacggaaatcctccggggtcggctgcccttgtccgaggctaggctcgggcgaggcgtgatcgagtcgctcgaatggactgatccttgacttaatcgcacccatcgggcctttgcagctttatgctgatgggggttaccagctgagaattaggcgtcttgagggtacccctaattatggtccccgacaaccacaaacgcccacgtcgtgcgcgtggaggtaaggctatctgcattcatcatactttaaactagttgggtgcccgtgcgttgcaacagatatcatataaattcatgtgttttgctacgcgacacgagggatcggtattattagtagtcatttttctattggacctagtgaggtactcgtacgttgctacggagatcatataaatccatgtgttttgctacgcgacacgagggatcggtattattagaagtcattttctattggacctagtgaggtacctgtatgtgcccgtacgttaccacgagagttaaaacctagtataaaacataaatacagaatgacaaacatcattatgatatacaaattcgtgtaacaaaatatcactgtagcactaatattcaataaaatgtagcaactcactgctcactaatgatgtgtccagggtaagtgggtaaagcacggtagacgtcttcttttgacttagtacaatgctcgtgtgttgagacggtgcacaattattcgataaaatgtttgagcacaagtgcacaacgattacataaaattgaaaaatacttatattaacaaagtctaattgtctcaaattctttttgccaacaaccaattcactgtgttgcgatgatacacaataatatttcatgaatgactcaggcaatccacctaagtgggtaacccaaaagcacaccaatgtgatgcctacacgtgaacatctaacctctattactacaatagtcttgttggaaatttacaactcatctagaatttcaaaatactcaaaattatttagactctctctaaaccggagcatacaaaatagatcaggcagttttaacggaaacatgtatgactctcaccatcctgtgcagcgctgctcgaataccagaaagtcccagctcagccaatactgcatcaagttctgctagttcctttttttcatctcctttttagacaactgtctttctgtctctttgggtggcgcagctagggcccacaactgtcttgatagcaggttcggctggggcatctttcggatcatgctttaggttcatcctcagctccatcatcaacctcaaaatcaagatccttgtcatcactctcaatgtcctgcaacatatatagaagtacatctaagaacactatcagagaggctaactataatgacaatcagccaaacatgctccatccccctcgagatgagtaaattatacttccacttaatagtttagttttgatgcaaaaattatgacaaaaaacaagtagaacaataaccagagtttgctatgacaaacatgcagcacctgtcatgtataaccatttccaaatcacttgcttacccaagatatagaaaaacttggaacaagtccctatccaaggtacatattttttatttttgtttagcaggtggtcagctctgaaaattttctgtcaaggtgaagtttgccttatgacttgctcatagcagggtctgctttgaactcctccactgggaatgcaatgtcgtgatcccacagaccgatcaaatgggattcaaatttaggctgtgctatatcgcgctctgaatctagtgataatgcgtctatccttggtttcttgggagaatgttgcatgatctctgggtagtcatctaagcttggaggtgaatcagaaagtttctgaccctcagaagctttaattgatccaccaagcttttgttgctcctcaatgatcatctgcaagtatattccttgtgctttaattgttagttgcagttgtctttgaacctgaaaacataacttatttagacaagcaaaagaaagttggcaaggaaaatttagattgatcttgaagctaaaaaggactcataaactacaagcaataagacaaaacaggagaactgccaacaatagattattgacaactaagcattactacaaccatgagaagaaaccactgttaggtgtaacgtgacagttaataagtgaatattgagaatgggccaaaatatcagcttgtagaagtagccccaactaagtaggacttctggtcatagtaggattgtcggtaaactaaaatgatgtaaaaaacagaaatctctactacttattaagtaagcaatagtagtctgcctccctcgttctgccgttctgccatccatcgatctggaccgttcatatcgcatcgtgcgtctgcgtctcccacactctatctccctccaccgcacgaccacccaatccctaaccttcccccacacgttcctctctctctcgcgttgcccgccccctgcccctgccgcgatagaatgcctcgcggcctccaccgccgacgcggcctccaccgcttcccttcctccctttgcctccaccgcccctcccccaacgtcgtcgccaccgccgctctagggcctcgacgcaggcagcttgggaaccgccctcggcctcggtgtcgcacggccccacgaggaccgaccttgccgcatggcggttgtggaggcgtgcgaccccgcaaggatcgacatctcgtccaagacagcagccccctcagagcggacgacgcagcttatctctggtggaaggcacgtagccacgcccccactccctcctcgtgctcccgccgacgcctgcctcgcgctcctcgtcgaccgtctctccctctcctccgtcgttgcatctcgcctctcgcgcacgcacaaaggtgagtctcccctcccccgactcacccctctaggtctctgattcttctcatcggcgagcaaggacggaggagctggcggaggagctgtcgaatataacctaattatgtcggtctcgggtgggatttggctattttgggcgccatggcctaggtgagcgtacagatctggttctgcattttgttttcttatctgtcaatcatgttttttcatattactgcaggtgggtctgattaaatattacagacatgttttgcttcgaagccctacacctgtccatctaattttaggaactgacgattgacacagctttgttgtggcgctatttagtataagttatagaaatcggatctttggctctcatctgcttgtagttgcaacattgaggtagaacctgggtgggtctgattgctcattgctgtgatatatgtctggaaaagcagagttatagtttggaaactagcgcgtagtacatgtcggtttctttaagtaattgcttatgctctgttgttttgatttccagatgccccaaatgtgctgaacttaagctatcgcgtgagaacacaactttctggtaagtggcaagctcctccgtttcttattttaccgcattggaagttggaacaccatgatagctctcaggacgaatgagtatcagctaattttattgttttaacaatagagcataaaaccttatgcatattttaaaggttcatgtatcatttagttatggccttatgaggaagcttcatcatcatatctgtagataccttgattcgtggggatggtaattttttgtattcttgttcttttgatttttgaaggaaacacatcttataatacgatagcacccattggaagtcctcgcatacagtgcagggtagaattatgcttcatgtgttgccccttcaccacgatatgccaaattgaatgtagtttcatcagttatgctcaattatggatgttcagaggcatccaatttcagtgtgtactgcaatacttgggtccacctatagttgatagatgttctgtattttgttttcttataaattagatttggcttgcattatattgttctcttttggaacagagtcactctccgacagctcatcgccgcctgcttcgaccgcctgtacacaaggtttaagaagcgctctgcgaacttccacggccgcgccgtgctgcttctagctatttacctttttctatgatgcaaatgtttatatgcatactatgttacttgagaaacattaaagtacttgatgtacctaaacacattttgtttagtgatgtatagtgatatagcattattgtctatattaatatttatattgctggtagcttctactttaattgatctcaatggggcatttgggtggctagcaattcacattgataatttaaaagtgaatttcaggtgtacatttgatggcctccgatatggtgctgccttcaattctctacaatgcgcgagaatgctgctcaggagggtattaatggctcaacacagatgacctcctcggagtcatgtttctaattatctacactatgattctccttctgttgataaaatattgttttattgtgctgtgagctaatgataacagtgatggtaagtaaatatggtccatgcatattctcatcatagatggctgaaaaactccgagtgctgctacgctaccagagtcttcatgtgcatacttacttcaagaactcaaggtacatagttttctcaacagaagaatatgtatctgtttgattccagctgaattgcttactaaactcagtgtgtcactttaaatgatatgggatgaagttgggcaagaccaaagtgaaagtgggagaatacccgaagaacttcttgttggacgaacttggagaaaccaatactaaaactcagtgtcaaccgcttgcaacaggcaatttaggtcgatgtgctcgcacgctgtgtgaccatgtctgagcactccccacccacccaatcgcttcccacgtcatgccgccacgtcgagaatttgtacacaactcaggttgcccattttactctgttattgaacctcgcttttctgtagacccaggtatgctagaagtaggtaatggtagcatgaccttagcagagtatcgctcacattttagcatttgggttgtcatgaaggtaagttttcactgagattggaccgatgttgtgtcatcatattttgagtaaagggtttgaccgaagaattttgaaaaataaaagactgtagttcattgaaggtgataactggtatgcaagtattactattaatgattctccacttactgatattacatttggataagaggaaggagatatcctaattctaatgggttaactgctagcagttccttatgtactgttatgcttcaggcccctttattaattgcctcatgtggaaagagggtgtgatgatcttttgttgtttttgtagcgagaagctcaaagaaggggaagacatctacatctatcagtaagtgatccagtttagtagatgaatcaccgctatgggtgtttttctattcttgaataggcatgtggttctattgatggttgtttgatgtttggtatattgtgttctgactgtaggggtgacaaatccttttgcagcatggagtgcagagaaaatttcatggtagacgagatggaaggtgagccagagagtatgtataatcagatcaattttagactttttttcactaaccacttatccatagcacacttgtgtttatttgagatatgtgtcgtcattttgtgttcatcggctattgctatgaagatgaccacagggttaattcttgtttatgagttcatcctctagaatgtattgggttgtcgccaagaaaaaacacacgaagacataaattcaaataatttctggtgctgtggagtattcataattgtgtgcttttgttgaatccttcatgtaccataattcttactgcttgcaagcccttttagaatgtgactttaggatgtagaatttggtgaaaggagacaagaaattattctctaaactactatttttataggcaagggaggctggaagcaccttttttgcatgggagctgcatggagagaacttattggtagaaaacaaactttgaccagattcttgaatgtgccaagggaaaaaggtattaattgggaccttctatttatacaagggaaaaaggtattttttatacaattgctcttccttctcatgtatggcaacttcctgttttgtagagattgagcgcccttcctcactgtttgaactttactcatcctcatgaaactgtgatgctacctgtaggagcggtttgttcaaggagggaatgacttttagaccctaataacttgtctacacttaagataaaaattgttgtcattgctatggttacctcctttagtgtcgtaaactcagaataatcatagatccctttgttgcttacacattattcatgttctacaagctattgagattttgactagccgctacattttagtgcaggttttcataatttcttacctttatatctacattttagatttcctcccttttgacactacattttagccgctcactcggaagctttccatccctgctggagtactcagcccataaaggtaaatgcatgcctttacctgcctgaaatgcattgtctttcttttcaaccgtgaatgtgaattggatccatcattcatgtgcacacacaaggccggtttgaatttggaatgcactgttgttctgcctgtgatccacttggtggtttttatttgcgttcacatattaaaaaatatattataccctgattctgagtcaaactttggttagacctggatttgttgattagtttccgttgttgtgatctgttgaacaaactataggttaggtgagttatcagattcttagatctgtcctgtacggttgtgatctgttgaacaaactataggttaggtgagttatcagattcttagatctgtcttgtacgtctgatctctaccatgttacaaacatctgaaagttaataataatcactactacattcacacctatcttgtatggatttgctgttgaaattgcagaatgcttcccaacttgtgcatttttattacatccccacaacttcatcgtatagtccagacatcctttgtttgtgtagcaaaatagatgtgcaattgtttcattgtaacaatgtcctgtatattaacctcggcggctctggtgctttctgcaggcttctcattcttatttgcatggcctgtaactgctgcacagcgcgctacggctggcgtagcggcagcaactgctggtatgaacaggatccgtccaccctcattagcgacgatgaagtgacacccaattctaggcgcggacgtacgatggcgccctcgcgcgggatatcgggctgagtgatgagacgctgctgccattggggttccaggcgcgcctgaccgctcccactcctaggcccggcatgtctctccgacgctacctaccggtgctggtgaaacgcaaacttaaaatcgtgcattgcaagatgttgccttctctttatgtctcctctactctacgcctacgagctttctttgtttataactttttctgtggtttcgctttcaacaagctcaagcggtcaacagatcaacttagacaaaatgcagatgcagtggaaatattaaggaagaccagattccctcatgttcatggagcaggtgaaaagaagtcaccagagacaattctggatcatgagactatgagaggactttggcaacaaatgttcggtttggacttctctgggtggttctatgatactttataatttcttttggcttatgtgtcatttcagaagatatgaaaatagctaagcattgtcaataatattagcttccttgtttcttgttaacctaagatgactgccctatttcacttgttttttctagctgtggtagtaggtcattagagtagttcccttcaatcgtagcactcagccatgttgtaaatggtttacttctattgtgaatcgtgtttttcttttttaatggtggggttagtggaaaatctggacgtatccgcgaatggtggagaagcacacaaaacaacaattatatgcaaaaactaaactatgttttctttctttctatggtatatgaatttagtaccttgataatcacaatgattagagtctgtttgtatttatattaaaacataactgcttaggaggtgtatgaggaggataacgagatgtgcagtgcgcgcaacagtaagcagactaccatgacttggttgctcttcaagtgtgcaagtgtgtctatggattgtatggttctttggtttttgttgttcgctaaggtgcaaagtaggaagaaaatacggccctgaccctgcaagtggggaatgtatcgtttttgctggaactgaaatatgcggtgttcttttttatgcactaatattttgttgaatattttgtataccgttgcaacgcacgggcatctacctagtaaattaatagttttcaataaaagacctcgagtttctcatgtagtcgcttctgaacctccatttacatctttagtgccttaaaaatcgtgccaatgtttccatatatcaaatcacggtgatcaacaattaaacaaaataactcttaaccaaaaaaatggaagtgtcacgcactcatgaactacagatgtcaatagctaacatataaacaggctcaagccttccttcaaggataccaggttgttctaagcagcatctctatatttagagaggaagacttgtctcgattcatctcttcctgagaccccactcatgtgggtagttctaccttttttatgaatacagatgcaacatcaacatataaacaggctcatgcctcagatactactctcaattggtctactgaaattctattgcatttatgacgaatgcagttacagatttaaaagtaaaggacgagtacagctgcatgatgaaaagtaaacagaacggtaactgcaaatttacttcagacatgctgctgctttgatgagatcggaacagggttgttgctcacaatctgtggatttaaagcctgcaacacatgtcacaatttaatcatgaggttcactaagacaacattacacaaaagaggtgttggtactgagaacataaaagatcatgtcatccttgtctgaaaggaagtgcattccaactaagaacaaagatcactgcttctcaatgaagcaaggctacgacatgatgcatatttagctcaaattacccaagcaagtgtttattaaaataaaagcatgcatcttagacatcagcaataggttatctaagacgtcaatgcatatttagcccagttttagacaacaatgcatatttagctaaaatattaaacatgcaatgcctctttagctcaaatttcagaccacagtattaaccggtggtgctacacttgaagaacaagcttatctggagaagcagcccacatccagtcctgaaggcaaatcagatgtttgaacaaaatcagtgcttagccaaatctagaaaccacaaccactcgaacgctgactcagatggtagagccatcacaccaatggtgctaccatcagtaaaataatagaatcaatttgtttttccttactgatacagtacccttcgaataattgtttataagcaattgaacttgctgcccaatgtattatagtcttggtcnnnnnnnnnnnnnnnnnnnnnnnnnnnnnnnnnnnnnnnnnnnnnnnnnnnnnnnnnnnnnnnnnnnnnnnnnnnnnnnnnnnnnnnnnnnnnnnnnnnnttagagacatatagagtagtatagataaggataatggacagtagtacttgaagttaatacataaaacttgcagctaataaacaaacatagtactattttagttaacatacaacaattttccagctcttctttgcacttatagcatttttagtacctacacacaacctgaactgaacaccatcaagaacagtactgcatttggaagtttgaataaaaatggtgtccaattaacagttttctaatattgtaacttaattattgaatggtgcaatagggtgttcacttgttgaattggttgataatcttgtgtgggctttaaatataacattgttagtgaatgctaaataattctgcactcttggaatggtcaagctgagaatgagccagagattaactggtgcgaacctgggaagcctgcagggatggaggtccttcttgggagtaaggatgggttcttgacgaagaagattaagagctatagcacatgccgaagtgatcctacaaagccacgtgcattgcaatgcctttcaccactgatagcaggtcatgtaagatacatcatttaaccatctggatatgtgttaatgttagacaactaatttataaaattttcgattcaggtgggcaatggaattgtttgttgaatgagagtaatgtttattattggtaaagtatcacaattcagtctgattcaggtgggcatggtaaaatgaagtgcatctgccaaaaagtaaggtaagtaactaagtatcttttggatgtttggaggatcagatgttgttgcagaatgtttattgactaattgcaagtcaaatgaattaaaggggaaaacagataagcactaagatttttatatgaaagctgtgtgagtcaacctgctaagagctctaaatgtcctgtcccagaagtagtggcggagccagcccaaatttgaagcctatcgactcagaaaattcatccatgccaaccaaacaaatagaataattaccttatctgttgcacgggtgtgaaggagctggagatgcagatcaggtgtcacaaattctataaccaaattgcataatgcataagcaatcaaacaatacacccctaattctttaggctaaacgaactgcactaagcctatgtttcagatttcaagattactattggattgtgttcatcacaccaataggttaagtaccaacatgctaatcaataagaacagtaaaggggcattacctacaacaaatgttacgtctaaatagaactaacttggaggcaatgtaagctctgaatgtccgaaacattgaaacaaagtctgaactctgaaattgtctccctaatcctcacctcatcccatctgtgtcgatggatggtgggtgcctcgcctgagctgttgtgtggtgccgcggacgaggtgagcgcttgtgtagaatgaagatggggtcgcagagcgacgtggccgacggcggaccgatgatggagagggtactttttactttcattaacagatcatcaagcaaaataaaatagtaatgagcaattgagcccagatcacatttgtaatcatctagcatgtaagcactattttttaatttgatacccctcattcagagtttttgcacaaacttagaactggaggctgaaagtaagcaaattgacttcatcttttagtttgatgaagatcaaatgaatttaaaagcttgagaagatgaaaagatctcatatgtatgaccaagagatgatagcaaatggcttcaagccaataaagtcacgagagatgaaagcaaataggttcacatgcaggatacaacagaaagttatgtatacaggaacaaatgctaatagaactatgcatttatcatattttagaaactgtagcccttgttcatcctacccccaatgagtattcctatcagtacacatgtaggctagcatttttttagttgtaatacttgcttagctacagatcactggctagctgaaaaaaacctaagtagcaacagtggaacagtttgagtatagctgtatgaaaaaggctatctgaataatagcaatatttggattcatgttcatttcaagaacttcaccattgggaaaactccaacggtactaccatttgattgctgcaatgtttgtaatgataaagagatctcacttactcacttgtggtaccatagaaacctgcaaaaaagaggaaaataatataaattggtgtaaaaattaaggaattcatagtacaaatatgatcgactttataggaccacccttttgttaaatttttcagtgtcaacaggaaggtgtgattcaggcctttgtggatcaagtcagcacagaaccttggcttcttcattcggtagaatgatgacaagactaccgaatgatgacaagacttttaaaaatatcctgttgaaaatgcatttaccatgtcagctgtgttaccaagacgggtaattact

SEQ ID NO: 27 - DNA, 1515 bp, Artificial Sequence
  cDNA
atggcggttgtggaggcgtgcgaccccgcaaggatcgacatctcgtccaagacagcagccccctcagagcggacgacgcagcttatctctggtggaaggcacgtagccacgcccccactccctcctcgtgctcccgccgacgcctgcctcgcgctcctcgtcgaccgtctctccctctcctccgtcgttgcatctcgcctctcgcgcacgcacaaagatgccccaaatgtgctgaacttaagctatcgcgtgagaacacaactttctgcttctactttaattgatctcaatggggcatttgggtggctagcaattcacattgataatttaaaagtgaatttcaggtgtacatttgatggcctccgatatggtgctgccttcaattctctacaatgcgcgagaatgctgctcaggaggatggctgaaaaactccgagtgctgctacgctaccagagtcttcatgtgcatacttacttcaagaactcaagcgagaagctcaaagaaggggaagacatctacatctatcagggtgacaaatccttttgcagcatggagtgcagagaaaatttcatggtagacgagatggaaggcaagggaggctggaagcaccttttttgcatgggagctgcatggagagaacttattggtagaaaacaaactttgaccagattcttgaatgtgccaagggaaaaaggtattaattgggaccttctatttatacaagggaaaaaggcgcggacgtacgatggcgccctcgcgcgggatatcgggctgagtgatgagacgctgctgccattggggttccaggcgcgcctgaccgctcccactcctaggcccggcatgtctctccgacgctacctaccggtgctggtgaaacgcaaacttaaaatcgtgcattgcaagatgttgccttctctttatgtctcctctactctacgcctacgagctttctttgtttataactttttctgtggtttcgctttcaacaagctcaagcggtcaacagatcaacttagacaaaatgcagatgcagtggaaatattaaggaagaccagattccctcatgttcatggagcaggtgaaaagaagtcaccagagacaattctggatcatgagactatgagaggactttggcaacaaatgttcggtttggacttctctgggtggttctatgatactttataatttcttttggcttatgtgtcatttcagaagatatgaaaatagctaagcattgtcaataatattagcttccttgtttcttgttaacctaagatgactgccctatttcacttgttttttctagctgtggtagtaggtcattagagtagttcccttcaatcgtagcactcagccatgttgtaaatggtttacttctattgtgaatcgtgtttttcttttttaatggtggggttagtggaaaatctggacgtatccgcgaatggtggagaagcacacaaaacaacaattatatgcaaaaactaaactatgttttctttctttctatggtatatg

SEQ ID NO: 28 - DNA, 2229 bp, Artificial Sequence
  cDNA
attgatctcaatggggcatttgggtggctagcaattcacattgataatttaaaagtgaatttcaggtgtacatttgatggcctccgatatggtgctgccttcaattctctacaatgcgcgagaatgctgctcaggagggtattaatggctcaacacagatgacctcctcggagtcatgtttctaattatctacactatgattctccttctgttgataaaatattgttttattgtgctgtgagctaatgataacagtgatggtaagtaaatatggtccatgcatattctcatcatagatggctgaaaaactccgagtgctgctacgctaccagagtcttcatgtgcatacttacttcaagaactcaagttgggcaagaccaaagtgaaagtgggagaatacccgaagaacttcttgttggacgaacttggagaaaccaatactaaaactcagtgtcaaccgcttgcaacaggcaatttaggtcgatgtgctcgcacgctgtgtgaccatgtctgagcactccccacccacccaatcgcttcccacgtcatgccgccacgtcgagaatttgtacacaactcaggttgcccattttactctgttattgaacctcgcttttctgtagacccaggtatgctagaagtaggtaatggtagcatgaccttagcagagtatcgctcacattttagcatttgggttgtcatgaaggtaagttttcactgagattggaccgatgttgtgtcatcatattttgagtaaagggtttgaccgaagaattttgaaaaataaaagactgtagttcattgaaggtgataactggtatgcaagtattactattaatgattctccacttactgatattacatttggataagaggaaggagatatcctaattctaatgggttaactgctagcagttccttatgtactgttatgcttcaggcccctttattaattgcctcatgtggaaagagggtgtgatgatcttttgttgtttttgtagcgagaagctcaaagaaggggaagacatctacatctatcagggtgacaaatccttttgcagcatggagtgcagagaaaatttcatggtagacgagatggaaggcaagggaggctggaagcaccttttttgcatgggagctgcatggagagaacttattggtagaaaacaaactttgaccagattcttgaatgtgccaagggaaaaaggtattaattgggaccttctatttatacaagggaaaaaggtattttttatacaattgctcttccttctcatgtatggcaacttcctgttttgtagagattgagcgcccttcctcactgtttgaactttactcatcctcatgaaactgtgatgctacctgtaggagcggtttgttcaaggagggaatgacttttagaccctaataacttgtctacacttaagataaaaattgttgtcattgctatggttacctcctttagtgtcgtaaactcagaataatcatagatccctttgttgcttacacattattcatgttctacaagctattgagattttgactagccgctacattttagtgcaggttttcataatttcttacctttatatctacattttagatttcctcccttttgacactacattttagccgctcactcggaagctttccatccctgctggagtactcagcccataaaggcttctcattcttatttgcatggcctgtaactgctgcacagcgcgctacggctggcgtagcggcagcaactgctggtatgaacaggatccgtccaccctcattagcgacgatgaagtgacacccaattctaggcgcggacgtacgatggcgccctcgcgcgggatatcgggctgagtgatgagacgctgctgccattggggttccaggcgcgcctgaccgctcccactcctaggcccggcatgtctctccgacgctacctaccggtgctggtgaaacgcaaacttaaaatcgtgcattgcaagatgttgccttctctttatgtctcctctactctacgcctacgagctttctttgtttataactttttctgtggtttcgctttcaacaagctcaagcggtcaacagatcaacttagacaaaatgcagatgcagtggaaatattaaggaagaccagattccctcatgttcatggagcaggtgaaaagaagtcaccagagacaattctggatcatgagactatgagaggactttggcaacaaatgttcg

SEQ ID NO: 29 - DNA, 579 bp, Artificial Sequence
  cDNA
aagttttcactgagattggaccgatgttgtgtcatcatattttgagtaaagggtttgaccgaagaattttgaaaaataaaagactgtagttcattgaaggtgataactggtatgcaagtattactattaatgattctccacttactgatattacatttggataagaggaaggagatatcctaattctaatgggttaactgctagcagttccttatgtactgttatgcttcaggcccctttattaattgcctcatgtggaaagagggtgtgatgatcttttgttgtttttgtagcgagaagctcaaagaaggggaagacatctacatctatcagggtgacaaatccttttgcagcatggagtgcagagaaaatttcatggtagacgagatggaaggcaagggaggctggaagcaccttttttgcatgggagctgcatggagagaacttattggtagaaaacaaactttgaccagattcttgaatgtgccaagggaaaaaggtattaattgggaccttctatttatacaagggaaaaaggtattttttatacaattgctcttccttctcatgtatggcaac

SEQ ID NO: 30 - DNA, 2512 bp, Zea mays
cccgctacctgttcaccgcgcgccagcgaaacctccgcacgcccactgcccatctgttccccgtgcgccagcgaaacatccgcacgcccgcggcccgcctgttccccgcgcatcccgctgcacgacttctgctaccgcaacggccacccacgcacgcccgcctgttcaccgcgcatcccgctgacctccccttcacgctcgcacacgctccgttcccccaccccaccgcaatccccgacgctataagagcggtaaccaactccatctccctggtgccacgcattgttgagttcttaaggtgcgtttcgttgaggacttgttcatttttgttggtcatgtattccattttactgctctaccattttgtggaataaagggaggaatgttttcactagaagagttcatcaatcttatgttggtttcttggatcagttttgctctatggctaaatggtcgaattgagcctatttcattataaagttagcgagcgaataattgttcagcctcttcctagaactcattaccagtagaatcagttactaactgcttttctttttcttggattagaatggctggggctatctctcaccatgcgctagcattttcacaatcccactggtgcagtgcgaagaactctagattcggaaagaggacgggcaatgctcgcctggtttatctaaaaggaagatgtggttcaggcagcagaaaactgggtttgatgtgggcctcgagctcgcagtcttctgtcatggagccgacgcacctaccatctgatggcaacagcagccacaccccaaaaaaatcaagtaattttaacgacctcctatggtggttatttgtttttaatttgagaaaactatccatttgacacatttaactttgggcttctcagaatttgggggcatataataagatctgctaatctgttatctctatgtcgttgtaggtgaaagcgctcttatattgatttggcatggtgaatccctgtggaacgagaaaaatctatttcctggctgcatcgatgtacccctgacaccgaagggtgttgaggaggccattgaggcaggtaaaaggatatgcaatatcccaatcgatgtgatatatacttcatcactgatttgtgctcagatgaccgcaatgcttgccatgatgcagcatcgacgcaagaaggtttgtgtctttcctttgaaattccagtaatttcttctagcatttgtatgaacttgccggagaaatcatgctttgctggtgatatatgtatttatagatcctagttatcacgcataatgagagtgaacaagctcacaggtggagtcagatatacagtgaggagacaatgaaacagtccattcctgtcatcacagcttggcaattgaatgaacggatgtaatactttctccatactctttgatttgctaattactccctctgtctcaaaatagtattaattttagctcttgatttttatgtctatattcaaatagatgatgataaatctagattctagacacaaatataaaacatatacatcaagtattatatgaatctattaatttactaagaccaattttaatttgggacagagggagtatacgattataatagttgtttgactgtgcttctctttaaatatcccttgacatttctaggtatggtgagctacaaggccttaacaagcaagaaactgtagatcgatttggcaaagaacaagttcatgagtggcgccgcagttatgatattcctccgccaaatggagaaagtctagagaagtgtgctgagagagctgttgcttatttcaaagatcaggcacatctagcaaggccactttacactaattgaaagatacactttttacttgggttattggtcttgctgcagtattggtatgcatgctaaaggttattcttgaatcgatgaattcctctactatgggatgcagaaatgcatgtgcttagttttctttctattgtgctagctcatatcaaatttataacctgaattttttatttatgttcgactctaaaaaacagttttttctagctcgatttgacctatagtaatttttccgtaatagattattccacaacttgtggctggaaaacatgtgatggttgctgcacatgggaattcacttcgttcaattataatgcatctggacaaattaacttctcagaaggtaattcactgtcgtttttgtctttccatcaaaaaggactcggctaaacagaacatgtagcattatgttaagtttgggagtgagcctttcgtcccttcaggtaataagccttgagctgtctactggcattcccatgctttacatattcaaagagggaaagtttattcgacgtgggactccagtaggaccttcggaggccagtgtttatgcttataccagggtaagattctttcccccacatgttctaccataggacgatactccagtttacaaaccttatctgtacagaccaaacgatttgctgagcacattacatttcagaacaaattggcctag

SEQ ID NO: 31 - DNA, 1005 bp, Artificial Sequence
  cDNA
atggctggggctatctctcaccatgcgctagcattttcacaatcccactggtgcagtgcgaagaactctagattcggaaagaggacgggcaatgctcgcctggtttatctaaaaggaagatgtggttcaggcagcagaaaactgggtttgatgtgggcctcgagctcgcagtcttctgtcatggagccgacgcacctaccatctgatggcaacagcagccacaccccaaaaaaatcaagtgaaagcgctcttatattgatttggcatggtgaatccctgtggaacgagaaaaatctatttcctggctgcatcgatgtacccctgacaccgaagggtgttgaggaggccattgaggcaggtaaaaggatatgcaatatcccaatcgatgtgatatatacttcatcactgatttgtgctcagatgaccgcaatgcttgccatgatgcagcatcgacgcaagaagatcctagttatcacgcataatgagagtgaacaagctcacaggtggagtcagatatacagtgaggagacaatgaaacagtccattcctgtcatcacagcttggcaattgaatgaacggatgtatggtgagctacaaggccttaacaagcaagaaactgtagatcgatttggcaaagaacaagttcatgagtggcgccgcagttatgatattcctccgccaaatggagaaagtctagagaagtgtgctgagagagctgttgcttatttcaaagatcagattattccacaacttgtggctggaaaacatgtgatggttgctgcacatgggaattcacttcgttcaattataatgcatctggacaaattaacttctcagaaggtaataagccttgagctgtctactggcattcccatgctttacatattcaaagagggaaagtttattcgacgtgggactccagtaggaccttcggaggccagtgtttatgcttataccaggaccaaacgatttgctgagcacattacatttcagaacaaattggcc

SEQ ID NO: 32 - protein, 394 aa, Zea mays
MAVVEACDPARIDISSKTAAPSERTTQLISGGRHVATPPLPPRAPADACLALLVDRLSLSSVVASRLSRTHKDAPNVLNLSYRVRTQLSASTLIDLNGAFGWLAIHIDNLKVNFRCTFDGLRYGAAFNSLQCARMLLRRMAEKLRVLLRYQSLHVHTYFKNSSEKLKEGEDIYIYQGDKSFCSMECRENFMVDEMEGKGGWKHLFCMGAAWRELIGRKQTLTRFLNVPREKGINWDLLFIQGKKARTYDGALARDIGLSDETLLPLGFQARLTAPTPRPGMSLRRYLPVLVKRKLKIVHCKMLPSLYVSSTLRLRAFFVYNFFCGFAFNKLKRSTDQLRQNADAVEILRKTRFPHVHGAGEKKSPETILDHETMRGLWQQMFGLDFSGWFYDTL

SEQ ID NO: 33 - protein, 128 aa, Zea mays
MYCYASGPFINCLMWKEGVMIFCCFCSEKLKEGEDIYIYQGDKSFCSMECRENFMVDEMEGKGGWKHLFCMGAAWRELIGRKQTLTRFLNVPREKGINWDLLFIQGKKVFFIQLLFLLMYGNFLFCRD

SEQ ID NO: 34 - protein, 335 aa, Zea mays
MAGAISHHALAFSQSHWCSAKNSRFGKRTGNARLVYLKGRCGSGSRKLGLMWASSSQSSVMEPTHLPSDGNSSHTPKKSSESALILIWHGESLWNEKNLFPGCIDVPLTPKGVEEAIEAGKRICNIPIDVIYTSSLICAQMTAMLAMMQHRRKKILVITHNESEQAHRWSQIYSEETMKQSIPVITAWQLNERMYGELQGLNKQETVDRFGKEQVHEWRRSYDIPPPNGESLEKCAERAVAYFKDQIIPQLVAGKHVMVAAHGNSLRSIIMHLDKLTSQKVISLELSTGIPMLYIFKEGKFIRRGTPVGPSEASVYAYTRTKRFAEHITFQNKLA

SEQ ID NO: 35 - DNA, 637 bp, Artificial Sequence
  cDNA
gctacgtgccttccaccagagataagctgcgtcgtccgctctgagggggctgctgtcttggacgagatgtcgatccttgcggggtcgcacgcctccacaaccgccatgcggcaaggttcaaagacaactgcaactaacaattaaagcacaaggaatatacttgcagatgatcattgaggagcaacaaaagcttggtggatcaattaaagcttctgagggacattgagagtgatgacaaggatcttgattttgaggttgatgatggagctgaggatgaacctaaagcatgatccgaaagatgccccagccgaacctgctatcaagacagttgtggccctagctgcgccacccaaagagacagaaagacagttgtctaaaaaggagatgaaaaaaaggaactagcagaacttgatgcagtattggctgagctgggactttctggtattcgagcagcgctgcacaggatggtgagagtcatacatgtttccgttaaaactgcctgatctattttgtatgctccggtttagagagagtctaaataattttgagtattttgaaattctagatgagttgtaaatttccaacaagactattgtagtaatagaggttagatgttcacgtgtaggcatcacattgg

SEQ ID NO: 36 - DNA, 691 bp, Artificial Sequence
  cDNA
tatagggagagcggccgccagatcttccggatggctcgagtttttcagcaagatgctacgtgccttccaccagagataagctgcgtcgtccgctctgagggggctgctgtcttggacgagatgtcgatccttgcggggtcgcacgcctccacaaccgccatgcggcaaggttcaaagacaactgcaactaacaattaaagcacaaggaatatacttgcagatgatcattgaggagcaacaaaagcttggtggatcaattaaagcttctgagggacattgagagtgatgacaaggatcttgattttgaggttgatgatggagctgaggatgaacctaaagcatgatccgaaagatgccccagccgaacctgctatcaagacagttgtggccctagctgcgccacccaaagagacagaaagacagttgtctaaaaaggagatgaaaaaaaggaactagcagaacttgatgcagtattggctgagctgggactttctggtattcgagcagcgctgcacaggatggtgagagtcatacatgtttccgttaaaactgcctgatctattttgtatgctccggtttagagagagtctaaataattttgagtattttgaaattctagatgagttgtaaatttccaacaagactattgtagtaatagaggttagatgttcacgtgtaggcatcacattgg

SEQ ID NO: 37 - DNA, 2146 bp, Artificial Sequence
  cDNA
atgagaagaatcagagacctagaggggtgagtcgggggaggggagactcacctttgtgcgtgcgcgagaggcgagatgcaacgacggaggagagggagagacggtcgacgaggagcgcgaggcaggcgtcggcgggagcacgaggagggagtgggggcgtggctacgtgccttccaccagagataagctgcgtcgtccgctctgagggggctgctgtcttggacgagatgtcgatccttgcggggtcgcacgcctccacaaccgccatgcggcaaggtcggtcctcgtggggccgtgcgacaccgaggccgagggcggttcccaagctgcctgcgtcgaggccctagagcggcggtggcgacgacgttgggggaggggcggtggaggcaaagggaggaagggaagcggtggaggccgcgtcggcggtggaggccgcgaggcattctatcgcggcaggggcagggggcgggcaacgcgagagagagaggaacgtgtgggggaaggttagggattgggtggtcgtgcggtggagggagatagagtgtgggagacgcagacgcacgatgcgatatgaacggtccagatcgatggatggcagaacggcagaacgagggaggcagactactattgcttacttaataagtagtagagatttctgttttttacatcattttagtttaccgacaatcctactatgaccagaagtcctacttagttggggctacttctacaagctgatattttggcccattctcaatattcacttattaactgtcacgttacacctaacagtggtttcttctcatggttgtagtaatgcttagttgtcaataatctattgttggcagttctcctgttttgtcttattgcttgtagtttatgagtcctttttagcttcaagatcaatctaaattttccttgccaactttcttttgcttgtctaaataagttatgttttcaggttcaaagacaactgcaactaacaattaaagcacaaggaatatacttgcagatgatcattgaggagcaacaaaagcttggtggatcaattaaagcttctgagggtcagaaactttctgattcacctccaagcttagatgactacccagagatcatgcaacattctcccaagaaaccaaggatagacgcattatcactagattcagagcgcgatatagcacagcctaaatttgaatcccatttgatcggtctgtgggatcacgacattgcattcccagtggaggagttcaaagcagaccctgctatgagcaagtcataaggcaaacttcaccttgacagaaaattttcagagctgaccacctgctaaacaaaaataaaaaatatgtaccttggatagggacttgttccaagtttttctatatcttgggtaagcaagtgatttggaaatggttatacatgacaggtgctgcatgtttgtcatagcaaactctggttattgttctacttgttttttgtcataatttttgcatcaaaactaaactattaagtggaagtataatttactcatctcgagggggatggagcatgtttggctgattgtcattatagttagcctctctgatagtgttcttagatgtacttctatatatgttgcaggacattgagagtgatgacaaggatcttgattttgaggttgatgatggagctgaggatgaacctaaagcatgatccgaaagatgccccagccgaacctgctatcaagacagttgtgggccctagctgcgccacccaaagagacagaaagacagttgtctaaaaaggagatgaaaaaaaggaactagcagaacttgatgcagtattggctgagctgggactttctggtattcgagcagcgctgcacaggatggtgagagtcatacatgtttccgttaaaactgcctgatctattttgtatgctccggtttagagagagtctaaataattttgagtattttgaaattctagatgagttgtaaatttccaacaagactattgtagtaatagaggttagatgttcacgtgtaggcatcacattggtgtgcttttgggttacccacttaggtggattgcctgagtcattcatgaaatattattgtgtatcatcgcaacacagtgaattggttgttggcaaaaagaatttgagaca

SEQ ID NO: 38 - DNA, 637 bp, Artificial Sequence
  cDNA
gctacgtgccttccaccagagataagctgcgtcgtccgctctgagggggctgctgtcttggacgagatgtcgatccttgcggggtcgcacgcctccacaaccgccatgcggcaaggttcaaagacaactgcaactaacaattaaagcacaaggaatatacttgcagatgatcattgaggagcaacaaaagcttggtggatcaattaaagcttctgagggacattgagagtgatgacaaggatcttgattttgaggttgatgatggagctgaggatgaacctaaagcatgatccgaaagatgccccagccgaacctgctatcaagacagttgtggccctagctgcgccacccaaagagacagaaagacagttgtctaaaaaggagatgaaaaaaaggaactagcagaacttgatgcagtattggctgagctgggactttctggtattcgagcagcgctgcacaggatggtgagagtcatacatgtttccgttaaaactgcctgatctattttgtatgctccggtttagagagagtctaaatagttttgagtattttgaaattctagatgagttgtaaatttccaacaagactattgtagtaatagaggttagatgttcacgtgtaggcatcacattgg

SEQ ID NO: 39 - protein, 55 aa, Zea mays
MARVFQQDATCLPPEISCVVRSEGAAVLDEMSILAGSHASTTAMRQGSKTTATNN

SEQ ID NO: 40 - protein, 56 aa, Zea mays
MTRILILRLMMELRMNLKHDPKDAPAEPAIKTVVALAAPPKETERQLSKKEMKKRN

SEQ ID NO: 41 - DNA, 1327 bp, Zea mays
tattgttgcctcctcctcatctcatcactagtcactcaaccgcaattgattgaaaattgtgttcatcatctcgttggatcgatcataattctttcatttctggcctcgacaagtatcgagctcattaatccatcaatccaatgtgtgttctgtcgaaggcgacaatggtgagctacttatcgcggcgtccatttaatggctgcagcacaaaggcgatggacgtgatcgtggtcgacaagaccatcgtgccggggggggaggggggtagagggtgacggtgctgatgatggatggcgatggtatccggggtctcatcccggaaaccattcttgccttcctcgaggcgagggtgcaggatctggacaggctggaggcgaggctcgcagactacttcgactacatcgccaggaccggtgggctcgtcatcacgctgctcacttcgcccggcaaggacaagcggcctctctacgttgccaagaacatcaaccacttgttcttgcatccattcacatcgccctaatcacatcaatgtatagaggactatgatggatggatgcaagaacaatgacgccagatggaattcacttttgagggaagacatgtgggctgttctccatgtagaagtggttgatgtccttggcaacgtagagagaccgcttgtttttgccggtcccgatgaacatggcggtgatgatctcatcggtgctattcctagtgatgtagtcgaagtagtccgcgagccttgccttcgtcccgtccaactcctacggcatggcctcgaggaaggtgaggatggttcccgagatgagaccccagatggcgcctctgtccaccgttatcactgtcaccctcggttcaacacgacgggctcatcgaccatgctcccggccatcgccttcgtgctgcatgtgttgcatggacgccttgatgagtagctcaccgttgccgcctttgaccaagcacacacccaattgatcgattaatgaactagatactcattgaggccacgaatgaaagaattatcatcaaaccaacaaatgacggacacaattttcaatcgattatggatgagtgtgagtagtgatgagctgaggaagatgcaatgatagatcgattgtgtacatatataggcactgcgtacgtgctgcccctttttggagtgacaaataggaactagcgcgcgtatttttgcatacaaccactactaaataagagatatatgtaaaatttaacgcaagggatatagggaagagatatttgtccattgcaatgtattttgaagctgtccacatatactatttatgaagaaacggattatgccaagtat

SEQ ID NO: 42 - DNA, 714 bp, Zea mays
atcattacataacttatgctatattttcccgagtatgtcctaacatcttccacagtgtttttatgggctccttagaagttccagcccaggggcctgaaactattaaagttccaactgctcattatgaatttggtgccaattttttagatccaaagttaatgctcattggaagggtgataacagatggaaggcttaatgctcgcgtgaaatgtgatttgacagacaatctcacgctgaaagtaaatgcacagcttacccaagaggcacattactcacaaggaatgtttaactttgactacaaggttgacgtttctgacaagtcagacgtaacgagggcgtccacaccgcggctccgccggacatcgcaacaatctccccgccccagctctcctctccctgcgccgaggccacaatccctgccgccccggctctcctcgtccccaaatcttgcacgcggtcgtaatccccgccgcctcgctctcctcgcccctagatcgccgcctccactatcgctgatataccagaccaagcaggtagagcagaccaagatgtcgctcgaggaggccaagctggagatggccacgctgctgcagcagcaggcgagcaagtcatgcatggtactaagtcctgcatggtactaatggttgtaatgtagtgatgaaatagctagattaaaataacaaaatttatgtatggctaggatcacaaatagat

SEQ ID NO: 43 - DNA, 460 bp, Zea mays
ccagcccaggggcctgaaactattaaagttccaactgctcattatgaatttggtgccaattttttagatccaaagttaatgctcattggaagggtgataacagatggaaggcttaatgctcgcgtgaaatgtgatttgacagacaatctcacgctgaaagtaaatgcacagcttacccaagaggcacattactcacaaggaatgtttaactttgactacaaggacgtaacgagggcgtccacaccgcggctccgccggacatcgcaacaatctccccgccccagctctcctctccctgcgccgaggccacaatccctgccgccccggctctcctcgtccccaaatcttgcacgcggtcgtaatccccgccgcctcgctctcctcgcccctagatcgccgcctccactatcgctgatataccagaccaagcaggtagagcagaccaagatgtcgctcgagg

SEQ ID NO: 44 - protein, 192 aa, Zea mays
MGSLEVPAQGPETIKVPTAHYEFGANFLDPKLMLIGRVITDGRLNARVKCDLTDNLTLKVNAQLTQEAHYSQGMFNFDYKVDVSDKSDVTRASTPRLRRTSQQSPRPSSPLPAPRPQSLPPRLSSSPNLARGRNPRRLALLAPRSPPPLSLIYQTKQVEQTKMSLEEAKLEMATLLQQQASKSCMVLSPAWY

SEQ ID NO: 45 - protein, 127 aa, Zea mays
MLIGRVITDGRLNARVKCDLTDNLTLKVNAQLTQEAHYSQGMFNFDYKDVTRASTPRLRRTSQQSPRPSSPLPAPRPQSLPPRLSSSPNLARGRNPRRLALLAPRSPPPLSLIYQTKQVEQTKMSLE

SEQ ID NO: 46 - DNA, 2979 bp, Helianthus annuus
atgaataacatcaatcttgtaatagtttcgcttgtaatcgcgattgtagccatccaaccccttgcgcaagagcaaaccgatgtaggtgaggcaaatttcgtcactgttcttagcatcgatggtgggggtgttcgtggcattgttcccgccaccttgcttgcttttcttgaatccaaaattcaggtactcgaacttaaaatgcacatgtgcatcatattacaagctgtaacttattattgaaatgtgccgtctcttcggataggaaatagatgggccagatgcacgaattgcggattattttgatgtaatagccggaacaagcacaggagggctgatgacaactatgcttgcagctcctaatgagaaaaatcgtcccatgttcgccgcaaaagacattaccaacttctactttcaacattcgcctaggatcttccctaaaatagggtaaactctaactagtttccggatctataagatcatcattaaatacaagtttcattttctttttcgaatcaaatacagacacacatttgatgaggcgcaaccttatccttctcaaaacgaagcctgcgaaatggggtattctcctacaaagacttttgtaattcatgttctagtgggtgtttggatgtgcgttttaaaactgattattatttacatgtagtttctgaagaaaataaaacagttattcaaacactttttgttaataattctactagaaaaaaaaaatccttgtcaggaaattaattaaaaaaaagttaccatctattaaagttctttcttactaatcaaaagtttttaaattttattatcatgttattataactaaacatacacatccaaacactatctcataccacatgattacacaagtctattatttgaatatgctaacttagtattttcatataataagtttttaaaacgccacatccaaaacccttgattcttattttacattgtgtagctaaaacagtgtttatacataaaaacaatcagttatataaatcaaagcattatttaactaaagtaagctcggttcaaactcgataagagaattaatatatacgagtcgagttcctgttgaccagatttcgctagtgttaagtttcgagttcaaaattgtatatgaacttgaacctgtgtatcatcatacttgacatttaaaccataatgttgttgaataaataaagtgattttattttgtagtcggaccaaattcatgaattcggtagtaaccgtacttggtgaggccaccggaccaaagtatgatggtaaatatcttcgagccatggcaaagatgatgttaaaaaacctcactattaaagatacgttgacgaatgttgtcatacctgctttcgacattaggcggcttcaacctgttatcttctcctctgctcaagtaattaaactcgttttttatatttatagcagttctctatttaaaattgattgtgtatcataaaatggtttctgtttgatacgtttagggaaaagaggtcgcgtggaaaaatgctttgctagcagacgtatgcattagtaccgcggcggcaccaacatttttcccgccatactattttgagactagagacgtcgatggaaccaagcacacttttgatctaatcgatggcggggtagctgcaaacaatccggtagttacatttcaacaatattgagtttgcattttatttttaggacaagtagtcacattagggtgaagggtgtgttcaagctcatcccgaaggtgggagcggtgttcccactcgtacctcatggcgcattttcttctttgttgcagctccaattttaaaaagccaccccgccttttccattccatagcgccacgtcaactgggaaatggtgttcccactggtattggagatttggaggcgctacgccacctctgtcatcccgaagccacaccctccacccttaggagtgttatcggttcagttttcggtttatacagtttaaaggtttttttttggttgaaaccaaaaaccgaactgaactgaacggaattcgggtagttcacaactgaaccaaaaactgaatccatattcggttttctgtttgaccgaataatcattatttgttatttgattgtgcgaggttaaataagattgagcaaaaattgtaattaattggatttggctaaatgacaatttaaataaccgttatttgttatccgattcaaaccgaacacccaactcgatttggtttaataccgaaccgacaaccggatacgtaattcagttcgctattaaaaggttcgggtttggtagggtttaacccatttgaaatcgaatcttcagagaaagggttcgctaatgtcacccacataaccaaagaaatcttgtttaaatgttaatggcagacacatttggctatcacacatataaccaaagaagcggtgatggggaaatacaggttctctggcccggaggttttcgacggaagacggatgcttgtgctttcactcggcactggtacgcagacgtacaatgacttatatactgcacaaaaggctgcaaaatgggggttgcttagttggatctttaccaatggtactgcgccaatcctccgcatttttggtgatgccatgtcagatatggtcgacatccatgtgtcaactatattccaatcgttgcaagtcgaaaaaaactatctgcgtattcaggtataactaagaacatataaatataatgttgtataggttacatgtttagtaacaaggagtttttttatgggcaggaagataacttgaaaggggaagcaactgcaatggatatttcatcacctgagaacatgagggcgctagaggacattggcaagaaattgttgaagaaaccgttgtcgagattggatgtggagacaggcaagcttgaaccagttaaaggagaaggtacgaatgctgatgcattagcacgtttcgccactttgctttgtgccgaacgaaagcgccgcaatccagcttaa

SEQ ID NO: 47 - DNA, 1302 bp, Artificial Sequence
  cDNA
atgaataacatcaatcttgtaatagtttcgcttgtaatcgcgattgtagccatccaaccccttgcgcaagagcaaaccgatgtaggtgaggcaaatttcgtcactgttcttagcatcgatggtgggggtgttcgtggcattgttcccgccaccttgcttgcttttcttgaatccaaaattcaggaaatagatgggccagatgcacgaattgcggattattttgatgtaatagccggaacaagcacaggagggctgatgacaactatgcttgcagctcctaatgagaaaaatcgtcccatgttcgccgcaaaagacattaccaacttctactttcaacattcgcctaggatcttccctaaaataggacacacatttgatgaggcgcaaccttatccttctcaaaacgaagcctgcgaaatgggtcggaccaaattcatgaattcggtagtaaccgtacttggtgaggccaccggaccaaagtatgatggtaaatatcttcgagccatggcaaagatgatgttaaaaaacctcactattaaagatacgttgacgaatattgtcatacctgctttcgacatcaggcggcttcaacctgttatcttctcctctgctcaaggaaaagaggtcgcgtggaaaaatgctttgctagcagacgtatgcattagtaccgcggcggcaccaacgtttttcccgccatactattttgagactagagatgtcgatggaaccaagcacacttttgatctaatcgatggcggggtagctgcaaacaatccgacacatttggctatcacacatataaccaaagaagcggtgatggggaaatacaggttctctggcccggaggttttcgacggcagacggatgcttgtgctttcactcggcactggtacgcagacgtacaatgacttatacactgcacaaaaggctgcaaaatgggggttgcttagttggatctttaccaatggtactgcgccaatcctccgcatttttggtgatgccatgtcagatatggtcgacatccatgtgtcaactatattccaatcgttgcaagtcgaaaaaaactatctgcgtattcaggaagataacttgaaaggggaagcaactgcaatggatatttcatcacccgagaacatgagggcgctagaggacattggcaagaaattgttgaagaaaccgttgtcgagattggatgtggagacaggcaagcttgaaccagttaaaggagaaggtacgaatgctgatgcattagcacgtttcgccactttgctttgtgccgaacgaaagcgccgcaatccagct

SEQ ID NO: 48 - protein, 433 aa, Helianthus annuus
MNNINLVIVSLVIAIVAIQPLAQEQTDVGEANFVTVLSIDGGGVRGIVPATLLAFLESKIQEIDGPDARIADYFDVIAGTSTGGLMTTMLAAPNEKNRPMFAAKDITNFYFQHSPRIFPKIGHTFDEAQPYPSQNEACEMGRTKFMNSVVTVLGEATGPKYDGKYLRAMAKMMLKNLTIKDTLTNIVIPAFDIRRLQPVIFSSAQGKEVAWKNALLADVCISTAAAPTFFPPYYFETRDVDGTKHTFDLIDGGVAANNPTHLAITHITKEAVMGKYRFSGPEVFDGRRMLVLSLGTGTQTYNDLYTAQKAAKWGLLSWIFTNGTAPILRIFGDAMSDMVDIHVSTIFQSLQVEKNYLRIQEDNLKGEATAMDISSPENMRALEDIGKKLLKKPLSRLDVETGKLEPVKGEGTNADALARFATLLCAERKRRNP

SEQ ID NO: 49 - DNA, 1795 bp, Artificial Sequence
  TILLING mutant D74N
agttcatcactaatcacacttattgtgccctcgacgagtatctatagctagctcattaatcgattcgggggtgtgttgtcgaaggcggcaatggcgagctactcgtcgcggcgtccatgcaatacctgtagcacgaaggcgatggccgggagcgtggtcggcgagcccgtcgtgctggggcagagggtgacggtgctgacggtggacggcggcggcgtccggggtctcatcccgggaaccatcctcgccttcctggaggccaggctgcaggagctggacggaccggaggcgaggctggcggactacttcaactacatcgccggaaccagcaccggcggtctcatcaccgccatgctcaccgcgcccggcaaggacaagcggcctctctacgctgccaaggacatcaaccacttttacatgcagaactgcccgcgcatctttcctcagaagtgagtccgatgctgccgccattgttcttgcatccatccagcatcgtacgtacgtcctctatacatctgcggatcatcatgtgcgcatgtttgtggcatgcatgcatgcatgtgagcaggagcaggcttgcggccgccatgtccgcgctgaggaagccaaagtacaacggcaagtgcatgcgcagcctgattaggagcatcctcggcgagacgagggtaagcgagacgctgaccaacgtcatcatccctgccttcgacatcaggctgctgcagcctatcatcttctctacctacgacgtacgtacgtcgtcacgaatgattcatctgtacgtcgtcgcatgcgaatggctgcctacgtacgccgtgcgctaacatactcagctctttcctatctgctgcgccaatttgcaggccaagagcacgcctctgaagaacgctctgctctcggacgtgtgcattggcacgtccgccgcgccgacctacctcccggcgcactacttccagactgaagacgccaacggcaaggagcgcgaatacaacctcatcgacggcggtgtggcggccaacaacccggtaactgactagctaactggaaaacggacgcacagactccatgtccatggcggcccacaaggtcgatgctaattgttgcttatgtatgtcgcccgattgcacatgcgtagacgatggttgcgatgacgcagatcaccaaaaagatgcttgccagcaaggacaaggccgaggagctgtacccagtgaagccgtcgaactgccgcaggttcctggtgctgtccatcgggacggggtcgacgtccgagcagggcctctacacggcgcggcagtgctcccggtggggtatctgccggtggctccgcaacaacggcatggcccccatcatcgacatcttcatggcggccagctcggacctggtggacatccacgtcgccgcgatgttccagtcgctccacagcgacggcgactacctgcgcatccaggacaactcgctccgtggcgccgcggccaccgtggacgcggcgacgccggagaacatgcggacgctcgtcgggatcggggagcggatgctggcacagagggtgtccagggtcaacgtggagacagggaggtacgaaccggtgactggcgaaggaagcaatgccgatgccctcggtgggctcgctaggcagctctccgaggagaggagaacaaggctcgcgcgccgcgtctctgccatcaacccaagaggctctagatgtgcgtcgtacgatatctaagacaagtggctttactgtcagtcacatgcttgtaaataagtagactttattttaataaaacataaaaatatatat

SEQ ID NO: 50 - DNA, 1284 bp, Artificial Sequence
  TILLING mutant D74N
atggcgagctactcgtcgcggcgtccatgcaatacctgtagcacgaaggcgatggccgggagcgtggtcggcgagcccgtcgtgctggggcagagggtgacggtgctgacggtggacggcggcggcgtccggggtctcatcccgggaaccatcctcgccttcctggaggccaggctgcaggagctggacggaccggaggcgaggctggcggactacttcaactacatcgccggaaccagcaccggcggtctcatcaccgccatgctcaccgcgcccggcaaggacaagcggcctctctacgctgccaaggacatcaaccacttttacatgcagaactgcccgcgcatctttcctcagaagagcaggcttgcggccgccatgtccgcgctgaggaagccaaagtacaacggcaagtgcatgcgcagcctgattaggagcatcctcggcgagacgagggtaagcgagacgctgaccaacgtcatcatccctgccttcgacatcaggctgctgcagcctatcatcttctctacctacgacgccaagagcacgcctctgaagaacgctctgctctcggacgtgtgcattggcacgtccgccgcgccgacctacctcccggcgcactacttccagactgaagacgccaacggcaaggagcgcgaatacaacctcatcgacggcggtgtggcggccaacaacccgacgatggttgcgatgacgcagatcaccaaaaagatgcttgccagcaaggacaaggccgaggagctgtacccagtgaagccgtcgaactgccgcaggttcctggtgctgtccatcgggacggggtcgacgtccgagcagggcctctacacggcgcggcagtgctcccggtggggtatctgccggtggctccgcaacaacggcatggcccccatcatcgacatcttcatggcggccagctcggacctggtggacatccacgtcgccgcgatgttccagtcgctccacagcgacggcgactacctgcgcatccaggacaactcgctccgtggcgccgcggccaccgtggacgcggcgacgccggagaacatgcggacgctcgtcgggatcggggagcggatgctggcacagagggtgtccagggtcaacgtggagacagggaggtacgaaccggtgactggcgaaggaagcaatgccgatgccctcggtgggctcgctaggcagctctccgaggagaggagaacaaggctcgcgcgccgcgtctctgccatcaacccaagaggctctagatgtgcgtcgtacgatatc

SEQ ID NO: 51 - protein, 428 aa, Artificial Sequence
  TILLING mutant D74N
MASYSSRRPCNTCSTKAMAGSVVGEPVVLGQRVTVLTVDGGGVRGLIPGTILAFLEARLQELDGPEARLADYFNYIAGTSTGGLITAMLTAPGKDKRPLYAAKDINHFYMQNCPRIFPQKSRLAAAMSALRKPKYNGKCMRSLIRSILGETRVSETLTNVIIPAFDIRLLQPIIFSTYDAKSTPLKNALLSDVCIGTSAAPTYLPAHYFQTEDANGKEREYNLIDGGVAANNPTMVAMTQITKKMLASKDKAEELYPVKPSNCRRFLVLSIGTGSTSEQGLYTARQCSRWGICRWLRNNGMAPIIDIFMAASSDLVDIHVAAMFQSLHSDGDYLRIQDNSLRGAAATVDAATPENMRTLVGIGERMLAQRVSRVNVETGRYEPVTGEGSNADALGGLARQLSEERRTRLARRVSAINPRGSRCASYDI

SEQ ID NO: 52 - DNA, 1795 bp, Artificial Sequence
  TILLING mutant G78R
agttcatcactaatcacacttattgtgccctcgacgagtatctatagctagctcattaatcgattcgggggtgtgttgtcgaaggcggcaatggcgagctactcgtcgcggcgtccatgcaatacctgtagcacgaaggcgatggccgggagcgtggtcggcgagcccgtcgtgctggggcagagggtgacggtgctgacggtggacggcggcggcgtccggggtctcatcccgggaaccatcctcgccttcctggaggccaggctgcaggagctggacggaccggaggcgaggctggcggactacttcgactacatcgccagaaccagcaccggcggtctcatcaccgccatgctcaccgcgcccggcaaggacaagcggcctctctacgctgccaaggacatcaaccacttttacatgcagaactgcccgcgcatctttcctcagaagtgagtccgatgctgccgccattgttcttgcatccatccagcatcgtacgtacgtcctctatacatctgcggatcatcatgtgcgcatgtttgtggcatgcatgcatgcatgtgagcaggagcaggcttgcggccgccatgtccgcgctgaggaagccaaagtacaacggcaagtgcatgcgcagcctgattaggagcatcctcggcgagacgagggtaagcgagacgctgaccaacgtcatcatccctgccttcgacatcaggctgctgcagcctatcatcttctctacctacgacgtacgtacgtcgtcacgaatgattcatctgtacgtcgtcgcatgcgaatggctgcctacgtacgccgtgcgctaacatactcagctctttcctatctgctgcgccaatttgcaggccaagagcacgcctctgaagaacgctctgctctcggacgtgtgcattggcacgtccgccgcgccgacctacctcccggcgcactacttccagactgaagacgccaacggcaaggagcgcgaatacaacctcatcgacggcggtgtggcggccaacaacccggtaactgactagctaactggaaaacggacgcacagactccatgtccatggcggcccacaaggtcgatgctaattgttgcttatgtatgtcgcccgattgcacatgcgtagacgatggttgcgatgacgcagatcaccaaaaagatgcttgccagcaaggacaaggccgaggagctgtacccagtgaagccgtcgaactgccgcaggttcctggtgctgtccatcgggacggggtcgacgtccgagcagggcctctacacggcgcggcagtgctcccggtggggtatctgccggtggctccgcaacaacggcatggcccccatcatcgacatcttcatggcggccagctcggacctggtggacatccacgtcgccgcgatgttccagtcgctccacagcgacggcgactacctgcgcatccaggacaactcgctccgtggcgccgcggccaccgtggacgcggcgacgccggagaacatgcggacgctcgtcgggatcggggagcggatgctggcacagagggtgtccagggtcaacgtggagacagggaggtacgaaccggtgactggcgaaggaagcaatgccgatgccctcggtgggctcgctaggcagctctccgaggagaggagaacaaggctcgcgcgccgcgtctctgccatcaacccaagaggctctagatgtgcgtcgtacgatatctaagacaagtggctttactgtcagtcacatgcttgtaaataagtagactttattttaataaaacataaaaatatatat

SEQ ID NO: 53 - DNA, 1284 bp, Artificial Sequence
  TILLING mutant G78R
atggcgagctactcgtcgcggcgtccatgcaatacctgtagcacgaaggcgatggccgggagcgtggtcggcgagcccgtcgtgctggggcagagggtgacggtgctgacggtggacggcggcggcgtccggggtctcatcccgggaaccatcctcgccttcctggaggccaggctgcaggagctggacggaccggaggcgaggctggcggactacttcgactacatcgccagaaccagcaccggcggtctcatcaccgccatgctcaccgcgcccggcaaggacaagcggcctctctacgctgccaaggacatcaaccacttttacatgcagaactgcccgcgcatctttcctcagaagagcaggcttgcggccgccatgtccgcgctgaggaagccaaagtacaacggcaagtgcatgcgcagcctgattaggagcatcctcggcgagacgagggtaagcgagacgctgaccaacgtcatcatccctgccttcgacatcaggctgctgcagcctatcatcttctctacctacgacgccaagagcacgcctctgaagaacgctctgctctcggacgtgtgcattggcacgtccgccgcgccgacctacctcccggcgcactacttccagactgaagacgccaacggcaaggagcgcgaatacaacctcatcgacggcggtgtggcggccaacaacccgacgatggttgcgatgacgcagatcaccaaaaagatgcttgccagcaaggacaaggccgaggagctgtacccagtgaagccgtcgaactgccgcaggttcctggtgctgtccatcgggacggggtcgacgtccgagcagggcctctacacggcgcggcagtgctcccggtggggtatctgccggtggctccgcaacaacggcatggcccccatcatcgacatcttcatggcggccagctcggacctggtggacatccacgtcgccgcgatgttccagtcgctccacagcgacggcgactacctgcgcatccaggacaactcgctccgtggcgccgcggccaccgtggacgcggcgacgccggagaacatgcggacgctcgtcgggatcggggagcggatgctggcacagagggtgtccagggtcaacgtggagacagggaggtacgaaccggtgactggcgaaggaagcaatgccgatgccctcggtgggctcgctaggcagctctccgaggagaggagaacaaggctcgcgcgccgcgtctctgccatcaacccaagaggctctagatgtgcgtcgtacgatatc

SEQ ID NO: 54 - protein, 428 aa, Artificial Sequence
  TILLING mutant G78R
MASYSSRRPCNTCSTKAMAGSVVGEPVVLGQRVTVLTVDGGGVRGLIPGTILAFLEARLQELDGPEARLADYFDYIARTSTGGLITAMLTAPGKDKRPLYAAKDINHFYMQNCPRIFPQKSRLAAAMSALRKPKYNGKCMRSLIRSILGETRVSETLTNVIIPAFDIRLLQPIIFSTYDAKSTPLKNALLSDVCIGTSAAPTYLPAHYFQTEDANGKEREYNLIDGGVAANNPTMVAMTQITKKMLASKDKAEELYPVKPSNCRRFLVLSIGTGSTSEQGLYTARQCSRWGICRWLRNNGMAPIIDIFMAASSDLVDIHVAAMFQSLHSDGDYLRIQDNSLRGAAATVDAATPENMRTLVGIGERMLAQRVSRVNVETGRYEPVTGEGSNADALGGLARQLSEERRTRLARRVSAINPRGSRCASYDI

SEQ ID NO: 55 - DNA, 13516 bp, Zea mays
tcttgctatatatgagatgacaaaattttccaaagaagagagaagccggcagaacccatcctgtttcaaatctcttctactacttaagtttctaacgtaggcgtcgacaaaacggattggtgcacggttctgccgatgtctcccacacacgcgcatggaaggaggcaggcacccttccccgccgccccggatctcgcgccagccccagccctaccccgcctgcccttccattcttccccagccgccccccggtcaacgtcacgaacccgggcctcgtgccgttcgccgtggccacgcggttcgacgagcgggtcacggagctgctgagcgcgctcgctgacgcggcggcggggcgaccaggcaggtgggccatcggcgaagcgccatggtcgtcgtcggggggcaggaaccaggcggtgtacgcgcgccgcgcgcccggctcttcatcgcctccacccgctccagcgtctccaccacctccttcatcgagggccgactgcgaggctcgccggccaggcagccgagcgtcagttgcgccgcttggaacgcctgcttttgttgatcgtttgttttggtctgatttcggtgggtctatccgcagagaggaagaagcagaagctctccgagatccaatccggcgttgaggaagctgaatcgctggtaaatagatgccgcgacacgttctggtttggggatccccttggctaacaggacatacgacatttggggaatgggtagaaaagcagagattagggatttttcgtttccgtcggtgcagttttggtgttccaacggagttgcgagatgtttatgtgccttagtcttcaatttgggggttgggggaaaagtaattttatgtttttgttttgtgtctgcagattcagaaaatggacctggaggcaaggagcctacagcctagcattaaggctagtttgcttgcaaagctgagggagtataaatctgacctcaacaacgtcaagagtgagctcaagaggatatctgcgcccaatgccaggcaggctacccgggaggagctcctggagtctggaatggctgatactctcgcagtgagctaatgataggacttgactgtgtctacgagactgctcctaacaataaactgaagaaagcaaaagaaatcattcaacgtattcgccgaagagaactctacaaggtagtatgatgctttaattgctcatatacaagtgtcattttgtcatgtcattacacatggttaggatacataggagattctgttttttaacacatagttgtcccatgtccatgaattcatttgaattaatttactcttcgcaatcttatacattaaaatcgtgttacctattacatcacaacttcatgagagcatgcttgttctgtgtagatatggtagtcctgggaggaagagccatcgccgctatgtatggcagaaccacccgcgaaagcaacctctctggtctcgcatagccagagcaggagcagctcgcttgcgcggccgcagcgctggcggtcggccccgcgtacgagcgcctgcaggtaggccagcttctgctgcaatgcccgaatctcggcgtccacgcgcagcagcgtcgtcgcctcctcctccgtcagctcacccagcttggccagcacccccgtcacccccgcgtccgccatggctgtcgccgggaccgaaaggctaaaactgtcacaatgacgtaaagtttggttggtgttggcggctcacgcaaaaccagacctttccaagttttactttagcagagtttttttggaacgagagcaaagcagcacagtttcaagaatgtggggcaatttgaatgttcgttcctgctgcactgctactgcttttagaattgtagtatgcttcatcatttatttatttctaaaaaaacttgcatgaattctatcgtgacttttattgagaaaataatgtattcacgtatcttcatgtttctgataaaggtatttgtatatgcatcggtgctacatatgcgaatacaagttttgtttcaactctgaagtctcaagttgaattctaaactccagtttgttttctactgtgctgctgcaggaagccaggaacccatccgaacaaggttgcaatcatgataagcagatagagcaagcatatgatgatattttgaattcgtcgaagcatactttggccagcatgatggagctgcaggaggttcagttatttgcacacattgtttttctttcactcctatgattttcctcaatatgatcaaaatgtttcttttgcaaataatgattgaaatgtttctcattgtactcaacctcttaaactacctataggctttgcttgagagtaatcaggctacaaaggatgccaatggtattgctgctctctatattgttcttgttctaatgtaaaaactacaacacaactctttacttgatcccagaaattccttctgcctcaaatggagacaatgacgagtggtcagaagtacagagattgcagacaaggtaaattttgcaatagaaataactaaccaaccattagtgcttgaaaaaaactggactggtgactggggcacgtggtttcatcaacatttggacctcaacggtctaatcagtataacttagaagttggctagctcttgaaaaacactgcatgacactaagcatttgtttattttcagctgcttgcacccctatgatttcaagtaactacttgtctacttgtgataatcacctgaatatgagtatttgaaatgcttatcacgtctcggcaattgcatttcttttatgcgtaactgaagtctgctctagcttcctaatagagttcattttttaatacagaaaccactttgagatagccacaatatagtaaaagtggcagctaaggtactaaaaacacccatgcaaataagaaaaaaaatgaatcttgtattttaattttgttaaatacctctatagtttggcgatatattatgttaccatcctgcttgtagcctgtaggtcattttatatgagccatcaaattgcgatgacagttgccacaaatccagtttcatatgaaggtattagctgtgtaacaagctaactgctgctctctgcccaataagttattcaattggattagtaggttgcatccaaggttattcaattggatcagtaggttgcatccaaggtatactgctgctctctgcccaataagttattcaattcgatcagtaggttgcctgttcccttcattttattaaaaaatacataataatataataagtacctgtttgttctaaaaataatacttctgtaaatgaggttattaattttccttttggtaataatgcaggttgatgatactgaagtcatcagttttttgttgcaaactgaaataatttctctgtgcttgcgaaccatggagatgggtagtgagctatccaaaactgtatgtagctagccatatattctcattcaaatatcataatttatctcttctgcttaatactggcaaaggtgtaatagtttttttagtattgatttgtcacctgaagtttatcttgtgcactactactttgccatcatcagttatctctagaatactcttatcctgtaccatcttctctctgataagcctaaatttgtacaattcataagcctaaaaggtgacttatataatatatacaaggaccctcaagagttgtttggcaattcagtgactgtcctgggtcctgttttggggagcttctggtagcttttgcttctccaaaagaaaagctagaagctccccccaaacagagcagcttcttcaagccggtaaaagcttcaaaagctataattatactaaaaacagtgaagctccctcagagcagcttcccagctctccaggagatgcttttggagaagctacagtttccccaaacagggccctgctctgttgaaccccccttcctgatacatatttgaatatgagtttatagtgtgtgtgggggggtgtaagtaggggggtaatgggttctaaattttatactataaaaattaaggatcagattagaattgagctctatttctattcatttttgaactaaaattaattaagggctcaaatgaattatgaagaagcattaggatcatgatccattaccacccctacgtgtaagatgttttttggtggttgtggttgattttgaattttaaggccgcatatgtctcatggactacacaagctcatattcatctacatttgtagccgtcactaacttagccaaatatgcatatgtggcggctgagagcacctagagggggggggggtgaataggtgatcctataaaaacttgaaacataatgccacaaaacttgattaggagttagcacaataaagccaagtgactagagaggagttcttgcaagacacgataaccacacgaagatcaacacagatagacacaatggtttatcccgttgttcggccaagtccaacacttgcctactccacgttgtggcgtcccaacggacgagggttgcaatcaacccctctcaagcggtccaaggacccacttgaataccacggtgttttgcttagtttcactatatcccgcttgcgaggaatctacacaacttggagcctctcgcccttacaatttgatgttcacaaagaagcacgaaagtaaggctgggatgagcaacgcacacaagacacaaaatcagagcacaacacgcacacaagtcacaacacgagctcacaacacaacccaaagagttctctactcaaatggagctctagttgctatcacaaagaatcgaatacgcggaattggagtcttggtgcttagaaacgcttagagaatgcttggtgtgttcctccatgcgcctaggggtcccttttatagccccaaggcagctaggagccgttgagagcattccaggaaggcaattcttgccttctgtcgcctggcgcaccggacagtccggtgcaccaccggacactgtccggtgcggatttctttccttctttagcgaagccgaccgttggagattcagagccgttggcgcaccggacagtgtccggtgcacaccggacagtccggtgcccccttctgaccgttggctctgccacgcgtcgcacgcggattacgcggccgaccgttggcccggccgactgttggctcaccggatagtccggtgcaccaccggacagtccggtgatttatagccgtacgccgccgacgaaacccgagagcagccagttcgccagagccagcctggcgcaccagacactgtccggtgcacccagactacgcagtcttggctgcacagccaagtcttttccaaattggtctttttctgtttctagcacttagacacattacattagtatccaaaacaatgtactaagtcttagaaacatacctttactcttgatttgcactttgtccatcatttggcatagattaacacatgaccacttgtgttggcactcaatctccaaaatacttagaaatggcccaatggcacatttccctttcaatctccccctttttggtgatttatgccaacacaacaaaaagcaactaaaagaagtgcaacatcaatgcaaatgagaacaaaaaattgttttgattcaaatttggcatatttggatcattctttgccaccacttggttttgtttttgcaaatcaacctcaatttcctatctctaagtcaaacacacttgttgaaacataaagagagttgttccatgagaaattgatcaaagatttcaaaaactcccccttttttccataatcaaacattctccccacaagagaccaacttttgacagaagagacaataagagaattttgacaaaccaaaaagctctattctactattttcaaaattctcaagtggtagctgatccatttattgctttggccttattttctccccctttggcatcaagcaccagaacgggataaatcttggcccttaaaaccccattgcctcaccaaaatcttcaattaagagtaaaaaggcaataagagcatgaagatgaacttggagttagttactctttcatcggagtgcagtggaagtctttcatggtccaagtccaacatttcctttcaatccacctttgagactaaatcaagcaaactcaagcacacagttagtctcaaggggtcaagttgtagcacaactccccctaaatatgtgcattacttgcaaatggacttgtgaggtccggggagtgtttgtacaacttgagcaccatacataaacaacaaaatgcataaaggaacatgatcaaggcataaaacacatgtatgctataaatcaatccaagttccgcgaatctaagacatttagctcactacgcagcctacaaaaggtcttctcatctagaggcttggtaaagatatcggctagctggttctcggtgctaacatgaaacacttcgatatctcccttttgctggtgatctctcaaaaagtgatgccggatgtctatgtgcttagtgcggctgtgttcaacaggattatccgccatgcggatggcactctcattatcacataggagtgggactttgctcagattgtagccaaagtccttgagggtttgcctcatccaaagtagttgcgcgcaacactgtcctgcggtaacgtactcggcctcagcggtggatagggcaacggaggtttgtttcttagaattccacgacaccagggaccttcctaagaattgacacgtccccgatgtactctttctatcgaccttacatccaacatagtcggagtctgaatatccaatcaagtcaaaggtagacccctttggataccagatcccgaagcaaggcgtagcgactaaatatctaagaattcgcttcacaaccactaagtgacactcctttggatcggattgaaatctagcacacatgcatacacttagcataatatctggtctactagcacataaataaagtaaggaccctatcatagaccggtatgccttttgatcaacggacttacctcctttgttgaggtcggtgtgtccgtcagttcccattgtagtctttgcgggcttggcgttcttcatcccaaactgctttagcagatcttgcgtgtacttcgtttgggagatgaaagtgccgtccttgagttgcttcacttggaacccaaggaagtagttcaactcgcccatcatcgacatctcgaatttctgagtcatcaccctgctaaactcttcacaagacttttggttagtagaaccaaatattatgtcatcgacataaatttggcacacaaaaagatcaccatcacaagtcttagtgaataaagttggatcggctttcccaaccttgaaagcattagcaagtaaaaagtctctaaggcattcataccatgctcttggggcttgcttaagtccatagagggccttagagagcttacacacgtggtcggggtaccgttcatcctcgaagccagggggttgctccacgtgcacctcctccttgattagcccgttgaggaaagcactcttcacatccatttggaacaacctgaaggaatggtgagcggcataggctaacaaaatacgaatagactctagcctagccacaggagcaaaagtctcctcaaagtccaaacctgcgacttgggcatagccttttgccacaagtctcgccttgttccttgtcaccaccctgtgctcgtcctgtttgttgcggaacacccacttggttcccacaacgttttgcttgggacgaggcaccagtgtccaaacttcatttcgcttgaagttgatgagctcttcctgcatggccaacacccagtccggatctagcaaggcctcttctaccctgaaaggctcaatagaagagacaaaagagtaatgctcacaaaatttaactaatctagagcgagtagttactcccttgctaatgtcacccaaaatctggtcgacgggatgattcctttgaatcgtcgctcgaacttgagttgaaggggcttgaggtgcttcttcctccataacatgatcatcttgtgctcccccttgatcacatgcctcctcttgatgaacctgttcatcgtcttgagttgggggatgtaccaatgttgaggaagaaggttgatcttgctccttttgttcctgtggccgcacatctccaatcgtcatggtgcgtattgcggccgttggaatgtcttcttcatctacatcattaagatcaacaacttgctctcttggagagccattagtctcatcaaatacaacgtcgctagagacttcaaccaaactcgatgatttgttgaaaaccctatacgcctttgtatttgagtcataacctaacaaaaacccttctacagctttgggagcaaacttagaatttctacctttcttcactagaatgtagcatttactcccaaatacacgaaagtatgaaacattgggtttgttaccggttaggagctcatacgaagtcttcttgaggaggtgatgaaggtagacccggtttatggcgtggcaagccgtgttcacggcttccgaccaaaatcgctcgggggtcttgaactctccaagcatcgtcctcgccatgtcaatgagcgtcctatttttcctctctaccacaccattttgctgtggtgtgtagggagcggagaactcgtgcttgattccttcctcctcaaggtactcttctacttgaagattcttgaactccgacccgttgtcgctccttatcttcttcaccttgagctcaaactcattttgagctctccttaggaagcgcttgagggtcccttgggtttcagatttatcctgcaaaaagaatacccaagtgaagcgggaaaaatcatcaactataacaagaccatacttacttcctcctaagcttaggtaggcgacgggcctgaagaggtccatatgtagcaactccaaaggtcttgatgtggtcatcacatttttggtatgatgagagcttcccacttgtttacctgcttgacaagctgcataaggtctatctttttcgaaagtaacatttgttagtcctatcacgtgttctccctttagaagcttgtgaaggttcttcatccccacatgtgctaagcggcgatgccacagccagcccatgctagtcttagcaattaagcatgcatctagaccggcctcctcttttgcaaaatcaactaagtagagtttgccgtctaatacacccttaaaagctaatgaaccatcactccttctaaagacggacacatctacatttgtgaataagcaattatatcccatattacaaagctaactcacagacaataagttatatccaagagactcaactaaaaacacattagaaatagagtgctcggatgaaatggcaatcttccctagtcctttgaccttgccttgattcccgtcaccgaatatgattgagtcttgggaatccttgttcttgacgtaggaggtgaacatcttcttctcccccgtcatgtggtttgtgcatccgctgtcgataatccagcttgatcccccggatgcataaacctgcaaggcaaattaggcttgggtcttaggtacccaactcttgttgggtcctacaaggttagtacaaatagccttagggacccaaatgcaagttttatctcccttgcattttgcccctaattttctagcaaccaccttcttatcctttctacaaatatcaaaggaagcatttaaagcatgataaattgtagaaggttcattacttgttttcctaggtacatgagcatttctcctaggcacatgatgaatgatatttttcctagccaaatttctatcatgcataatagaagaacttgaagcaaacattgcatttgaatcataagcatgtgaaatgacatcattgcaacttctatcatgatgaacattcctggaatatctcctatcatggtataagaaagcatggttcttttgaatactatttgccataggggccttccctttctccttgatggagataggagccttatgacttgtcaagttcttggcttccctcttgaagccaagcccatccttaattgaggggtgtctaccaaccgtgtaggcatcccttgcaaattttagtttatcaaaatcatttttgctagtcttaagttgagcattaagactagccacttcatcttttagtttagaaatgcaaactaggtgttcactacaagcatcaacattgaaatctttacacctattgcaaatcgtaacatgttcttcacgagaggttaatttactagctatttctaacttagcactcaaatcatcattaacactttttaggctagagatagattcatggcatgtagacaattcacatgaaagcatttcatttcttttaatttctaaagcaagagaattttgtgcttctacaaacttatcatgttcttcatacaaaagatcctcttgcttttctaataatctattcttatcattcaaggcatcaatcaactcattgatcttatcaatcttagttctatctaagcccttgaacaaactagcatagtctatttcatcatcgctagattcatcatcactagaagcataagtagactttcgagtgtttaccttcttctcctttgccattaagcatgtgtgatgctcgttgggggaagaggaacgacttgttgaaggccgaggcgacgagtccttcgttgtcggagtcggacgacgaacaatccgagtcccactccttgccaaggtgtgcctcacccttagccttcttataagccttcttcttttccctcttcttctcttgttcctggtcactatcattatcgggacaattagcgataaatgaccaatcttaccacatttgaagcatgagcgcttccccttcgtcttgttgggatgctccttgcgaccctttagtgctgtcttgaatcgcttgatgatgagggccatttcttcttcattaagcccgaccgcctcaacttgcgccaccttgctaggtagcgcctccttgctcctcgttgctttgagagccacagtttgaggctcgtggattgggccattcaacgcatcatcgacgtatcttgcctccttgatcatcatccgcccgcttacgaactttccaagtatttcttcgggcgacatcttggtgtacctaggattttcacgaatattgtttacaagatgtggatcaaggatagtgaaggaccttagcattaggcggacgacgtcgtgatccgtccatcgcgtgcttccatagcttcttattttgttgacgagggtcttgagccggttgtacgtttgggttggctcttctcccctgatcattgcgaatctcccaagttcgccctccaccaactccatcttggtgagcatggtgacatcgttcccctcatgtgagatcttgagggtgtcccagatctgcttggcgttatccaagccgctcaccttatggtattcatccctgcacaatgatgctagaagaacagtagtagcttgtgcatttttgtgaatttgctcattgataaatatgggactatcagtactatcaaattgcattccactctctactatctcccatatgcttggatggagagagaacaagtgactacgcattttgtgactccaaaatccgtagtcctctccatcaaagtgaggaggtttaccaagtggaatggagagtaaatgagcatttgtactttgcggaatacgagaataatcaaaagaaaagtttgaattgactgttttctttttctcgtagttgtcgtcgtccttttgggaagaagaggactcgtcgctgtcgtcgtagtagacgatctccttgatgcaccttgttttcttcttcttcctgtcttttcttttgtggctcgagcccgagtcagtaggcttgtcatcttttggatcattgacgaaggactccttctccttatcattgaccaccatccccttgcccttaggatccatctcttcgggcgattagtcccttacgtgaagagaacgactcagataccaattgagagcacctagaggggggtgaataggtgatcctataaaaacttgaaacttaatgccacaaaacttgattaggagttagcacaataaagccaagtgactagagagttcttgcaagacacgataaccacacaaagatcaacacagatagacacagtggtttatctcgtggttcggccaagtccaacacttgcctactccacgttgtggcgtcccaacggacgagggttgcaatcaacccctctcaagcggtccaaggacccacttgaataccacagtgttttgcttagtttcactatatcccgcttgcgaggaatctccacaacttgtagcctctcgcccttacaatttgatgttcacaaagaagcacgaaagtaaggctgggatgagcaacgcacacaagacacaaaatcagagcacaacacgcacacaagtcacaactcgagctcacaacacaacccaaagagttctctactcaaatggagctctagttgctatcacaaagaatcgaatgcgcggaattggagtcttggtgcttaggaacgcttagagaatgctttgtgtgttcctccatacgcctaggggtcccttttatagccccaaggcagctaggagccgttgagagcattccaggaaggcaattcttgccttctgtcgcctggcgcaccggacagtccggtgcaccatcggacactgtccggtgcagatttctttccttttttagcgaagccgaccgtcggagattcagagccgttggcgcactggacactgtccgatggacaccggacagtccggtgcccccttctgaccgttggctctgccacgcgtcgcgcgcggattacgcggccgaccgttggctcgaccgactgttggctcactgaacagtccggtgcaccaccggacagtccggtgatttatagccgtacgccgccgacgaaacccgagagcagctagttcgctagagccagtctggcgcaccagacattgtccggtgcaccaccggacagttcggtgcacccagactgcgcagagtcttggctgcacagccaagtcttttccaaattggtcttttcctgtttctagcacttagacacattacattagtctccaaaacaatgtactaagtattagaaacatacctttactcttgatttgcactttgtccatcatttggcatagattaacacatgaccacttgtgttggcactcaatctccaaaatacttagaaatggcccaagggcacatttccctttcagcggctagcaacaggtccttggtttcttgggttatttattctctttttatcgtgtttgaatgttttcgtgttcatttgcataacatcttaggtctacatcagtatatgaattgagatcaaatgtgaattggaccacacaagctcatattcatctacatttgtagtcgtcactaacttagccaaatatgcatatgtccgcttctgatttcattgtgtcttttcttcaggagtttggggatcaaggagaggactccattatcttgtcaccgcgactgaaggagattagtactcctgaccgccccgctgccctccgtttcctaggtac

SEQ ID NO: 56 - DNA, 1026 bp, Artificial Sequence
  cDNA Snare T1
gcgcccggctcttcatcgcctccacccgctccagcgtctccaccacctccttcatcgagggccgactgcgaggctcgccggccaggcagccgagcgtcagttgcgccgcttggaacgcctgcttttgttgatcgtttgttttggtctgatttcggtgggtctatccgcagagaggaagaagcagaagctctccgagatccaatccggcgttgaggaagctgaatcgctgattcagaaaatggacctggaggcaaggagcctacagcctagcattaaggctagtttgcttgcaaagctgagggagtataaatctgacctcaacaacgtcaagagtgagctcaagaggatatctgcgcccaatgccaggcaggctacccgggaggagctcctggagtctggaatggctgatactctcgcagtgagctaatgataggacttgactgtgtctacgagactgctcctaacaataaactgaagaaagcaaaagaaatcattcaacgtattcgccgaagagaactctacaagatatggtagtcctgggaggaagagccatcgccgctatgtatggcagaaccacccgcgaaagcaacctctctggtctcgcatagccagagcaggagcagctcgcttgcgcggccgcagcgctggcggtcggccccgcgtacgagcgcctgcaggaagccaggaacccatccgaacaaggttgcaatcatgataagcagatagagcaagcatatgatgatattttgaattcgtcgaagcatactttggccagcatgatggagctgcaggaggctttgcttgagagtaatcaggctacaaaggatgccaatgaaattccttctgcctcaaatggagacaatgacgagtggtcagaagtacagagattgcagacaaggtaaattttgcaatagaaataactaaccaaccattagtgcttgaaaaaaactggactggtgactggggcacgtggtttcatcaacatttggacctcaacggtctaatcagtataacttagaagttggc

SEQ ID NO: 57 - DNA, 874 bp, Artificial Sequence
  cDNA Snare T1
gcgcccggctcttcatcgcctccacccgctccagcgtctccaccacctccttcatcgagggccgactgcgaggctcgccggccaggcagccgagcgtcagttgcgccgcttggaacgcctgcttttgttgatcgtttgttttggtctgatttcggtgggtctatccgcagagaggaagaagcagaagctctccgagatccaatccggcgttgaggaagctgaatcgctgattcagaaaatggacctggaggcaaggagcctacagcctagcattaaggctagtttgcttgcaaagctgagggagtataaatctgacctcaacaacgtcaagagtgagctcaagaggatatctgcgcccaatgccaggcaggctacccgggaggagctcctggagtctggaatggctgatactctcgcagtgagctaatgataggacttgactgtgtctacgagactgctcctaacaataaactgaagaaagcaaaagaaatcattcaacgtattcgccgaagagaactctacaaggaagccaggaacccatccgaacaaggttgcaatcatgataagcagatagagcaagcatatgatgatattttgaattcgtcgaagcatactttggccagcatgatggagctgcaggaggctttgcttgagagtaatcaggctacaaaggatgccaatgaaattccttctgcctcaaatggagacaatgacgagtggtcagaagtacagagattgcagacaaggtaaattttgcaatagaaataactaaccaaccattagtgcttgaaaaaaactggactggtgactggggcacgtggtttcatcaacatttggacctcaacggtctaatcagtataacttagaagttggc

SEQ ID NO: 58 - DNA, 553 bp, Zea mays
cgatgtgcagtggcctgattagctacaagaagctcttgttccatggactcgatctctggaccgcactatcgttgcctcagcccctaggtcatgctgccctctggcctcctcatcgtacaattcaccaacatctccaatgtaagtgcagctggttcagtaatgaactcagaagtggcatcagaatactccaagagttttttgttctttttgcctggatatataccaagggaaatgcattcaaaactcctatagatgacgaatcccatctctccctcttttctcggacacggatccccaggtccgtctccgtgctttactcatttgttttttacaagttcagatccacttgcgtactcacacagtggacatctgttatgcacatgtgtaaaccagcataagaattaggaattatgctcattttatctaagaagtccttacactcgaaaatgcatgtgttatttagcttgagaataaataaaattattagcaaggagaaaaaaaataggactaaagaatagagtcacattggtttaaattagtacctagaagcaaa

SEQ ID NO: 59 - DNA, 527 bp, Artificial Sequence
  cDNA Snare T2
gcttctcgatgtgcagtggcctgattagctacaagaagctcttgttccatggactcgatctctggaccgcactatcgttgcctcagcccctaggtcatgctgccctctggcctcctcatcgtacaattcaccaacatctccaatgtaagtgcagctggttcagtaatgaactcagaagtggcatcagaatactccaagagttttttgttctttttgcctggatatataccaagggaaatgcattcaaaactcctatagatgacgaatcccatctctccctcttttctcggacacggatccccaggtccgtctccgtgctttactcatttgttttttacaagttcagatccacttgcgtactcacacagtggacatctgttatgcacatgtgtaaaccagcataagaattaggaattatgctcattttatctaagaagtccttacactcgaaaatgcatgtgttatttagcttgagaataaataaaattattagcaaggagaaaaaaaataggactaaagaatagagt

SEQ ID NO: 60 - DNA, 9062 bp, Zea mays
gttgcgagatgtttatgtgccttagtcttcaatttgggggttgggggaaaagtaattttatgtttttgttttgtgtctgcagattcggaagatggacttggaggcaaggagcctacagcctagcattaaggctggtttgcttgcaaagctgagggagtataaatctgacctcaacaacgtcaagagtgagctcaagaggatatttgcgcccaatgccaggcaggctacccgggaggagctcctagagtttggaatggctgatactctcgctgtgagctaatgctaggacttgactgtgtctacgagactgctcctaacaataaactgaagaaagcaaaagaaatcattcaacgtattcgccgaagagaactctacaaggtagtatgatgctttaattgctcatatacaagtgtcattttgtcatgtcattacacatggttaggatacatacttaagtttctaacgtaggcgtccacacaacggattggtgcacggttctgccgatgtatcccacgcacgtgcatggaaggaggcaggcacccttccccgccgccccggatctcgcgccagcccccgccctaccccgcctgcccttccactcttcccccgctgcccccggtcaacgtcacgaacccgggcctcgtgccgctcgtcgtggccacactgttcgacgagcgagtcacagagctgctgagcgtgctcgctgatgcggcggtggggcgaccaggcaggtggtccatcggcgaagcgccatggtcgtcgtcggggggcacgaaccaggcggtgtacgcgcgccgcgcgcccggctcttcatcgcctccacccgctccagcgtctccaccacttccttcatcgagggccgactgcttggctcgctggccaggcagccgagcattagttgcgccgcttggaacgcctgcttttgttgatcgtttgttttggtctgatttcagtgggtctatccgcagagaggaagaagcagaagctctccgagatccaatccggcgttgaggaagctgaatcgctggtaaatagatgtcgcgacgcgttctgttttggggatccccttggctaacgggacatacgacatttggggaatgggtagaaaagcagagattagggatttttcgtttccgtcggtgcagttttggtgttccaacagagttgcgagatgtttatgtgccttagtcttcaatttgggggttgggggaaaagtaattttatgtttttgttttgtgtctgcagattcagaaaatggacctggaggcaaggagcctacagcctagcattaaggctggtttgcttgcaaagccgagggattataaatctgacctcaacaacgtcaagagtgagctcaagaggatatctgcgcccaatgccaggtaggctacccgggaggagctcgtggagtctagaatggctgatactctcgcagtgagctaatgctaggacttgactgtgtctacgagactgctcctaataataaactgaagaaagcaaaagaaatcattcaacgtattcgccgaagagaactctacaaggtagtatgatgctttaattgctcatatacaagtgtcattttgtcatgtcattacacatggttaggatacatacttaagtttctaacgtaggcatccacacaatggattggtgcacggttctgccgatgtatcccacgcacgcgcatggaaggaggcaggcacccttccctgccgccccggatctcgcgccagccatcgccctaccccgcctgcccttccactcttccccctgaaagtcgcctagagggggggtgaatagggcgaatctgaaatttacaaacttaagcacaactacaagccgggttaacgttagaaatataaacgagtccgagagagagggcgcaaaacaaatcatgagcaaataaagagtgagacacgatgatttgttttaccgaggttcggttcttgcaaacctactccccgttgaggtggtcacaaagaccgggtctctttcaaccctttccctctctcaaacggtcacttagaccgagtgagcttctcttctcaatcaaacgaaacacaaagttcccgcaaggaccaccacacaattggtgtctcttgccttggttacaattgagtttgatcacaagaagaatgagaaagaaaagaagcgatccaagcgcaagagctcaaatgaacacaaatgtcgctctctctagtcactatttgatttggagtgattccggacttgggagaggatttgatcttttggagtgtctagaattgaatgctatagctcttgtaatatgttgaaggtgggaaacttggatgccattgaatgtggggtggttggggtatttatagccccaaaacaccaaaaaaggccgttggaaggctgctctcgcatggcgcaccggacagtccggtgcgccagccacgtcagcagaccgttggggttcgaccgttggagctctgacttgtggggcctctgggctgtccggtggtgcaccggacaggtcctgtaggatgtctggtgcgccaactgcacgtgctctgtcctctgcgcgcgcaggcgcgcattaaatgcgttgtagtcaaccgttgcgcgcgaagtagccattgctctgctggcacaccggacagtccggtgaattatagcggagcgccctctgattttcccgaaggtagcgagttcagcttcgagtgccctggtgcaccggacactgtccggtgcgccaaaccagggtgccttccgggatgtcttttgctctctttgtttgaaccctttcttggtctttttattggcttattgtgaacctttgacacctgtaaaacttatagactagagcaaactagttagtccaattatttgtgttggacaattcaaccaccaaaatcaattaggaaataggtgtgagcctaattccctttcaatctccccctttttggtgattgatgccaacacaaaccaaagcaagtatagaagtgcataattgaactagtttgcataatgtaagtgcaaaggttacttagaattgaaccaataaatattttcataagttatgcatggattgtttctttattttcatcattttggaccacgcttgcaccacatgttttgtttttgcaaatccttttgtaaatagtcaaaggtaaatgaataagattttgagaagcattttcaaaatttgaaattttctccccctgtttcaaatgcttttcctttgacttaaacaaaactcccccctcaaaaatcctactcatagtgttcaagagggttttaagatatcaattttgaaaatgctactttctcccccttttgaatataataagatatcaattgaaaaattcatcattttaaaaccttttgaaaatgggtggtggtgcggtccttttgctttgggctaatactttctccccctttggcatgaatcgccaaaaacgaatacttgagtgaaatataagcccctttaactactttctcctgctttggcgaacataatatgagtgaagattataccaaagttggagagttgcttgaagcgacggtgaaggatgagttatggagtggaggttaagcctttgtcttcgccgaagattccaattccctttcaatacacctatgacttggtttgaaatatacttgaaaacacattagtcatagcacatgaaagagatatgatcaaaggtatattaatgagctatgtatgcaagacatcaaaagaaattcctagaatcaagaatatttagctcgtgtctaagtttgttcatctagtggcttggtaaagatatcggctaattgttccttagtgttaatataggcaatctcgatatctccctttttttggtgatcccttaggaaatgataccgaatggctatgtgtttagtgcggctatgctcaacgggattatccgccatgcggattgcactctcattatcacatagaagaggaactttggttaatttttaaccatagtccctaagggtttgcctcatccaaagtaattgtgcgcaacaatggcctgcggcaatatactcggcttcggcggtagaaagagctacggaattttgcttctttgaagcccaagacaccagggaccttcccaagaactggcaagtccccgatgtactctttctattaattttacaccccgcccaatcggcatccgaataaccaatcaaatcaaatgtggatcccgtaggataccaaagcccaaacttaggagtatgaactaaatatctcaagattcgttttacggccgtaaggtgagcttccttagggtcggcttggaatcttgcacacatgcatacggaaagcataatatccggtcgagatgcacataaatagagtaaagagcctatcatcgaccggtataccttttgatcgacggatttacctcccgtgtcgaggtcgagatgcccattggttcccatgggtgtcttgatgggtttggcatccttcatcccatacttgtttagaatgtcttgaatgtacttcgtttggctaatgaaggtgccctcttagcgttgcttcacttgaaatcacaagaagtacttcaactcccccatcatagacatctcgaatttctgtgtcatgatcctactaaattcctcacatgtagattcattagtagacccaaatataatatcatcaacataaatttggcatacaaacaaatcattgtcaagagttttagtaaataaagtaggatcggcctttccgactttgaaaccattagtgataaggaaatctctaaggcattcataccatgctcttggggcttgcttgagcccataaagcgccttagagagtttatatacgtgattagggtactcactatcttcaaagccgggaggttgctcaacatagacctcttccttgattggtccgttgaggaaggcacttttcacgtccatttgataaagcttgaagccatggtaagtagcataggcaagtaatatgcgaattgactcaagcctagctacgggtgcataggtttcaccaaaatccaaaccttcgacttgtgaataacccttggccacaagtcgggctttgttccttgtcaccacaccatgctcatcttgtttgttgcggaagacccacttggttcctacaacattttgattaggacgtggaactaagtgacatacctcattcctagtgaagttgttgagctcctcttgcatcgccaccacccaatctgaatcctgtagtgcttcctctaccctttgtggctcaatagaggaaacaaaagagtaatgttcacaaaaatgagcaacacgagatcgagtagttacccccttttgaatatcgccgaggatggtgttcacggggtgatctcgttggattgcttggtggactcttgggtgtggcggtcttggttcttcatcctccttgtcttgatcatttgcatctcccccttgattattgccgtcatcttgaggtggctcatcttcttgatcttctcctttatcatcttgagcctcatcctcattttgagttggtggagatgcttgcgtggaggaggatggttgatcttgtgcatttggaggctctttggattccttaggacacacatccccaatggacatgttccttagcgcgacgcacggagcctcttcatcacctatctcatcaagatcaacttgctctacttgagagccgttagtttcatcaaacacaatgtcaccagaaacttcaactagtcccgaggacttgttaaagactctatatgcccttgtgtttgaatcataccctagtaaaaagccttctacagccttaggagcaaatttagattttctacctcttttaacaagaatgaagcatttgctaccaaagactctaaaatatgaaacattgggcttttaccggttaggagttcatatgatgtcttcttgaggattcggtgtagatataaccggttgatggtgtagcaagcggtgttgaccgcctcgatccaaaaccgatccgaagtcttgtactcatcaagcatggttcttgccatgtccaatagagttcgattcttcctctccactacaccattttgttgtggggtgtagggagaagagaactcatgcttgatgccctcctcctcaaggaagccttcgatttgagaattcttgaactccgtcccgttgtcgcttctaatctttttgattcttaagccgaactcattttgagcccatctcaagaatccctttaaggtctcttgggtatgagatttttcctgcaaaaagaatacccaagtgaagcgagtataatcatccacaataactagatagtacttactcccgccgatgcttatgtaagctatcgggccgaataggtccatatgtaggagctcgagtggcctgtcagtcatcatgatgttcttgtgtggatgatgagtaccaacttgcttccctgtctgacatgcgctacaaatcctatctttctcaaagtgaacatttgttagtcccaaaatgtgttctccctttagaagcttgtgaagattcttcattccaacatgtgctagtcggtgatgccagagccagcccatgttagtcttagcaattaagcaagtgtcgagttcagctctatcaaaatctaccaagtatagctgaccctctaacactcccttaaatgctactgaatcatcacttcttctaaagacagtaacacctatatctgtaaaaagacagttgtagcccattttacataattgcgaaactgaaagcaagttgtaatctaaagaatctacaagaaacacattggaaatggaatggtcaggagatatagcaattttacccaatcctttgaccaaaccttggtttccatccccgaatgtgatcgctctttggggatcttggtttttctcataggaggagaacattttcttctcccctgtcatatggtttgtgcacccgctatcgatgatccaacttgggcccccggatgcataaacctacaaaacaagtttagttcttgattttaggtacccaaatggttttgggtcctttgacattagatacaagaactttgggtacccaaacacaagtctttgatcccttgtgtttgcccccaacatacttggcaactatcttgtcggatttgttagttaaaacataagatgcatcaaaagttttgaatgaaatgttatgatcatttgatgcagcaggagttttcttcttaggcaattttgcacgggttgattgcctagagctagatgtctcacccttatacataaaagcatgattatggccagagtgagacttcctagaatgaattctcctaattttgctctcgggataaccggcagggtacaaaatgtaaccctcattatcctgaggcatgggagccttgcccttaacaaagtttgacaatcttttaggagaggcattaagtttgacattgtttcccttttggaagccaatgccatccttgatgccagggcgtctcccactatagagcatgcttctagcaaatttaaatttttcattttttaagtcatgctcggcaattttagcatctaattttgctatatgattattttgttgtttaattaaagccatatgatcatgaatagcatcaatgttaatatctctacatctagtgcaaataatgacatgctcaatggcagatgtagagggtttgcaagaattaagttcaacaatcttagcacgtaaaatatcattgttatttctaagatcagaaatggaagcattgcaaacatctaattctttagccttagcaatcaatttttcattttcaaccctaaggctagcaagagagacattcaattcttcaatcttagcaagcaaattaacattatcatctctaagattgggaattgaaacatcacaaatattagaatcaaccttagcaattagtttagtatttttatttctaaggatggtaatagtatcatggcaagtgcttagctcactagataatttttcacatttttctacttctagagcataagcatttttaaccttaacatgcttcttattttccttaattaggaagtcctcttgaaagtccaagagatcatctttctcatgaatagcactaattaattcatttagtttttcctgtagttgcatgtttaggttggcaaaaagggtacgcaaattatcctcctcatcactagcattatcttcatcactagaggatgcatatttagtggaggattttgattttaccttcttctttttgccgtcctttgccatgaggcacttgtggccgacgttggggaagaggagccctttggtgacggcgatgttggcggcgtcctcgtcggatgaggagtcggaggaactctcgtcggagtcccactcgcggcacacatgggcatcgccgcccttcttcttgtaatacctcctcttttctctcctcttgcccttcttgtcgtcgcccctgtcactatcactagataaaggacatttaacaatgaaatgaccgggcttaccacacttgtagcacacccttttggaacaaggcttgtaatctttccccttcctttgtttgaggatttggtggaagctcttgatgatgagcgccattttctagttgtcgagcttagaggcgtcgatgggttgtctacttgatgtagactcctctttcttctcctctgtcgccttgaatgcgaccggttgtgcttcgggcgtggagggaccgtcgtgctcgataattttctttgagcctttgatcatcaactcaaagctcacaaagtttcctattacttcctcgggagtcattagtgtatatctaggattaccacgaattaattgaacttgcgtagggttaaggaacacaagtgatctaagaataaccttaaccatttcatggtcatcccattttttgctcccgaggttgcgcacttggttcaccaaggtcttgagccggttgtacatatcttgtggctcctccccttggcgaagccggaagcgaccgagctccccctcgatcgtctcccgcttggtgatcttggttacctcgtctccttcgtgcgcggtctttagcacgtcccagatatcctttgcactcttcaacccttgcaccttattatactcctctcgacttggatttgaaatgttgg

SEQ ID NO: 61 - DNA, 1082 bp, Artificial Sequence
  cDNA Snare T3
cctgcccttccactcttcccccgctgcccccggtcaacgtcacgaacccgggcctcgtgccgctcgtcgtggccacactgttcgacgagcgagtcacagagctgctgagcgtgctcgctgatgcggcggtggggcgaccaggcaggtggtccatcggcgaagcgccatggtcgtcgtcggggggcacgaaccaggcggtgtacgcgcgccgcgcgcccggctcttcatcgcctccacccgctccagcgtctccaccacttccttcatcgagggccgactgcttggctcgctggccaggcagccgagcattagttgcgccgcttggaacgcctgcttttgttgatcgtttgttttggtctgatttcagtgggtctatccgcagagaggaagaagcagaagctctccgagatccaatccggcgttgaggaagctgaatcgctgattcagaaaatggacctggaggcaaggagcctacagcctagcattaaggctggtttgcttgcaaagccgagggattataaatctgacctcaacaacgtcaagagtgagctcaagaggatatctgcgcccaatgccagattcggaagatggacctggaagcaaggagcctacaacctagcattaagagtgagctcaagaggatatctgcgcccattgccaggcaggctacccgggaggagctcctggagtctggaatggctgatactctcgcagtgagctaatgctaggacttgactgtgtctacgagactgctcctaacaataaactgaagaaagcaaaagaaatcattcaacgtattcgccgaagagaactctacaagatatggtagtcctgggaggaagagccatcgccgctatgtatggcagaaccacccgcgaaagcaacctctctggtctcgcgtagccagagcaggagcagctcgcttgcgcggtcgcggcgctggcggccggccccgcgtacgagcgcctgcaggaagccaggaacccatccgaacaaggttgcaatcatgataagcagatagagcaagcatatgatgatattttgaattcgtcgaagcatactttggccagcatgatggagct

SEQ ID NO: 62 - DNA, 1154 bp, Artificial Sequence
  cDNA Snare T3
cctgcccttccactcttcccccgctgcccccggtcaacgtcacgaacccgggcctcgtgccgctcgtcgtggccacactgttcgacgagcgagtcacagagctgctgagcgtgctcgctgatgcggcggtggggcgaccaggcaggtggtccatcggcgaagcgccatggtcgtcgtcggggggcacgaaccaggcggtgtacgcgcgccgcgcgcccggctcttcatcgcctccacccgctccagcgtctccaccacttccttcatcgagggccgactgcttggctcgctggccaggcagccgagcattagttgcgccgcttggaacgcctgcttttgttgatcgtttgttttggtctgatttcagtgggtctatccgcagagaggaagaagcagaagctctccgagatccaatccggcgttgaggaagctgaatcgctgattcagaaaatggacctggaggcaaggagcctacagcctagcattaaggctggtttgcttgcaaagccgagggattataaatctgacctcaacaacgtcaagagtgagctcaagaggatatctgcgcccaatgccagactgctcctaataataaactgaagaaagcaaaagaaatcattcaacgtattcgccgaagagaactctacaagattcggaagatggacctggaagcaaggagcctacaacctagcattaagagtgagctcaagaggatatctgcgcccattgccaggcaggctacccgggaggagctcctggagtctggaatggctgatactctcgcagtgagctaatgctaggacttgactgtgtctacgagactgctcctaacaataaactgaagaaagcaaaagaaatcattcaacgtattcgccgaagagaactctacaagatatggtagtcctgggaggaagagccatcgccgctatgtatggcagaaccacccgcgaaagcaacctctctggtctcgcgtagccagagcaggagcagctcgcttgcgcggtcgcggcgctggcggccggccccgcgtacgagcgcctgcaggaagccaggaacccatccgaacaaggttgcaatcatgataagcagatagagcaagcatatgatgatattttgaattcgtcgaagcatactttggccagcatgatggagct

SEQ ID NO: 63 - protein, 107 aa, Zea mays
MIGLDCVYETAPNNKLKKAKEIIQRIRRRELYKEARNPSEQGCNHDKQIEQAYDDILNSSKHTLASMMELQEALLESNQATKDANEIPSASNGDNDEWSEVQRLQTR

SEQ ID NO: 64 - protein, 131 aa, Zea mays
MCSGLISYKKLLFHGLDLWTALSLPQPLGHAALWPPHRTIHQHLQCKCSWFSNELRSGIRILQEFFVLFAWIYTKGNAFKTPIDDESHLSLFSRTRIPRSVSVLYSFVFYKFRSTCVLTQWTSVMHMCKPA

SEQ ID NO: 65 - protein, 162 aa, Zea mays; identical to SEQ ID NO: 18